European Patent Specification EP 3 481 849 B1, published December 10, 2025. Title: CHIMERIC DENGUE/ZIKA VIRUSES AS LIVE-ATTENUATED ZIKA VIRUS VACCINES. Applicant: THE UNITED STATES OF AMERICA, AS REPRESENTED BY THE SECRETARY, DEPARTMENT OF HEALTH AND HUMAN SERVICES. The sequence listing filed with the application follows.

SEQUENCE LISTING (26 sequences)

SEQ ID NO: 1 - DNA, 10768 bp, Artificial Sequence
  Synthetic construct
agttgttagtctacgtggaccgacaaagacagattctttgagggagctaagctcaatgtagttctaacagttttttaattagagagcagatctctgatgaataaccaacggaaaaaggcgaaaaacacgcctttcaatatgctgaaacgcgagagaaaccgcgtgtcgactgtgcaacagctgacaaagagattctcacttggaatgctgcagggacgaggaccattaaaactgttcatggccctggtggcgttccttcgtttcctaacaatcccaccaacagcagggatattgaagagatggggaacaattaaaaaatcaaaagctattaatgttttgagagggttcaggaaagagattggaaggatgctgaacatcttgaataggagacgcagatccgcgggtactagtgtcggaattgttggcctcctgctgaccacagctatggcagcggaggtcactagacgtgggagtgcatactatatgtacttggacagaaacgatgctggggaggccatatcttttccaaccacattggggatgaataagtgttatatacagatcatggatcttggacacatgtgtgatgccaccatgagctatgaatgccctatgctggatgagggggtggaaccagatgacgtcgattgttggtgcaacacgacgtcaacttgggttgtgtacggaacctgccatcacaaaaaaggtgaagcacggagaagtagaagagctgtgacgctcccctcccattccactaggaagctgcaaacgcggtcgcaaacctggttggaatcaagagaatacacaaagcacttgattagagtcgaaaattggatattcaggaaccctggcttcgcgttagcagcagctgccatcgcttggcttttgggaagctcaacgagccaaaaagtcatatacttggtcatgatactgctgattgccccggcatacagcatcaggtgcataggagtcagcaatagggactttgtggaaggtatgtcaggtgggacttgggttgatattgtcttggaacatggaggttgtgtcaccgtaatggcacaggacaaaccgactgtcgacatagagctggttacaacaacagtcagcaacatggcggaggtaagatcctactgctatgaggcatcaatatcagacatggcttcggacagccgctgcccaacacaaggtgaagcctaccttgacaagcaatcagacactcaatatgtctgcaaaagaacgttagtggacagaggctggggaaatggatgtggactttttggcaaagggagtctggtgacatgcgctaagtttgcatgctccaagaaaatgaccgggaagagcatccagccagagaatctggagtaccggataatgctgtcagttcatggctcccagcacagtgggatgatcgttaatgacacaggacatgaaactgatgagaatagagcgaaggttgagataacgcccaattcaccaagagccgaagccaccctggggggttttggaagcctaggacttgattgtgaaccgaggacaggccttgacttttcagatttgtattacttgactatgaataacaagcactggttggttcacaaggagtggttccacgacattccattaccttggcacgctggggcagacaccggaactccacactggaacaacaaagaagcactggtagagttcaaggacgcacatgccaaaaggcaaactgtcgtggttctagggagtcaagaaggagcagttcacacggcccttgctggagctctggaggctgagatggatggtgcaaagggaaggctgtcctctggccacttgaaatgtcgcctgaaaatggataaacttagattgaagggcgtgtcatactccttgtgtaccgcagcgttcacattcaccaagatcccggctgaaacactgcacgggacagtcacagtggaggtacagtacgcagggacagatggaccttgcaaggttccagctcagatggcggtggacatgcaaactctgaccccagttgggaggttgataaccgctaaccccgtaatcactgaaagcactgagaactctaagatgatgctggaacttgatccaccatttggggactcttacattgtcataggagtcggggagaagaagatcacccaccactggcacaggagtggcagcaccattggaaaagcatttgaagccactgtgagaggtgccaagagaatggcagtcttgggagacacagcctgggactttggatcagttggaggcgctctcaactcattgggcaagggcatccatcaaatttttggagcagctttcaaatcattgtttggaggaatgtcctggttctcacaaattctcattggaacgttgctgatgtggttgggtctgaacacaaagaatggatctatttcccttatgtgcttggccgccggcattgtgacactgtatttgggagtcatggtgcaggccgatagtggttgcgttgtgagctggaaaaacaaagaactgaaatgtggcagtgggattttcatcacagacaacgtgcacacatggacagaacaatacaagttccaaccagaatccccttcaaaactagcttcagctatccagaaagcccatgaagaggacatttgtggaatccgctcagtaacaagactggagaatctgatgtggaaacaaataacaccagaattgaatcacattctatcagaaaatgaggtgaagttaactattatgacaggagacatcaaaggaatcatgcaggcaggaaaacgatctctgcggcctcagcccactgagctgaagtattcatggaaaacatggggcaaagcaaaaatgctctctacagagtctcataaccagacctttctcattgatggccccgaaacagcagaatgccccaacacaaatagagcttggaattcgttggaagttgaagactatggctttggagtattcaccaccaatatatggctaaaattgaaagaaaaacaggatgtattctgcgactcaaaactcatgtcagcggccataaaagacaacagagccgtccatgccgatatgggttattggatagaaagtgcactcaatgacacatggaagatagagaaagcctctttcattgaagttaaaaactgccactggccaaaatcacacaccctctggagcaatggagtgctagaaagtgagatgataattccaaagaatctcgctggaccagtgtctcaacacaactatagaccaggctaccatacacaaataacaggaccatggcatctaggtaagcttgagatggactttgatttctgtgatggaacaacagtggtagtgactgaggactgcggaaatagaggaccctctttgagaacaaccactgcctctggaaaactcataacagaatggtgctgccgatcttgcacattaccaccgctaagatacagaggtgaggatgggtgctggtacgggatggaaatcagaccattgaaggagaaagaagagaatttggtcaactccttggtcacagctggacatgggcaggtcgacaacttttcactaggagtcttgggaatggcattgttcctggaggaaatgcttaggacccgagtaggaacgaaacatgcaatactactagttgcagtttcttttgtgacattgatcacagggaacatgtcctttagagacctgggaagagtgatggttatggtaggcgccactatgacggatgacataggtatgggcgtgacttatcttgccctactagcagccttcaaagtcagaccaacttttgcagctggactactcttgagaaagctgacctccaaggaattgatgatgactactataggaattgtactcctctcccagagcaccataccagagaccattcttgagttgactgatgcgttagccttaggcatgatggtcctcaaaatggtgagaaatatggaaaagtatcaattggcagtgactatcatggctatcttgtgcgtcccaaacgcagtgatattacaaaacgcatggaaagtgagttgcacaatattggcagtggtgtccgtttccccactgttcttaacatcctcacagcaaaaaacagattggataccattagcattgacgatcaaaggtctcaatccaacagctatttttctaacaaccctctcaagaaccagcaagaaaaggagctggccattaaatgaggctatcatggcagtcgggatggtgagcattttagccagttctctcctaaaaaatgatattcccatgacaggaccattagtggctggagggctcctcactgtgtgctacgtgctcactggacgatcggccgatttggaactggagagagcagccgatgtcaaatgggaagaccaggcagagatatcaggaagcagtccaatcctgtcaataacaatatcagaagatggtagcatgtcgataaaaaatgaagaggaagaacaaacactgaccatactcattagaacaggattgctggtgatctcaggactttttcctgtatcaataccaatcacggcagcagcatggtacctgtgggaagtgaagaaacaacgggccggagtattgtgggatgttccttcacccccacccatgggaaaggctgaactggaagatggagcctatagaattaagcaaaaagggattcttggatattcccagatcggagccggagtttacaaagaaggaacattccatacaatgtggcatgtcacacgtggcgctgttctaatgcataaaggaaagaggattgaaccatcatgggcggacgtcaagaaagacctaatatcatatggaggaggctggaagttagaaggagaatggaaggaaggagaagaagtccaggtattggcactggagcctggaaaaaatccaagagccgtccaaacgaaacctggtcttttcaaaaccaacgccggaacaataggtgctgtatctctggacttttctcctggaacgtcaggatctccaattatcgacaaaaaaggaaaagttgtgggtctttatggtaatggtgttgttacaaggagtggagcatatgtgagtgctatagcccagactgaaaaaagcattgaagacaacccagagatcgaagatgacattttccgaaagagaagactgaccatcatggacctccacccaggagcgggaaagacgaagagataccttccggccatagtcagagaagctataaaacggggtttgagaacattaatcttggcccccactagagttgtggcagctgaaatggaggaagcccttagaggacttccaataagataccagaccccagccatcagagctgtgcacaccgggcgggagattgtggacctaatgtgtcatgccacatttaccatgaggctgctatcaccagttagagtgccaaactacaacctgattatcatggacgaagcccatttcacagacccagcaagtatagcagctagaggatacatctcaactcgagtggagatgggtgaggcagctgggatttttatgacagccactcccccgggaagcagagacccatttcctcagagcaatgcaccaatcatagatgaagaaagagaaatccctgaacgctcgtggaattccggacatgaatgggtcacggattttaaagggaagactgtttggttcgttccaagtataaaagcaggaaatgatatagcagcttgcctgaggaaaaatggaaagaaagtgatacaactcagtaggaagacctttgattctgagtatgtcaagactagaaccaatgattgggacttcgtggttacaactgacatttcagaaatgggtgccaatttcaaggctgagagggttatagaccccagacgctgcatgaaaccagtcatactaacagatggtgaagagcgggtgattctggcaggacctatgccagtgacccactctagtgcagcacaaagaagagggagaataggaagaaatccaaaaaatgagaatgaccagtacatatacatgggggaacctctggaaaatgatgaagactgtgcacactggaaagaagctaaaatgctcctagataacatcaacacgccagaaggaatcattcctagcatgttcgaaccagagcgtgaaaaggtggatgccattgatggcgaataccgcttgagaggagaagcaaggaaaacctttgtagacttaatgagaagaggagacctaccagtctggttggcctacagagtggcagctgaaggcatcaactacgcagacagaaggtggtgttttgatggagtcaagaacaaccaaatcctagaagaaaacgtggaagttgaaatctggacaaaagaaggggaaaggaagaaattgaaacccagatggttggatgctaggatctattctgacccactggcgctaaaagaatttaaggaatttgcagccggaagaaagtctctgaccctgaacctaatcacagaaatgggtaggctcccaaccttcatgactcagaaggcaagagacgcactggacaacttagcagtgctgcacacggctgaggcaggtggaagggcgtacaaccatgctctcagtgaactgccggagaccctggagacattgcttttactgacacttctggctacagtcacgggagggatctttttattcttgatgagcgcaaggggcatagggaagatgaccctgggaatgtgctgcataatcacggctagcatcctcctatggtacgcacaaatacagccacactggatagcagcttcaataatactggagttttttctcatagttttgcttattccagaacctgaaaaacagagaacaccccaagacaaccaactgacctacgttgtcatagccatcctcacagtggtggccgcaaccatggcaaacgagatgggtttcctagaaaaaacgaagaaagatctcggattgggaagcattgcaacccagcaacccgagagcaacatcctggacatagatctacgtcctgcatcagcatggacgctgtatgccgtggccacaacatttgttacaccaatgttgagacatagcattgaaaattcctcagtgaatgtgtccctaacagctatagccaaccaagccacagtgttaatgggtctcgggaaaggatggccattgtcaaagatggacatcggagttccccttctcgccattggatgctactcacaagtcaaccccataactctcacagcagctcttttcttattggtagcacattatgccatcatagggccaggactccaagcaaaagcaaccagagaagctcagaaaagagcagcggcgggcatcatgaaaaacccaactgtcgatggaataacagtgattgacctagatccaataccttatgatccaaagtttgaaaagcagttgggacaagtaatgctcctagtcctctgcgtgactcaagtattgatgatgaggactacatgggctctgtgtgaggctttaaccttagctaccgggcccatctccacattgtgggaaggaaatccagggaggttttggaacactaccattgcggtgtcaatggctaacatttttagagggagttacttggccggagctggacttctcttttctattatgaagaacacaaccaacacaagaaggggaactggcaacataggagagacgcttggagagaaatggaaaagccgattgaacgcattgggaaaaagtgaattccagatctacaagaaaagtggaatccaggaagtggatagaaccttagcaaaagaaggcattaaaagaggagaaacggaccatcacgctgtgtcgcgaggctcagcaaaactgagatggttcgttgagagaaacatggtcacaccagaagggaaagtagtggacctcggttgtggcagaggaggctggtcatactattgtggaggactaaagaatgtaagagaagtcaaaggcctaacaaaaggaggaccaggacacgaagaacccatccccatgtcaacatatgggtggaatctagtgcgtcttcaaagtggagttgacgttttcttcatcccgccagaaaagtgtgacacattattgtgtgacataggggagtcatcaccaaatcccacagtggaagcaggacgaacactcagagtccttaacttagtagaaaattggttgaacaacaacactcaattttgcataaaggttctcaacccatatatgccctcagtcatagaaaaaatggaagcactacaaaggaaatatggaggagccttagtgaggaatccactctcacgaaactccacacatgagatgtactgggtatccaatgcttccgggaacatagtgtcatcagtgaacatgatttcaaggatgttgatcaacagatttacaatgagatacaagaaagccacttacgagccggatgttgacctcggaagcggaacccgtaacatcgggattgaaagtgagataccaaacctagatataattgggaaaagaatagaaaaaataaagcaagagcatgaaacatcatggcactatgaccaagaccacccatacaaaacgtgggcataccatggtagctatgaaacaaaacagactggatcagcatcatccatggtcaacggagtggtcaggctgctgacaaaaccttgggacgtcgtccccatggtgacacagatggcaatgacagacacgactccatttggacaacagcgcgtttttaaagagaaagtggacacgagaacccaagaaccgaaagaaggcacgaagaaactaatgaaaataacagcagagtggctttggaaagaattagggaagaaaaagacacccaggatgtgcaccagagaagaattcacaagaaaggtgagaagcaatgcagccttgggggccatattcactgatgagaacaagtggaagtcggcacgtgaggctgttgaagatagtaggttttgggagctggttgacaaggaaaggaatctccatcttgaaggaaagtgtgaaacatgtgtgtacaacatgatgggaaaaagagagaagaagctaggggaattcggcaaggcaaaaggcagcagagccatatggtacatgtggcttggagcacgcttcttagagtttgaagccctaggattcttaaatgaagatcactggttctccagagagaactccctgagtggagtggaaggagaagggctgcacaagctaggttacattctaagagacgtgagcaagaaagagggaggagcaatgtatgccgatgacaccgcaggatgggatacaagaatcacactagaagacctaaaaaatgaagaaatggtaacaaaccacatggaaggagaacacaagaaactagccgaggccattttcaaactaacgtaccaaaacaaggtggtgcgtgtgcaaagaccaacaccaagaggcacagtaatggacatcatatcgagaagagaccaaagaggtagtggacaagttggcacctatggactcaatactttcaccaatatggaagcccaactaatcagacagatggagggagaaggagtctttaaaagcattcagcacctaacaatcacagaagaaatcgctgtgcaaaactggttagcaagagtggggcgcgaaaggttatcaagaatggccatcagtggagatgattgtgttgtgaaacctttagatgacaggttcgcaagcgctttaacagctctaaatgacatgggaaagattaggaaagacatacaacaatgggaaccttcaagaggatggaatgattggacacaagtgcccttctgttcacaccatttccatgagttaatcatgaaagacggtcgcgtactcgttgttccatgtagaaaccaagatgaactgattggcagagcccgaatctcccaaggagcagggtggtctttgcgggagacggcctgtttggggaagtcttacgcccaaatgtggagcttgatgtacttccacagacgcgacctcaggctggcggcaaatgctatttgctcggcagtaccatcacattgggttccaacaagtcgaacaacctggtccatacatgctaaacatgaatggatgacaacggaagacatgctgacagtctggaacagggtgtggattcaagaaaacccatggatggaagacaaaactccagtggaatcatgggaggaaatcccatacttggggaaaagagaagaccaatggtgcggctcattgattgggttaacaagcagggccacctgggcaaagaacatccaagcagcaataaatcaagttagatcccttataggcaatgaagaatacacagattacatgccatccatgaaaagattcagaagagaagaggaagaagcaggagttctgtggtagaaagcaaaactaacatgaaacaaggctagaagtcaggtcggattaagccatagtacggaaaaaactatgctacctgtgagccccgtccaaggacgttaaaagaagtcaggccatcataaatgccatagcttgagtaaactatgcagcctgtagctccacctgagaaggtgtaaaaaatccgggaggccacaaaccatggaagctgtacgcatggcgtagtggactagcggttagaggagacccctcccttacaaatcgcagcaacaatgggggcccaaggcgagatgaagctgtagtctcgctggaaggactagaggttagaggagacccccccgaaacaaaaaacagcatattgacgctgggaaagaccagagatcctgctgtctcctcagcatcattccaggcacagaacgccagaaaatggaatggtgctgttgaatcaacaggttct

SEQ ID NO: 2 - protein, 3406 aa, Artificial Sequence
  Synthetic polypeptide
MNNQRKKAKNTPFNMLKRERNRVSTVQQLTKRFSLGMLQGRGPLKLFMALVAFLRFLTIPPTAGILKRWGTIKKSKAINVLRGFRKEIGRMLNILNRRRRSAGTSVGIVGLLLTTAMAAEVTRRGSAYYMYLDRNDAGEAISFPTTLGMNKCYIQIMDLGHMCDATMSYECPMLDEGVEPDDVDCWCNTTSTWVVYGTCHHKKGEARRSRRAVTLPSHSTRKLQTRSQTWLESREYTKHLIRVENWIFRNPGFALAAAAIAWLLGSSTSQKVIYLVMILLIAPAYSIRCIGVSNRDFVEGMSGGTWVDIVLEHGGCVTVMAQDKPTVDIELVTTTVSNMAEVRSYCYEASISDMASDSRCPTQGEAYLDKQSDTQYVCKRTLVDRGWGNGCGLFGKGSLVTCAKFACSKKMTGKSIQPENLEYRIMLSVHGSQHSGMIVNDTGHETDENRAKVEITPNSPRAEATLGGFGSLGLDCEPRTGLDFSDLYYLTMNNKHWLVHKEWFHDIPLPWHAGADTGTPHWNNKEALVEFKDAHAKRQTVVVLGSQEGAVHTALAGALEAEMDGAKGRLSSGHLKCRLKMDKLRLKGVSYSLCTAAFTFTKIPAETLHGTVTVEVQYAGTDGPCKVPAQMAVDMQTLTPVGRLITANPVITESTENSKMMLELDPPFGDSYIVIGVGEKKITHHWHRSGSTIGKAFEATVRGAKRMAVLGDTAWDFGSVGGALNSLGKGIHQIFGAAFKSLFGGMSWFSQILIGTLLMWLGLNTKNGSISLMCLAAGIVTLYLGVMVQADSGCVVSWKNKELKCGSGIFITDNVHTWTEQYKFQPESPSKLASAIQKAHEEDICGIRSVTRLENLMWKQITPELNHILSENEVKLTIMTGDIKGIMQAGKRSLRPQPTELKYSWKTWGKAKMLSTESHNQTFLIDGPETAECPNTNRAWNSLEVEDYGFGVFTTNIWLKLKEKQDVFCDSKLMSAAIKDNRAVHADMGYWIESALNDTWKIEKASFIEVKNCHWPKSHTLWSNGVLESEMIIPKNLAGPVSQHNYRPGYHTQITGPWHLGKLEMDFDFCDGTTVVVTEDCGNRGPSLRTTTASGKLITEWCCRSCTLPPLRYRGEDGCWYGMEIRPLKEKEENLVNSLVTAGHGQVDNFSLGVLGMALFLEEMLRTRVGTKHAILLVAVSFVTLITGNMSFRDLGRVMVMVGATMTDDIGMGVTYLALLAAFKVRPTFAAGLLLRKLTSKELMMTTIGIVLLSQSTIPETILELTDALALGMMVLKMVRNMEKYQLAVTIMAILCVPNAVILQNAWKVSCTILAVVSVSPLFLTSSQQKTDWIPLALTIKGLNPTAIFLTTLSRTSKKRSWPLNEAIMAVGMVSILASSLLKNDIPMTGPLVAGGLLTVCYVLTGRSADLELERAADVKWEDQAEISGSSPILSITISEDGSMSIKNEEEEQTLTILIRTGLLVISGLFPVSIPITAAAWYLWEVKKQRAGVLWDVPSPPPMGKAELEDGAYRIKQKGILGYSQIGAGVYKEGTFHTMWHVTRGAVLMHKGKRIEPSWADVKKDLISYGGGWKLEGEWKEGEEVQVLALEPGKNPRAVQTKPGLFKTNAGTIGAVSLDFSPGTSGSPIIDKKGKVVGLYGNGVVTRSGAYVSAIAQTEKSIEDNPEIEDDIFRKRRLTIMDLHPGAGKTKRYLPAIVREAIKRGLRTLILAPTRVVAAEMEEALRGLPIRYQTPAIRAVHTGREIVDLMCHATFTMRLLSPVRVPNYNLIIMDEAHFTDPASIAARGYISTRVEMGEAAGIFMTATPPGSRDPFPQSNAPIIDEEREIPERSWNSGHEWVTDFKGKTVWFVPSIKAGNDIAACLRKNGKKVIQLSRKTFDSEYVKTRTNDWDFVVTTDISEMGANFKAERVIDPRRCMKPVILTDGEERVILAGPMPVTHSSAAQRRGRIGRNPKNENDQYIYMGEPLENDEDCAHWKEAKMLLDNINTPEGIIPSMFEPEREKVDAIDGEYRLRGEARKTFVDLMRRGDLPVWLAYRVAAEGINYADRRWCFDGVKNNQILEENVEVEIWTKEGERKKLKPRWLDARIYSDPLALKEFKEFAAGRKSLTLNLITEMGRLPTFMTQKARDALDNLAVLHTAEAGGRAYNHALSELPETLETLLLLTLLATVTGGIFLFLMSARGIGKMTLGMCCIITASILLWYAQIQPHWIAASIILEFFLIVLLIPEPEKQRTPQDNQLTYVVIAILTVVAATMANEMGFLEKTKKDLGLGSIATQQPESNILDIDLRPASAWTLYAVATTFVTPMLRHSIENSSVNVSLTAIANQATVLMGLGKGWPLSKMDIGVPLLAIGCYSQVNPITLTAALFLLVAHYAIIGPGLQAKATREAQKRAAAGIMKNPTVDGITVIDLDPIPYDPKFEKQLGQVMLLVLCVTQVLMMRTTWALCEALTLATGPISTLWEGNPGRFWNTTIAVSMANIFRGSYLAGAGLLFSIMKNTTNTRRGTGNIGETLGEKWKSRLNALGKSEFQIYKKSGIQEVDRTLAKEGIKRGETDHHAVSRGSAKLRWFVERNMVTPEGKVVDLGCGRGGWSYYCGGLKNVREVKGLTKGGPGHEEPIPMSTYGWNLVRLQSGVDVFFIPPEKCDTLLCDIGESSPNPTVEAGRTLRVLNLVENWLNNNTQFCIKVLNPYMPSVIEKMEALQRKYGGALVRNPLSRNSTHEMYWVSNASGNIVSSVNMISRMLINRFTMRYKKATYEPDVDLGSGTRNIGIESEIPNLDIIGKRIEKIKQEHETSWHYDQDHPYKTWAYHGSYETKQTGSASSMVNGVVRLLTKPWDVVPMVTQMAMTDTTPFGQQRVFKEKVDTRTQEPKEGTKKLMKITAEWLWKELGKKKTPRMCTREEFTRKVRSNAALGAIFTDENKWKSAREAVEDSRFWELVDKERNLHLEGKCETCVYNMMGKREKKLGEFGKAKGSRAIWYMWLGARFLEFEALGFLNEDHWFSRENSLSGVEGEGLHKLGYILRDVSKKEGGAMYADDTAGWDTRITLEDLKNEEMVTNHMEGEHKKLAEAIFKLTYQNKVVRVQRPTPRGTVMDIISRRDQRGSGQVGTYGLNTFTNMEAQLIRQMEGEGVFKSIQHLTITEEIAVQNWLARVGRERLSRMAISGDDCVVKPLDDRFASALTALNDMGKIRKDIQQWEPSRGWNDWTQVPFCSHHFHELIMKDGRVLVVPCRNQDELIGRARISQGAGWSLRETACLGKSYAQMWSLMYFHRRDLRLAANAICSAVPSHWVPTSRTTWSIHAKHEWMTTEDMLTVWNRVWIQENPWMEDKTPVESWEEIPYLGKREDQWCGSLIGLTSRATWAKNIQAAINQVRSLIGNEEYTDYMPSMKRFRREEEEAGVLW

SEQ ID NO: 3 - DNA, 10768 bp, Artificial Sequence
  Synthetic construct
agttgttagtctacgtggaccgacaaagacagattctttgagggagctaagctcaatgtagttctaacagttttttaattagagagcagatctctgatgaataaccaacggaaaaaggcgaaaaacacgcctttcaatatgctgaaacgcgagagaaaccgcgtgtcgactgtgcaacagctgacaaagagattctcacttggaatgctgcagggacgaggaccattaaaactgttcatggccctggtggcgttccttcgtttcctaacaatcccaccaacagcagggatattgaagagatggggaacaattaaaaaatcaaaagctattaatgttttgagagggttcaggaaagagattggaaggatgctgaacatcttgaataggagacgcagatccgcgggtatgatcgtcggaattgttggcctcctgctgaccacagctatggcagcggaggtcactagacgtgggagtgcatactatatgtacttggacagaaacgatgctggggaggccatatcttttccaaccacattggggatgaataagtgttatatacagatcatggatcttggacacatgtgtgatgccaccatgagctatgaatgccctatgctggatgagggggtggaaccagatgacgtcgattgttggtgcaacacgacgtcaacttgggttgtgtacggaacctgccatcacaaaaaaggtgaagcacggagaagtagaagagctgtgacgctcccctcccattccactaggaagctgcaaacgcggtcgcaaacctggttggaatcaagagaatacacaaagcacttgattagagtcgaaaattggatattcaggaaccctggcttcgcgttagcagcagctgccatcgcttggcttttgggaagctcaacgagccaaaaagtcatatacttggtcatgatactgctgattgccccggcatacagcatcaggtgcataggagtcagcaatagggactttgtggaaggtatgtcaggtgggacttgggttgatattgtcttggaacatggaggttgtgtcaccgtaatggcacaggacaaaccgactgtcgacatagagctggttacaacaacagtcagcaacatggcggaggtaagatcctactgctatgaggcatcaatatcagacatggcttcggacagccgctgcccaacacaaggtgaagcctaccttgacaagcaatcagacactcaatatgtctgcaaaagaacgttagtggacagaggctggggaaatggatgtggactttttggcaaagggagtctggtgacatgcgctaagtttgcatgctccaagaaaatgaccgggaagagcatccagccagagaatctggagtaccggataatgctgtcagttcatggctcccagcacagtgggatgatcgttaatgacacaggacatgaaactgatgagaatagagcgaaggttgagataacgcccaattcaccaagagccgaagccaccctggggggttttggaagcctaggacttgattgtgcaccgaggacaggccttgacttttcagatttgtattacttgactatgaataacaagcactggttggttcacaaggagtggttccacgacattccattaccttggcacgctggggcagacaccggaactccacactggaacaacaaagaagcactggtagagttcaaggacgcacatgccaaaaggcaaactgtcgtggttctagggagtcaagaaggagcagttcacacggcccttgctggagctctggaggctgagatggatggtgcaaagggaaggctgtcctctggccacttgaaatgtcgcctgaaaatggataaacttagattgaagggcgtgtcatactccttgtgtaccgcagcgttcacattcaccaagatcccggctgaaacactgcacgggacagtcacagtggaggtacagtacgcagggacagatggaccttgcaaggttccagctcagatggcggtggacatgcaaactctgaccccagttgggaggttgataaccgctaaccccgtaatcactgaaagcactgagaactctaagatgatgctggaacttgatccaccatttggggactcttacattgtcataggagtcggggagaagaagatcacccaccactggcacaggagtggcagcaccattggaaaagcatttgaagccactgtgagaggtgccaagagaatggcagtcttgggagacacagcctgggactttggatcagttggaggcgctctcaactcattgggcaagggcatccatcaaatttttggagcagctttcaaatcattgtttggaggaatgtcctggttctcacaaattctcattggaacgttgctgatgtggttgggtctgaacacaaagaatggatctatttcccttatgtgcttggccgccggcattgtgacactgtatttgggagtcatggtgcaggccgatagtggttgcgttgtgagctggaaaaacaaagaactgaaatgtggcagtgggattttcatcacagacaacgtgcacacatggacagaacaatacaagttccaaccagaatccccttcaaaactagcttcagctatccagaaagcccatgaagaggacatttgtggaatccgctcagtaacaagactggagaatctgatgtggaaacaaataacaccagaattgaatcacattctatcagaaaatgaggtgaagttaactattatgacaggagacatcaaaggaatcatgcaggcaggaaaacgatctctgcggcctcagcccactgagctgaagtattcatggaaaacatggggcaaagcaaaaatgctctctacagagtctcataaccagacctttctcattgatggccccgaaacagcagaatgccccaacacaaatagagcttggaattcgttggaagttgaagactatggctttggagtattcaccaccaatatatggctaaaattgaaagaaaaacaggatgtattctgcgactcaaaactcatgtcagcggccataaaagacaacagagccgtccatgccgatatgggttattggatagaaagtgcactcaatgacacatggaagatagagaaagcctctttcattgaagttaaaaactgccactggccaaaatcacacaccctctggagcaatggagtgctagaaagtgagatgataattccaaagaatctcgctggaccagtgtctcaacacaactatagaccaggctaccatacacaaataacaggaccatggcatctaggtaagcttgagatggactttgatttctgtgatggaacaacagtggtagtgactgaggactgcggaaatagaggaccctctttgagaacaaccactgcctctggaaaactcataacagaatggtgctgccgatcttgcacattaccaccgctaagatacagaggtgaggatgggtgctggtacgggatggaaatcagaccattgaaggagaaagaagagaatttggtcaactccttggtcacagctggacatgggcaggtcgacaacttttcactaggagtcttgggaatggcattgttcctggaggaagtgcttaggacccgagtaggaacgaaacatgcaatactactagttgcagtttcttttgtgacattgatcacagggaacatgtcctttagagacctgggaagagtgatggttatggtaggcgccactatgacggatgacataggtatgggcgtgacttatcttgccctactagcagccttcaaagtcagaccaacttttgcagctggactactcttgagaaagctgacctccaaggaattgatgatgactactataggaattgtactcctctcccagagcaccataccagagaccattcttgagttgactgatgcgttagccttaggcatgatggtcctcaaaatggtgagaaatatggaaaagtatcaattggcagtgactatcatggctatcttgtgcgtcccaaacgcagtgatattacaaaacgcatggaaagtgagttgcacaatattggcagtggtgtccgtttccccactgttcttaacatcctcacagcaaaaaacagattggataccattagcattgacgatcaaaggtctcaatccaacagctatttttctaacaaccctctcaagaaccagcaagaaaaggagctggccattaaatgaggctatcatggcagtcgggatggtgagcattttagccagttctctcctaaaaaatgatattcccatgacaggaccattagtggctggagggctcctcactgtgtgctacgtgctcactggacgatcggccgatttggaactggagagagcagccgatgtcaaatgggaagaccaggcagagatatcaggaagcagtccaatcctgtcaataacaatatcagaagatggtagcatgtcgataaaaaatgaagaggaagaacaaacactgaccatactcattagaacaggattgctggtgatctcaggactttttcctgtatcaataccaatcacggcagcagcatggtacctgtgggaagtgaagaaacaacgggccggagtattgtgggatgttccttcacccccacccatgggaaaggctgaactggaagatggagcctatagaattaagcaaaaagggattcttggatattcccagatcggagccggagtttacaaagaaggaacattccatacaatgtggcatgtcacacgtggcgctgttctaatgcataaaggaaagaggattgaaccatcatgggcggacgtcaagaaagacctaatatcatatggaggaggctggaagttagaaggagaatggaaggaaggagaagaagtccaggtattggcactggagcctggaaaaaatccaagagccgtccaaacgaaacctggtcttttcaaaaccaacgccggaacaataggtgctgtatctctggacttttctcctggaacgtcaggatctccaattatcgacaaaaaaggaaaagttgtgggtctttatggtaatggtgttgttacaaggagtggagcatatgtgagtgctatagcccagactgaaaaaagcattgaagacaacccagagatcgaagatgacattttccgaaagagaagactgaccatcatggacctccacccaggagcgggaaagacgaagagataccttccggccatagtcagagaagctataaaacggggtttgagaacattaatcttggcccccactagagttgtggcagctgaaatggaggaagcccttagaggacttccaataagataccagaccccagccatcagagctgtgcacaccgggcgggagattgtggacctaatgtgtcatgccacatttaccatgaggctgctatcaccagttagagtgccaaactacaacctgattatcatggacgaagcccatttcacagacccagcaagtatagcagctagaggatacatctcaactcgagtggagatgggtgaggcagctgggatttttatgacagccactcccccgggaagcagagacccatttcctcagagcaatgcaccaatcatagatgaagaaagagaaatccctgaacgctcgtggaattccggacatgaatgggtcacggattttaaagggaagactgtttggttcgttccaagtataaaagcaggaaatgatatagcagcttgcctgaggaaaaatggaaagaaagtgatacaactcagtaggaagacctttgattctgagtatgtcaagactagaaccaatgattgggacttcgtggttacaactgacatttcagaaatgggtgccaatttcaaggctgagagggttatagaccccagacgctgcatgaaaccagtcatactaacagatggtgaagagcgggtgattctggcaggacctatgccagtgacccactctagtgcagcacaaagaagagggagaataggaagaaatccaaaaaatgagaatgaccagtacatatacatgggggaacctctggaaaatgatgaagactgtgcacactggaaagaagctaaaatgctcctagataacatcaacacgccagaaggaatcattcctagcatgttcgaaccagagcgtgaaaaggtggatgccattgatggcgaataccgcttgagaggagaagcaaggaaaacctttgtagacttaatgagaagaggagacctaccagtctggttggcctacagagtggcagctgaaggcatcaactacgcagacagaaggtggtgttttgatggagtcaagaacaaccaaatcctagaagaaaacgtggaagttgaaatctggacaaaagaaggggaaaggaagaaattgaaacccagatggttggatgctaggatctattctgacccactggcgctaaaagaatttaaggaatttgcagccggaagaaagtctctgaccctgaacctaatcacagaaatgggtaggctcccaaccttcatgactcagaaggcaagagacgcactggacaacttagcagtgctgcacacggctgaggcaggtggaagggcgtacaaccatgctctcagtgaactgccggagaccctggagacattgcttttactgacacttctggctacagtcacgggagggatctttttattcttgatgagcgcaaggggcatagggaagatgaccctgggaatgtgctgcataatcacggctagcatcctcctatggtacgcacaaatacagccacactggatagcagcttcaataatactggagttttttctcatagttttgcttattccagaacctgaaaaacagagaacaccccaagacaaccaactgacctacgttgtcatagccatcctcacagtggtggccgcaaccatggcaaacgagatgggtttcctagaaaaaacgaagaaagatctcggattgggaagcattgcaacccagcaacccgagagcaacatcctggacatagatctacgtcctgcatcagcatggacgctgtatgccgtggccacaacatttgttacaccaatgttgagacatagcattgaaaattcctcagtgaatgtgtccctaacagctatagccaaccaagccacagtgttaatgggtctcgggaaaggatggccattgtcaaagatggacatcggagttccccttctcgccattggatgctactcacaagtcaaccccataactctcacagcagctcttttcttattggtagcacattatgccatcatagggccaggactccaagcaaaagcaaccagagaagctcagaaaagagcagcggcgggcatcatgaaaaacccaactgtcgatggaataacagtgattgacctagatccaataccttatgatccaaagtttgaaaagcagttgggacaagtaatgctcctagtcctctgcgtgactcaagtattgatgatgaggactacatgggctctgtgtgaggctttaaccttagctaccgggcccatctccacattgtgggaaggaaatccagggaggttttggaacactaccattgcggtgtcaatggctaacatttttagagggagttacttggccggagctggacttctcttttctattatgaagaacacaaccaacacaagaaggggaactggcaacataggagagacgcttggagagaaatggaaaagccgattgaacgcattgggaaaaagtgaattccagatctacaagaaaagtggaatccaggaagtggatagaaccttagcaaaagaaggcattaaaagaggagaaacggaccatcacgctgtgtcgcgaggctcagcaaaactgagatggttcgttgagagaaacatggtcacaccagaagggaaagtagtggacctcggttgtggcagaggaggctggtcatactattgtggaggactaaagaatgtaagagaagtcaaaggcctaacaaaaggaggaccaggacacgaagaacccatccccatgtcaacatatgggtggaatctagtgcgtcttcaaagtggagttgacgttttcttcatcccgccagaaaagtgtgacacattattgtgtgacataggggagtcatcaccaaatcccacagtggaagcaggacgaacactcagagtccttaacttagtagaaaattggttgaacaacaacactcaattttgcataaaggttctcaacccatatatgccctcagtcatagaaaaaatggaagcactacaaaggaaatatggaggagccttagtgaggaatccactctcacgaaactccacacatgagatgtactgggtatccaatgcttccgggaacatagtgtcatcagtgaacatgatttcaaggatgttgatcaacagatttacaatgagatacaagaaagccacttacgagccggatgttgacctcggaagcggaacccgtaacatcgggattgaaagtgagataccaaacctagatataattgggaaaagaatagaaaaaataaagcaagagcatgaaacatcatggcactatgaccaagaccacccatacaaaacgtgggcataccatggtagctatgaaacaaaacagactggatcagcatcatccatggtcaacggagtggtcaggctgctgacaaaaccttgggacgtcgtccccatggtgacacagatggcaatgacagacacgactccatttggacaacagcgcgtttttaaagagaaagtggacacgagaacccaagaaccgaaagaaggcacgaagaaactaatgaaaataacagcagagtggctttggaaagaattagggaagaaaaagacacccaggatgtgcaccagagaagaattcacaagaaaggtgagaagcaatgcagccttgggggccatattcactgatgagaacaagtggaagtcggcacgtgaggctgttgaagatagtaggttttgggagctggttgacaaggaaaggaatctccatcttgaaggaaagtgtgaaacatgtgtgtacaacatgatgggaaaaagagagaagaagctaggggaattcggcaaggcaaaaggcagcagagccatatggtacatgtggcttggagcacgcttcttagagtttgaagccctaggattcttaaatgaagatcactggttctccagagagaactccctgagtggagtggaaggagaagggctgcacaagctaggttacattctaagagacgtgagcaagaaagagggaggagcaatgtatgccgatgacaccgcaggatgggatacaagaatcacactagaagacctaaaaaatgaagaaatggtaacaaaccacatggaaggagaacacaagaaactagccgaggccattttcaaactaacgtaccaaaacaaggtggtgcgtgtgcaaagaccaacaccaagaggcacagtaatggacatcatatcgagaagagaccaaagaggtagtggacaagttggcacctatggactcaatactttcaccaatatggaagcccaactaatcagacagatggagggagaaggagtctttaaaagcattcagcacctaacaatcacagaagaaatcgctgtgcaaaactggttagcaagagtggggcgcgaaaggttatcaagaatggccatcagtggagatgattgtgttgtgaaacctttagatgacaggttcgcaagcgctttaacagctctaaatgacatgggaaagattaggaaagacatacaacaatgggaaccttcaagaggatggaatgattggacacaagtgcccttctgttcacaccatttccatgagttaatcatgaaagacggtcgcgtactcgttgttccatgtagaaaccaagatgaactgattggcagagcccgaatctcccaaggagcagggtggtctttgcgggagacggcctgtttggggaagtcttacgcccaaatgtggagcttgatgtacttccacagacgcgacctcaggctggcggcaaatgctatttgctcggcagtaccatcacattgggttccaacaagtcgaacaacctggtccatacatgctaaacatgaatggatgacaacggaagacatgctgacagtctggaacagggtgtggattcaagaaaacccatggatggaagacaaaactccagtggaatcatgggaggaaatcccatacttggggaaaagagaagaccaatggtgcggctcattgattgggttaacaagcagggccacctgggcaaagaacatccaagcagcaataaatcaagttagatcccttataggcaatgaagaatacacagattacatgccatccatgaaaagattcagaagagaagaggaagaagcaggagttctgtggtagaaagcaaaactaacatgaaacaaggctagaagtcaggtcggattaagccatagtacggaaaaaactatgctacctgtgagccccgtccaaggacgttaaaagaagtcaggccatcataaatgccatagcttgagtaaactatgcagcctgtagctccacctgagaaggtgtaaaaaatccgggaggccacaaaccatggaagctgtacgcatggcgtagtggactagcggttagaggagacccctcccttacaaatcgcagcaacaatgggggcccaaggcgagatgaagctgtagtctcgctggaaggactagaggttagaggagacccccccgaaacaaaaaacagcatattgacgctgggaaagaccagagatcctgctgtctcctcagcatcattccaggcacagaacgccagaaaatggaatggtgctgttgaatcaacaggttct

SEQ ID NO: 4 - protein, 3406 aa, Artificial Sequence
  Synthetic polypeptide
MNNQRKKAKNTPFNMLKRERNRVSTVQQLTKRFSLGMLQGRGPLKLFMALVAFLRFLTIPPTAGILKRWGTIKKSKAINVLRGFRKEIGRMLNILNRRRRSAGMIVGIVGLLLTTAMAAEVTRRGSAYYMYLDRNDAGEAISFPTTLGMNKCYIQIMDLGHMCDATMSYECPMLDEGVEPDDVDCWCNTTSTWVVYGTCHHKKGEARRSRRAVTLPSHSTRKLQTRSQTWLESREYTKHLIRVENWIFRNPGFALAAAAIAWLLGSSTSQKVIYLVMILLIAPAYSIRCIGVSNRDFVEGMSGGTWVDIVLEHGGCVTVMAQDKPTVDIELVTTTVSNMAEVRSYCYEASISDMASDSRCPTQGEAYLDKQSDTQYVCKRTLVDRGWGNGCGLFGKGSLVTCAKFACSKKMTGKSIQPENLEYRIMLSVHGSQHSGMIVNDTGHETDENRAKVEITPNSPRAEATLGGFGSLGLDCAPRTGLDFSDLYYLTMNNKHWLVHKEWFHDIPLPWHAGADTGTPHWNNKEALVEFKDAHAKRQTVVVLGSQEGAVHTALAGALEAEMDGAKGRLSSGHLKCRLKMDKLRLKGVSYSLCTAAFTFTKIPAETLHGTVTVEVQYAGTDGPCKVPAQMAVDMQTLTPVGRLITANPVITESTENSKMMLELDPPFGDSYIVIGVGEKKITHHWHRSGSTIGKAFEATVRGAKRMAVLGDTAWDFGSVGGALNSLGKGIHQIFGAAFKSLFGGMSWFSQILIGTLLMWLGLNTKNGSISLMCLAAGIVTLYLGVMVQADSGCVVSWKNKELKCGSGIFITDNVHTWTEQYKFQPESPSKLASAIQKAHEEDICGIRSVTRLENLMWKQITPELNHILSENEVKLTIMTGDIKGIMQAGKRSLRPQPTELKYSWKTWGKAKMLSTESHNQTFLIDGPETAECPNTNRAWNSLEVEDYGFGVFTTNIWLKLKEKQDVFCDSKLMSAAIKDNRAVHADMGYWIESALNDTWKIEKASFIEVKNCHWPKSHTLWSNGVLESEMIIPKNLAGPVSQHNYRPGYHTQITGPWHLGKLEMDFDFCDGTTVVVTEDCGNRGPSLRTTTASGKLITEWCCRSCTLPPLRYRGEDGCWYGMEIRPLKEKEENLVNSLVTAGHGQVDNFSLGVLGMALFLEEVLRTRVGTKHAILLVAVSFVTLITGNMSFRDLGRVMVMVGATMTDDIGMGVTYLALLAAFKVRPTFAAGLLLRKLTSKELMMTTIGIVLLSQSTIPETILELTDALALGMMVLKMVRNMEKYQLAVTIMAILCVPNAVILQNAWKVSCTILAVVSVSPLFLTSSQQKTDWIPLALTIKGLNPTAIFLTTLSRTSKKRSWPLNEAIMAVGMVSILASSLLKNDIPMTGPLVAGGLLTVCYVLTGRSADLELERAADVKWEDQAEISGSSPILSITISEDGSMSIKNEEEEQTLTILIRTGLLVISGLFPVSIPITAAAWYLWEVKKQRAGVLWDVPSPPPMGKAELEDGAYRIKQKGILGYSQIGAGVYKEGTFHTMWHVTRGAVLMHKGKRIEPSWADVKKDLISYGGGWKLEGEWKEGEEVQVLALEPGKNPRAVQTKPGLFKTNAGTIGAVSLDFSPGTSGSPIIDKKGKVVGLYGNGVVTRSGAYVSAIAQTEKSIEDNPEIEDDIFRKRRLTIMDLHPGAGKTKRYLPAIVREAIKRGLRTLILAPTRVVAAEMEEALRGLPIRYQTPAIRAVHTGREIVDLMCHATFTMRLLSPVRVPNYNLIIMDEAHFTDPASIAARGYISTRVEMGEAAGIFMTATPPGSRDPFPQSNAPIIDEEREIPERSWNSGHEWVTDFKGKTVWFVPSIKAGNDIAACLRKNGKKVIQLSRKTFDSEYVKTRTNDWDFVVTTDISEMGANFKAERVIDPRRCMKPVILTDGEERVILAGPMPVTHSSAAQRRGRIGRNPKNENDQYIYMGEPLENDEDCAHWKEAKMLLDNINTPEGIIPSMFEPEREKVDAIDGEYRLRGEARKTFVDLMRRGDLPVWLAYRVAAEGINYADRRWCFDGVKNNQILEENVEVEIWTKEGERKKLKPRWLDARIYSDPLALKEFKEFAAGRKSLTLNLITEMGRLPTFMTQKARDALDNLAVLHTAEAGGRAYNHALSELPETLETLLLLTLLATVTGGIFLFLMSARGIGKMTLGMCCIITASILLWYAQIQPHWIAASIILEFFLIVLLIPEPEKQRTPQDNQLTYVVIAILTVVAATMANEMGFLEKTKKDLGLGSIATQQPESNILDIDLRPASAWTLYAVATTFVTPMLRHSIENSSVNVSLTAIANQATVLMGLGKGWPLSKMDIGVPLLAIGCYSQVNPITLTAALFLLVAHYAIIGPGLQAKATREAQKRAAAGIMKNPTVDGITVIDLDPIPYDPKFEKQLGQVMLLVLCVTQVLMMRTTWALCEALTLATGPISTLWEGNPGRFWNTTIAVSMANIFRGSYLAGAGLLFSIMKNTTNTRRGTGNIGETLGEKWKSRLNALGKSEFQIYKKSGIQEVDRTLAKEGIKRGETDHHAVSRGSAKLRWFVERNMVTPEGKVVDLGCGRGGWSYYCGGLKNVREVKGLTKGGPGHEEPIPMSTYGWNLVRLQSGVDVFFIPPEKCDTLLCDIGESSPNPTVEAGRTLRVLNLVENWLNNNTQFCIKVLNPYMPSVIEKMEALQRKYGGALVRNPLSRNSTHEMYWVSNASGNIVSSVNMISRMLINRFTMRYKKATYEPDVDLGSGTRNIGIESEIPNLDIIGKRIEKIKQEHETSWHYDQDHPYKTWAYHGSYETKQTGSASSMVNGVVRLLTKPWDVVPMVTQMAMTDTTPFGQQRVFKEKVDTRTQEPKEGTKKLMKITAEWLWKELGKKKTPRMCTREEFTRKVRSNAALGAIFTDENKWKSAREAVEDSRFWELVDKERNLHLEGKCETCVYNMMGKREKKLGEFGKAKGSRAIWYMWLGARFLEFEALGFLNEDHWFSRENSLSGVEGEGLHKLGYILRDVSKKEGGAMYADDTAGWDTRITLEDLKNEEMVTNHMEGEHKKLAEAIFKLTYQNKVVRVQRPTPRGTVMDIISRRDQRGSGQVGTYGLNTFTNMEAQLIRQMEGEGVFKSIQHLTITEEIAVQNWLARVGRERLSRMAISGDDCVVKPLDDRFASALTALNDMGKIRKDIQQWEPSRGWNDWTQVPFCSHHFHELIMKDGRVLVVPCRNQDELIGRARISQGAGWSLRETACLGKSYAQMWSLMYFHRRDLRLAANAICSAVPSHWVPTSRTTWSIHAKHEWMTTEDMLTVWNRVWIQENPWMEDKTPVESWEEIPYLGKREDQWCGSLIGLTSRATWAKNIQAAINQVRSLIGNEEYTDYMPSMKRFRREEEEAGVLW

SEQ ID NO: 5 - DNA, 10768 bp, Artificial Sequence
  Synthetic construct
agttgttagtctacgtggaccgacaaagacagattctttgagggagctaagctcaatgtagttctaacagttttttaattagagagcagatctctgatgaataaccaacggaaaaaggcgaaaaacacgcctttcaatatgctgaaacgcgagagaaaccgcgtgtcgactgtgcaacagctgacaaagagattctcacttggaatgctgcagggacgaggaccattaaaactgttcatggccctggtggcgttccttcgtttcctaacaatcccaccaacagcagggatattgaagagatggggaacaattaaaaaatcaaaagctattaatgttttgagagggttcaggaaagagattggaaggatgctgaacatcttgaataggagacgcagatccgcgggtactagtgtcggaattgttggcctcctgctgaccacagctatggcagcggaggtcactagacgtgggagtgcatactatatgtacttggacagaaacgatgctggggaggccatatcttttccaaccacattggggatgaataagtgttatatacagatcatggatcttggacacatgtgtgatgccaccatgagctatgaatgccctatgctggatgagggggtggaaccagatgacgtcgattgttggtgcaacacgacgtcaacttgggttgtgtacggaacctgccatcacaaaaaaggtgaagcacggagaagtagaagagctgtgacgctcccctcccattccactaggaagctgcaaacgcggtcgcaaacctggttggaatcaagagaatacacaaagcacttgattagagtcgaaaattggatattcaggaaccctggcttcgcgttagcagcagctgccatcgcttggcttttgggaagctcaacgagccaaaaagtcatatacttggtcatgatactgctgattgccccggcatacagcatcaggtgcataggagtcagcaatagggactttgtggaaggtatgtcaggtgggacttgggttgatattgtcttggaacatggaggttgtgtcaccgtaatggcacaggacaaaccgactgtcgacatagagctggttacaacaacagtcagcaacatggcggaggtaagatcctactgctatgaggcatcaatatcagacatggcttcggacagccgctgcccaacacaaggtgaagcctaccttgacaagcaatcagacactcaatatgtctgcaaaagaacgttagtggacagaggctggggaaatggatgtggactttttggcaaagggagtctggtgacatgcgctaagtttgcatgctccaagaaaatgaccgggaagagcatccagccagagaatctggagtaccggataatgctgtcagttcatggctcccagcacagtgggatgatcgttaatgacacaggacatgaaactgatgagaatagagcgaaggttgagataacgcccaattcaccaagagccgaagccaccctggggggttttggaagcctaggacttgattgtgaaccgaggacaggccttgacttttcagatttgtattacttgactatgaataacaagcactggttggttcacaaggagtggttccacgacattccattaccttggcacgctggggcagacaccggaactccacactggaacaacaaagaagcactggtagagttcaaggacgcacatgccaaaaggcaaactgtcgtggttctagggagtcaagaaggagcagttcacacggcccttgctggagctctggaggctgagatggatggtgcaaagggaaggctgtcctctggccacttgaaatgtcgcctgaaaatggataaacttagattgaagggcgtgtcatactccttgtgtaccgcagcgttcacattcaccaagatcccggctgaaacactgcacgggacagtcacagtggaggtacagtacgcagggacagatggaccttgcaaggttccagctcagatggcggtggacatgcaaactctgaccccagttgggaggttgataaccgctaaccccgtaatcactgaaagcactgagaactctaagatgatgctggaacttgatccaccatttggggactcttacattgtcataggagtcggggagaagaagatcacccaccactggcacaggagtggcagcaccattggaaaagcatttgaagccactgtgagaggtgccaagagaatggcagtcttgggagacacagcctgggactttggatcagttggaggcgctctcaactcattgggcaagggcatccatcaaatttttggagcagctttcaaatcattgtttggaggaatgtcctggttctcacaaattctcattggaacgttgctgatgtggttgggtctgaacacaaagaatggatctatttcccttatgtgcttggccgccggcattgtgacactgtatttgggagtcatggtgcaggccgatagtggttgcgttgtgagctggaaaaacaaagaactgaaatgtggcagtgggattttcatcacagacaacgtgcacacatggacagaacaatacaagttccaaccagaatccccttcaaaactagcttcagctatccagaaagcccatgaagaggacatttgtggaatccgctcagtaacaagactggagaatctgatgtggaaacaaataacaccagaattgaatcacattctatcagaaaatgaggtgaagttaactattatgacaggagacatcaaaggaatcatgcaggcaggaaaacgatctctgcggcctcagcccactgagctgaagtattcatggaaaacatggggcaaagcaaaaatgctctctacagagtctcataaccagacctttctcattgatggccccgaaacagcagaatgccccaacacaaatagagcttggaattcgttggaagttgaagactatggctttggagtattcaccaccaatatatggctaaaattgaaagaaaaacaggatgtattctgcgactcaaaactcatgtcagcggccataaaagacaacagagccgtccatgccgatatgggttattggatagaaagtgcactcaatgacacatggaagatagagaaagcctctttcattgaagttaaaaactgccactggccaaaatcacacaccctctggagcaatggagtgctagaaagtgagatgataattccaaagaatctcgctggaccagtgtctcaacacaactatagaccaggctaccatacacaaataacaggaccatggcatctaggtaagcttgagatggactttgatttctgtgatggaacaacagtggtagtgactgaggactgcggaaatagaggaccctctttgagaacaaccactgcctctggaaaactcataacagaatggtgctgccgatcttgcacattaccaccgctaagatacagaggtgaggatgggtgctggtacgggatggaaatcagaccattgaaggagaaagaagagaatttggtcaactccttggtcacagctggacatgggcaggtcgacaacttttcactaggagtcttgggaatggcattgttcctggaggaagtgcttaggacccgagtaggaacgaaacatgcaatactactagttgcagtttcttttgtgacattgatcacagggaacatgtcctttagagacctgggaagagtgatggttatggtaggcgccactatgacggatgacataggtatgggcgtgacttatcttgccctactagcagccttcaaagtcagaccaacttttgcagctggactactcttgagaaagctgacctccaaggaattgatgatgactactataggaattgtactcctctcccagagcaccataccagagaccattcttgagttgactgatgcgttagccttaggcatgatggtcctcaaaatggtgagaaatatggaaaagtatcaattggcagtgactatcatggctatcttgtgcgtcccaaacgcagtgatattacaaaacgcatggaaagtgagttgcacaatattggcagtggtgtccgtttccccactgttcttaacatcctcacagcaaaaaacagattggataccattagcattgacgatcaaaggtctcaatccaacagctatttttctaacaaccctctcaagaaccagcaagaaaaggagctggccattaaatgaggctatcatggcagtcgggatggtgagcattttagccagttctctcctaaaaaatgatattcccatgacaggaccattagtggctggagggctcctcactgtgtgctacgtgctcactggacgatcggccgatttggaactggagagagcagccgatgtcaaatgggaagaccaggcagagatatcaggaagcagtccaatcctgtcaataacaatatcagaagatggtagcatgtcgataaaaaatgaagaggaagaacaaacactgaccatactcattagaacaggattgctggtgatctcaggactttttcctgtatcaataccaatcacggcagcagcatggtacctgtgggaagtgaagaaacaacgggccggagtattgtgggatgttccttcacccccacccatgggaaaggctgaactggaagatggagcctatagaattaagcaaaaagggattcttggatattcccagatcggagccggagtttacaaagaaggaacattccatacaatgtggcatgtcacacgtggcgctgttctaatgcataaaggaaagaggattgaaccatcatgggcggacgtcaagaaagacctaatatcatatggaggaggctggaagttagaaggagaatggaaggaaggagaagaagtccaggtattggcactggagcctggaaaaaatccaagagccgtccaaacgaaacctggtcttttcaaaaccaacgccggaacaataggtgctgtatctctggacttttctcctggaacgtcaggatctccaattatcgacaaaaaaggaaaagttgtgggtctttatggtaatggtgttgttacaaggagtggagcatatgtgagtgctatagcccagactgaaaaaagcattgaagacaacccagagatcgaagatgacattttccgaaagagaagactgaccatcatggacctccacccaggagcgggaaagacgaagagataccttccggccatagtcagagaagctataaaacggggtttgagaacattaatcttggcccccactagagttgtggcagctgaaatggaggaagcccttagaggacttccaataagataccagaccccagccatcagagctgtgcacaccgggcgggagattgtggacctaatgtgtcatgccacatttaccatgaggctgctatcaccagttagagtgccaaactacaacctgattatcatggacgaagcccatttcacagacccagcaagtatagcagctagaggatacatctcaactcgagtggagatgggtgaggcagctgggatttttatgacagccactcccccgggaagcagagacccatttcctcagagcaatgcaccaatcatagatgaagaaagagaaatccctgaacgctcgtggaattccggacatgaatgggtcacggattttaaagggaagactgtttggttcgttccaagtataaaagcaggaaatgatatagcagcttgcctgaggaaaaatggaaagaaagtgatacaactcagtaggaagacctttgattctgagtatgtcaagactagaaccaatgattgggacttcgtggttacaactgacatttcagaaatgggtgccaatttcaaggctgagagggttatagaccccagacgctgcatgaaaccagtcatactaacagatggtgaagagcgggtgattctggcaggacctatgccagtgacccactctagtgcagcacaaagaagagggagaataggaagaaatccaaaaaatgagaatgaccagtacatatacatgggggaacctctggaaaatgatgaagactgtgcacactggaaagaagctaaaatgctcctagataacatcaacacgccagaaggaatcattcctagcatgttcgaaccagagcgtgaaaaggtggatgccattgatggcgaataccgcttgagaggagaagcaaggaaaacctttgtagacttaatgagaagaggagacctaccagtctggttggcctacagagtggcagctgaaggcatcaactacgcagacagaaggtggtgttttgatggagtcaagaacaaccaaatcctagaagaaaacgtggaagttgaaatctggacaaaagaaggggaaaggaagaaattgaaacccagatggttggatgctaggatctattctgacccactggcgctaaaagaatttaaggaatttgcagccggaagaaagtctctgaccctgaacctaatcacagaaatgggtaggctcccaaccttcatgactcagaaggcaagagacgcactggacaacttagcagtgctgcacacggctgaggcaggtggaagggcgtacaaccatgctctcagtgaactgccggagaccctggagacattgcttttactgacacttctggctacagtcacgggagggatctttttattcttgatgagcgcaaggggcatagggaagatgaccctgggaatgtgctgcataatcacggctagcatcctcctatggtacgcacaaatacagccacactggatagcagcttcaataatactggagttttttctcatagttttgcttattccagaacctgaaaaacagagaacaccccaagacaaccaactgacctacgttgtcatagccatcctcacagtggtggccgcaaccatggcaaacgagatgggtttcctagaaaaaacgaagaaagatctcggattgggaagcattgcaacccagcaacccgagagcaacatcctggacatagatctacgtcctgcatcagcatggacgctgtatgccgtggccacaacatttgttacaccaatgttgagacatagcattgaaaattcctcagtgaatgtgtccctaacagctatagccaaccaagccacagtgttaatgggtctcgggaaaggatggccattgtcaaagatggacatcggagttccccttctcgccattggatgctactcacaagtcaaccccataactctcacagcagctcttttcttattggtagcacattatgccatcatagggccaggactccaagcaaaagcaaccagagaagctcagaaaagagcagcggcgggcatcatgaaaaacccaactgtcgatggaataacagtgattgacctagatccaataccttatgatccaaagtttgaaaagcagttgggacaagtaatgctcctagtcctctgcgtgactcaagtattgatgatgaggactacatgggctctgtgtgaggctttaaccttagctaccgggcccatctccacattgtgggaaggaaatccagggaggttttggaacactaccattgcggtgtcaatggctaacatttttagagggagttacttggccggagctggacttctcttttctattatgaagaacacaaccaacacaagaaggggaactggcaacataggagagacgcttggagagaaatggaaaagccgattgaacgcattgggaaaaagtgaattccagatctacaagaaaagtggaatccaggaagtggatagaaccttagcaaaagaaggcattaaaagaggagaaacggaccatcacgctgtgtcgcgaggctcagcaaaactgagatggttcgttgagagaaacatggtcacaccagaagggaaagtagtggacctcggttgtggcagaggaggctggtcatactattgtggaggactaaagaatgtaagagaagtcaaaggcctaacaaaaggaggaccaggacacgaagaacccatccccatgtcaacatatgggtggaatctagtgcgtcttcaaagtggagttgacgttttcttcatcccgccagaaaagtgtgacacattattgtgtgacataggggagtcatcaccaaatcccacagtggaagcaggacgaacactcagagtccttaacttagtagaaaattggttgaacaacaacactcaattttgcataaaggttctcaacccatatatgccctcagtcatagaaaaaatggaagcactacaaaggaaatatggaggagccttagtgaggaatccactctcacgaaactccacacatgagatgtactgggtatccaatgcttccgggaacatagtgtcatcagtgaacatgatttcaaggatgttgatcaacagatttacaatgagatacaagaaagccacttacgagccggatgttgacctcggaagcggaacccgtaacatcgggattgaaagtgagataccaaacctagatataattgggaaaagaatagaaaaaataaagcaagagcatgaaacatcatggcactatgaccaagaccacccatacaaaacgtgggcataccatggtagctatgaaacaaaacagactggatcagcatcatccatggtcaacggagtggtcaggctgctgacaaaaccttgggacgtcgtccccatggtgacacagatggcaatgacagacacgactccatttggacaacagcgcgtttttaaagagaaagtggacacgagaacccaagaaccgaaagaaggcacgaagaaactaatgaaaataacagcagagtggctttggaaagaattagggaagaaaaagacacccaggatgtgcaccagagaagaattcacaagaaaggtgagaagcaatgcagccttgggggccatattcactgatgagaacaagtggaagtcggcacgtgaggctgttgaagatagtaggttttgggagctggttgacaaggaaaggaatctccatcttgaaggaaagtgtgaaacatgtgtgtacaacatgatgggaaaaagagagaagaagctaggggaattcggcaaggcaaaaggcagcagagccatatggtacatgtggcttggagcacgcttcttagagtttgaagccctaggattcttaaatgaagatcactggttctccagagagaactccctgagtggagtggaaggagaagggctgcacaagctaggttacattctaagagacgtgagcaagaaagagggaggagcaatgtatgccgatgacaccgcaggatgggatacaagaatcacactagaagacctaaaaaatgaagaaatggtaacaaaccacatggaaggagaacacaagaaactagccgaggccattttcaaactaacgtaccaaaacaaggtggtgcgtgtgcaaagaccaacaccaagaggcacagtaatggacatcatatcgagaagagaccaaagaggtagtggacaagttggcacctatggactcaatactttcaccaatatggaagcccaactaatcagacagatggagggagaaggagtctttaaaagcattcagcacctaacaatcacagaagaaatcgctgtgcaaaactggttagcaagagtggggcgcgaaaggttatcaagaatggccatcagtggagatgattgtgttgtgaaacctttagatgacaggttcgcaagcgctttaacagctctaaatgacatgggaaagattaggaaagacatacaacaatgggaaccttcaagaggatggaatgattggacacaagtgcccttctgttcacaccatttccatgagttaatcatgaaagacggtcgcgtactcgttgttccatgtagaaaccaagatgaactgattggcagagcccgaatctcccaaggagcagggtggtctttgcgggagacggcctgtttggggaagtcttacgcccaaatgtggagcttgatgtacttccacagacgcgacctcaggctggcggcaaatgctatttgctcggcagtaccatcacattgggttccaacaagtcgaacaacctggtccatacatgctaaacatgaatggatgacaacggaagacatgctgacagtctggaacagggtgtggattcaagaaaacccatggatggaagacaaaactccagtggaatcatgggaggaaatcccatacttggggaaaagagaagaccaatggtgcggctcattgattgggttaacaagcagggccacctgggcaaagaacatccaagcagcaataaatcaagttagatcccttataggcaatgaagaatacacagattacatgccatccatgaaaagattcagaagagaagaggaagaagcaggagttctgtggtagaaagcaaaactaacatgaaacaaggctagaagtcaggtcggattaagccatagtacggaaaaaactatgctacctgtgagccccgtccaaggacgttaaaagaagtcaggccatcataaatgccatagcttgagtaaactatgcagcctgtagctccacctgagaaggtgtaaaaaatccgggaggccacaaaccatggaagctgtacgcatggcgtagtggactagcggttagaggagacccctcccttacaaatcgcagcaacaatgggggcccaaggcgagatgaagctgtagtctcgctggaaggactagaggttagaggagacccccccgaaacaaaaaacagcatattgacgctgggaaagaccagagatcctgctgtctcctcagcatcattccaggcacagaacgccagaaaatggaatggtgctgttgaatcaacaggttct

SEQ ID NO: 6 - protein, 3406 aa, Artificial Sequence
  Synthetic polypeptide
MNNQRKKAKNTPFNMLKRERNRVSTVQQLTKRFSLGMLQGRGPLKLFMALVAFLRFLTIPPTAGILKRWGTIKKSKAINVLRGFRKEIGRMLNILNRRRRSAGTSVGIVGLLLTTAMAAEVTRRGSAYYMYLDRNDAGEAISFPTTLGMNKCYIQIMDLGHMCDATMSYECPMLDEGVEPDDVDCWCNTTSTWVVYGTCHHKKGEARRSRRAVTLPSHSTRKLQTRSQTWLESREYTKHLIRVENWIFRNPGFALAAAAIAWLLGSSTSQKVIYLVMILLIAPAYSIRCIGVSNRDFVEGMSGGTWVDIVLEHGGCVTVMAQDKPTVDIELVTTTVSNMAEVRSYCYEASISDMASDSRCPTQGEAYLDKQSDTQYVCKRTLVDRGWGNGCGLFGKGSLVTCAKFACSKKMTGKSIQPENLEYRIMLSVHGSQHSGMIVNDTGHETDENRAKVEITPNSPRAEATLGGFGSLGLDCEPRTGLDFSDLYYLTMNNKHWLVHKEWFHDIPLPWHAGADTGTPHWNNKEALVEFKDAHAKRQTVVVLGSQEGAVHTALAGALEAEMDGAKGRLSSGHLKCRLKMDKLRLKGVSYSLCTAAFTFTKIPAETLHGTVTVEVQYAGTDGPCKVPAQMAVDMQTLTPVGRLITANPVITESTENSKMMLELDPPFGDSYIVIGVGEKKITHHWHRSGSTIGKAFEATVRGAKRMAVLGDTAWDFGSVGGALNSLGKGIHQIFGAAFKSLFGGMSWFSQILIGTLLMWLGLNTKNGSISLMCLAAGIVTLYLGVMVQADSGCVVSWKNKELKCGSGIFITDNVHTWTEQYKFQPESPSKLASAIQKAHEEDICGIRSVTRLENLMWKQITPELNHILSENEVKLTIMTGDIKGIMQAGKRSLRPQPTELKYSWKTWGKAKMLSTESHNQTFLIDGPETAECPNTNRAWNSLEVEDYGFGVFTTNIWLKLKEKQDVFCDSKLMSAAIKDNRAVHADMGYWIESALNDTWKIEKASFIEVKNCHWPKSHTLWSNGVLESEMIIPKNLAGPVSQHNYRPGYHTQITGPWHLGKLEMDFDFCDGTTVVVTEDCGNRGPSLRTTTASGKLITEWCCRSCTLPPLRYRGEDGCWYGMEIRPLKEKEENLVNSLVTAGHGQVDNFSLGVLGMALFLEEVLRTRVGTKHAILLVAVSFVTLITGNMSFRDLGRVMVMVGATMTDDIGMGVTYLALLAAFKVRPTFAAGLLLRKLTSKELMMTTIGIVLLSQSTIPETILELTDALALGMMVLKMVRNMEKYQLAVTIMAILCVPNAVILQNAWKVSCTILAVVSVSPLFLTSSQQKTDWIPLALTIKGLNPTAIFLTTLSRTSKKRSWPLNEAIMAVGMVSILASSLLKNDIPMTGPLVAGGLLTVCYVLTGRSADLELERAADVKWEDQAEISGSSPILSITISEDGSMSIKNEEEEQTLTILIRTGLLVISGLFPVSIPITAAAWYLWEVKKQRAGVLWDVPSPPPMGKAELEDGAYRIKQKGILGYSQIGAGVYKEGTFHTMWHVTRGAVLMHKGKRIEPSWADVKKDLISYGGGWKLEGEWKEGEEVQVLALEPGKNPRAVQTKPGLFKTNAGTIGAVSLDFSPGTSGSPIIDKKGKVVGLYGNGVVTRSGAYVSAIAQTEKSIEDNPEIEDDIFRKRRLTIMDLHPGAGKTKRYLPAIVREAIKRGLRTLILAPTRVVAAEMEEALRGLPIRYQTPAIRAVHTGREIVDLMCHATFTMRLLSPVRVPNYNLIIMDEAHFTDPASIAARGYISTRVEMGEAAGIFMTATPPGSRDPFPQSNAPIIDEEREIPERSWNSGHEWVTDFKGKTVWFVPSIKAGNDIAACLRKNGKKVIQLSRKTFDSEYVKTRTNDWDFVVTTDISEMGANFKAERVIDPRRCMKPVILTDGEERVILAGPMPVTHSSAAQRRGRIGRNPKNENDQYIYMGEPLENDEDCAHWKEAKMLLDNINTPEGIIPSMFEPEREKVDAIDGEYRLRGEARKTFVDLMRRGDLPVWLAYRVAAEGINYADRRWCFDGVKNNQILEENVEVEIWTKEGERKKLKPRWLDARIYSDPLALKEFKEFAAGRKSLTLNLITEMGRLPTFMTQKARDALDNLAVLHTAEAGGRAYNHALSELPETLETLLLLTLLATVTGGIFLFLMSARGIGKMTLGMCCIITASILLWYAQIQPHWIAASIILEFFLIVLLIPEPEKQRTPQDNQLTYVVIAILTVVAATMANEMGFLEKTKKDLGLGSIATQQPESNILDIDLRPASAWTLYAVATTFVTPMLRHSIENSSVNVSLTAIANQATVLMGLGKGWPLSKMDIGVPLLAIGCYSQVNPITLTAALFLLVAHYAIIGPGLQAKATREAQKRAAAGIMKNPTVDGITVIDLDPIPYDPKFEKQLGQVMLLVLCVTQVLMMRTTWALCEALTLATGPISTLWEGNPGRFWNTTIAVSMANIFRGSYLAGAGLLFSIMKNTTNTRRGTGNIGETLGEKWKSRLNALGKSEFQIYKKSGIQEVDRTLAKEGIKRGETDHHAVSRGSAKLRWFVERNMVTPEGKVVDLGCGRGGWSYYCGGLKNVREVKGLTKGGPGHEEPIPMSTYGWNLVRLQSGVDVFFIPPEKCDTLLCDIGESSPNPTVEAGRTLRVLNLVENWLNNNTQFCIKVLNPYMPSVIEKMEALQRKYGGALVRNPLSRNSTHEMYWVSNASGNIVSSVNMISRMLINRFTMRYKKATYEPDVDLGSGTRNIGIESEIPNLDIIGKRIEKIKQEHETSWHYDQDHPYKTWAYHGSYETKQTGSASSMVNGVVRLLTKPWDVVPMVTQMAMTDTTPFGQQRVFKEKVDTRTQEPKEGTKKLMKITAEWLWKELGKKKTPRMCTREEFTRKVRSNAALGAIFTDENKWKSAREAVEDSRFWELVDKERNLHLEGKCETCVYNMMGKREKKLGEFGKAKGSRAIWYMWLGARFLEFEALGFLNEDHWFSRENSLSGVEGEGLHKLGYILRDVSKKEGGAMYADDTAGWDTRITLEDLKNEEMVTNHMEGEHKKLAEAIFKLTYQNKVVRVQRPTPRGTVMDIISRRDQRGSGQVGTYGLNTFTNMEAQLIRQMEGEGVFKSIQHLTITEEIAVQNWLARVGRERLSRMAISGDDCVVKPLDDRFASALTALNDMGKIRKDIQQWEPSRGWNDWTQVPFCSHHFHELIMKDGRVLVVPCRNQDELIGRARISQGAGWSLRETACLGKSYAQMWSLMYFHRRDLRLAANAICSAVPSHWVPTSRTTWSIHAKHEWMTTEDMLTVWNRVWIQENPWMEDKTPVESWEEIPYLGKREDQWCGSLIGLTSRATWAKNIQAAINQVRSLIGNEEYTDYMPSMKRFRREEEEAGVLW

SEQ ID NO: 7 - DNA, 10807 bp, Zika virus strain R103451
agttgttgatctgtgtgaatcagactgcgacagttcgagtttgaagcgaaagctagcaacagtatcaacaggttttattttggatttggaaacgagagtttctggtcatgaaaaacccaaaaaagaaatccggaggattccggattgtcaatatgctaaaacgcggagtagcccgtgtgagcccctttgggggcttgaagaggctgccagccggacttctgctgggtcatgggcccatcaggatggtcttggcgattctagcctttttgagattcacggcaatcaagccatcactgggtctcatcaatagatggggttcagtggggaaaaaagaggctatggaaataataaagaagttcaagaaagatctggctgccatgctgagaataatcaatgctaggaaggagaagaagagacgaggcgcagatactagtgtcggaattgttggcctcctgctgaccacagctatggcagcggaggtcactagacgtgggagtgcatactatatgtacttggacagaaacgatgctggggaggccatatcttttccaaccacattggggatgaataagtgttatatacagatcatggatcttggacacatgtgtgatgccaccatgagctatgaatgccctatgctggatgagggggtggaaccagatgacgtcgattgttggtgcaacacgacgtcaacttgggttgtgtacggaacctgccatcacaaaaaaggtgaagcacggagatctagaagagctgtgacgctcccctcccattccactaggaagctgcaaacgcggtcgcaaacctggttggaatcaagagaatacacaaagcacttgattagagtcgaaaattggatattcaggaaccctggcttcgcgttagcagcagctgccatcgcttggcttttgggaagctcaacgagccaaaaagtcatatacttggtcatgatactgctgattgccccggcatacagcatcaggtgcataggagtcagcaatagggactttgtggaaggtatgtcaggtgggacttgggttgatgttgtcttggaacatggaggttgtgtcaccgtaatggcacaggacaaaccgactgtcgacatagagctggttacaacaacagtcagcaacatggcggaggtaagatcctactgctatgaggcatcaatatcagacatggcttcggacagccgctgcccaacacaaggtgaagcctaccttgacaagcaatcagacactcaatatgtctgcaaaagaacgttagtggacagaggctggggaaatggatgtggactttttggcaaagggagcctggtgacatgcgctaagtttgcatgctccaagaaaatgaccgggaagagcatccagccagagaatctggagtaccggataatgctgtcagttcatggctcccagcacagtgggatgatcgttaatgacacaggacatgaaactgatgagaatagagcgaaggttgagataacgcccaattcaccaagagccgaagccaccctggggggttttggaagcctaggacttgattgtgaaccgaggacaggccttgacttttcagatttgtattacttgactatgaataacaagcactggttggttcacaaggagtggttccacgacattccattaccttggcacgctggggcagacaccggaactccacactggaacaacaaagaagcactggtagagttcaaggacgcacatgccaaaaggcaaactgtcgtggttctagggagtcaagaaggagcagttcacacggcccttgctggagctctggaggctgagatggatggtgcaaagggaaggctgtcctctggccacttgaaatgtcgcctgaaaatggataaacttagattgaagggcgtgtcatactccttgtgtaccgcagcgttcacattcaccaagatcccggctgaaacactgcacgggacagtcacagtggaggtacagtacgcagggacagatggaccttgcaaggttccagctcagatggcggtggacatgcaaactctgaccccagttgggaggttgataaccgctaaccccgtaatcactgaaagcactgagaactctaagatgatgctggaacttgatccaccatttggggactcttacattgtcataggagtcggggagaagaagatcacccaccactggcacaggagtggcagcaccattggaaaagcatttgaagccactgtgagaggtgccaagagaatggcagtcttgggagacacagcctgggactttggatcagttggaggcgctctcaactcattgggcaagggcatccatcaaatttttggagcagctttcaaatcattgtttggaggaatgtcctggttctcacaaattctcattggaacgttgctgatgtggttgggtctgaacacaaagaatggatctatttcccttatgtgcttggccttagggggagtgttgatcttcttatccacagccgtctctgctgatgtggggtgctcggtggacttctcaaagaaggagacgagatgcggtacaggggtgttcgtctataacgacgttgaagcctggagggacaggtacaagtaccatcctgactccccccgtagattggcagcagcagtcaagcaagcctgggaagatggtatctgcgggatctcctctgtttcaagaatggaaaacatcatgtggagatcagtagaaggggagctcaacgcaatcctggaagagaatggagttcaactgacggtcgttgtgggatctgtaaaaaaccccatgtggagagctccacagagattgcccgtgcctgtgaacgagctgccccacggctggaaggcttgggggaaatcgtacttcgtcagagcagcaaagacaaataacagctttgtcgtggatggtgacacactgaaggaatgcccactcaaacatagagcatggaacagctttcttgtggaggatcatgggttcggggtatttcacactagtgtctggctcaaggttagagaagattattcattagagtgtgatccagccgttattggaacagctgttaagggaaaggaggctgtacacagtgatctaggctactggattgagagtgagaagaatgacacatggaggctgaagagggcccatctgatcgagatgaaaacatgtgaatggccaaagtcccacacattgtggacagatggaatagaagagagtgatctgatcatacccaagtctttagctgggccactcagccatcacaataccagagagggctacaggacccaaatgaaagggccatggcacagtgaagagcttgaaattcggtttgaggaatgcccaggcactaaggtccacgtggaggaaacatgtggaacaagaggaccatctctgagatcaaccactgcaagcggaagggtgatcgaggaatggtgctgcagggagtgcacaatgcccccactgtcgttccgggctaaagatggctgttggtatggaatggagataaggcccaggaaagaaccagaaagcaacttagtaaggtcaatggtgactgcaggatcaactgatcacatggatcacttctcccttggagtgcttgtgattctgctcatggtgcaggaagggctaaagaagagaatgaccacaaagatcatcataagcacatcaatggcagtgctggtagctatgatcctgggaggattttcaatgagtgacctggctaagcttgcaattttgatgggtgccaccttcgcggaaatgaacactggaggagatgtagctcatctggcgctgatagcggcattcaaagtcagaccagcgttgctggtatctttcatcttcagagctaattggacaccccgtgaaagcatgctactggccttggcctcgtgtcttttgcaaactgcgatctccgccttggaaggcgacctgatggttctcatcaatggttttgctttggcctggttggcaatacgagcgatggttgttccacgcactgataacatcaccttggcaatcctggctgctctgacaccactggcccggggcacactgcttgtggcgtggagagcaggccttgctacttgcggggggtttatgctcctctctctgaagggaaaaggcagtgtgaagaagaacttaccatttgtcatggccctgggactaaccgctgtgaggctggtcgaccccatcaacgtggtgggactgctgttgctcacaaggagtgggaagcggagctggccccctagcgaagtactcacagctgttggcctgatatgcgcattggctggagggttcgccaaggcagatatagagatggctgggcccatggccgcggtcggtctgctaattgtcagttacgtggtctcaggaaagagtgtggacatgtacattgaaagagcaggtgacatcacatgggaaaaagatgcggaagtcactggaaacagtccccggctcgatgtggcgctagatgagagtggtgatttctccctggtggaggatgacggtccccccatgagagagatcatactcaaggtggtcctgatgaccatctgtggcatgaacccaatagccatacccttcgcagctggagcgtggtacgtatacgtgaagactggaaaaaggagtggtgctctatgggatgtgcctgctcccaaggaagtaaaaaagggggagaccacagatggagtgtacagagtaatgactcgtagactgctaggttcaacacaagttggagtgggagttatgcaagagggggtctttcacactatgtggcacgtcacaaaaggatccgcactgagaagcggtgaagggagacttgatccatactggggagatgtcaagcaggatctggtgtcatactgtggtccatggaagctagatgccgcctgggacgggcacagcgaggtgcagctcttggccgtgccccccggagagagagcgaggaacatccagactctgcccggaatatttaagacaaaggatggggacattggagcggttgcgctggattacccagcaggaacttcaggatctccaatcctagacaagtgtgggagagtgataggactttatggcaatggggtcgtgatcaaaaatgggagttatgttagtgccatcacccaagggaggagggaggaagagactcctgttgagtgcttcgagccttcgatgctgaagaagaagcagctaactgtcttagacttacatcctggagctgggaaaaccaggagagttcttcctgaaatagtccgtgaagccataaaaacaagactccgtactgtgatcttagctccaaccagggttgtcgctgctgaaatggaggaggcccttagagggcttccagtgcgttatatgacaacagcagtcaatgtcacccactctggaacagaaatcgtcgacttaatgtgccatgccaccttcacttcacgtctactacagccaatcagagtccccaactataatctgtatattatggatgaggcccacttcacagatccctcaagtatagcagcaagaggatacatttcaacaagggttgagatgggcgaggcggctgccatcttcatgaccgccacgccaccaggaacccgtgacgcatttccggactccaactcaccaattatggacaccgaagtggaagtcccagagagagcctggagctcaggctttgattgggtgacggatcattctggaaaaacagtttggtttgttccaagcgtgaggaacggcaatgagatcgcagcttgtctgacaaaggctggaaaacgggtcatacagctcagcagaaagacttttgagacagagttccagaaaacaaaacatcaagagtgggactttgtcgtgacaactgacatttcagagatgggcgccaactttaaagctgaccgtgtcatagattccaggagatgcctaaagccggtcatacttgatggcgagagagtcattctggctggacccatgcctgtcacacatgccagcgctgcccagaggagggggcgcataggcaggaatcccaacaaacctggagatgagtatctgtatggaggtgggtgcgcagagactgacgaagaccatgcacactggcttgaagcaagaatgctccttgacaatatttacctccaagatggcctcatagcctcgctctatcgacctgaggccgacaaagtagcagccattgagggagagttcaagcttaggacggagcaaaggaagacctttgtggaactcatgaaaagaggagatcttcctgtttggctggcctatcaggttgcatctgccggaataacctacacagatagaagatggtgctttgatggcacgaccaacaacaccatactggaagacagcgtgccggcagaggtgtggaccagacacggagagaaaagagtgctcaaaccgaggtggatggacgccagagtttgttcagatcatgcggccctgaagtcattcaaggagtttgccgctgggaaaagaggagcggcttttggagtgatggaagccctgggaacactgccaggacacatgacagagagattccaggaagccattgacaacctcgctgtgctcatgcgggcagagactggaagcaggccttacaaagccgcggcggcccaattgccggagaccctagagaccattatgcttttggggttgctgggaacagtctcgctgggaatctttttcgtcttgatgaggaacaagggcatagggaagatgggctttggaatggtgacccttggggccagtgcatggctcatgtggctctcggaaattgagccagccagaattgcatgcgtcctcattgttgtgttcctattgctggtggtgctcatacctgagccagaaaagcaaagatctccccaggacaaccaaatggcaatcatcatcatggtagcagtaggtcttctgggcttgattaccgccaatgaactcggatggttggagagaacaaagagtgacctaagccatctaatgggaaggagagaggagggggcaaccataggattctcaatggacattgacctgcggccagcctcagcttgggccatctatgctgccttgacaactttcattaccccagccgtccaacatgcagtgaccacttcatacaacaactactccttaatggcgatggccacgcaagctggagtgttgtttggtatgggcaaagggatgccattctacgcatgggactttggagtcccgctgctaatgataggttgctactcacaattaacacccctgaccctaatagtggccatcattttgctcgtggcgcactacatgtacttgatcccagggctgcaggcagcagctgcgcgtgctgcccagaagagaacggcagctggcatcatgaagaaccctgttgtggatggaatagtggtgactgacattgacacaatgacaattgacccccaagtggagaaaaagatgggacaggtgctactcatagcagtagccgtctccagcgccatactgtcgcggaccgcctgggggtggggggaggctggggccctgatcacagccgcaacttccactttgtgggaaggctctccgaacaagtactggaactcctctacagccacttcactgtgtaacatttttaggggaagttacttggctggagcctctctaatctacacagtaacaagaaacgctggcttggtcaagagacgtgggggtggaacaggagagaccctgggagagaaatggaaggcccgcttgaaccagatgtcggccctggagttctactcctacaaaaagtcaggcatcaccgaggtgtgcagagaagaggcccgccgcgccctcaaggacggtgtggcaacgggaggccatgctgtgtcccgaggaagtgcaaagctgagatggttggtggagcggggatacctgcagccctatggaaaggtcattgatcttggatgtggcagagggggctggagttactacgccgccaccatccgcaaagttcaagaagtgaaaggatacacaaaaggaggccctggtcatgaagaacccgtgttggtgcaaagctatgggtggaacattgtccgtcttaagagtggggtggacgtctttcatatggcggctgagccgtgtgacacgttgctgtgtgacataggtgagtcatcatctagtcctgaagtggaagaagcacggacgctcagagtcctctccatggtgggggattggcttgaaaaaagaccaggagccttttgtataaaagtgttgtgcccatacaccagcactatgatggaaaccctggagcgactgcagcgtaggtatgggggaggactggtcagagtgccactctcccgcaactctacacatgagatgtactgggtctctggagcgaaaagcaacaccataaaaagtgtgtccaccacgagccagctcctcttggggcgcatggacgggcctaggaggccagtgaaatatgaggaggatgtgaatctcggctctggcacgcgggctgtggtaagctgcgctgaagctcccaacatgaagatcattggtaaccgcattgaaaggatccgcagtgagcacgcggaaacgtggttctttgacgagaaccacccatataggacatgggcttaccatggaagctatgaggcccccacacaagggtcagcgtcctctctaataaacggggttgtcaggctcctgtcaaaaccctgggatgtggtgactggagtcacaggaatagccatgaccgacaccacaccgtatggtcagcaaagagttttcaaggaaaaagtggacactagggtgccagacccccaagaaggcactcgtcaggttatgagcatggtctcttcctggttgtggaaagagctaggcaaacacaaacggccacgagtctgtaccaaagaagagttcatcaacaaggttcgtagcaatgcagcattaggggcaatatttgaagaggaaaaagagtggaagactgcagtggaagctgtgaacgatccaaggttctgggctctagtggacaaggaaagagagcaccacctgagaggagagtgccagagttgtgtgtacaacatgatgggaaaaagagaaaagaaacaaggggaatttggaaaggccaagggcagccgcgccatctggtatatgtggctaggggctagatttctagagttcgaagcccttggattcttgaacgaggatcactggatggggagagagaactcaggaggtggtgttgaagggctgggattacaaagactcggatatgtcctagaagagatgagttgcataccaggaggaaggatgtatgcagatgacactgctggctgggacacccgcatcagcaggtttgatctggagaatgaagctctaatcaccaaccaaatggagaaagggcacagggccttggcattggccataatcaagtacacataccaaaacaaagtggtaaaggtccttagaccagctgaaaaagggaaaacagttatggacattatttcgagacaagaccaaagggggagcggacaagttgtcacttacgctcttaacacatttaccaacctagtggtgcaactcattcggaatatggaggctgaggaagttctagagatgcaagacttgtggctgctgcggaggtcagagaaagtgaccaactggttgcagagcaacggatgggataggctcaaacgaatggcagtcagtggagatgattgcgttgtgaagccaattgatgataggtttgcacatgccctcaggttcttgaatgatatgggaaaagttaggaaggacacacaagagtggaaaccctcaactggatgggacaactgggaagaagttccgttttgctcccaccacttcaacaagctccatctcaaggacgggaggtccattgtggttccctgccgccaccaagatgaactgattggccgggcccgcgtctctccaggggcgggatggagcatccgggagactgcttgcctagcaaaatcatatgcgcaaatgtggcagctcctttatttccacagaagggacctccgactgatggccaatgccatttgttcatctgtgccagttgactgggttccaactgggagaactacctggtcaatccatggaaagggagaatggatgaccactgaagacatgcttgtggtgtggaacagagtgtggattgaggagaacgaccacatggaagacaagaccccagttacgaaatggacagacattccctatttgggaaaaagggaagacttgtggtgtggatctctcatagggcacagaccgcgcaccacctgggctgagaacattaaaaacacagtcaacatggtgcgcaggatcataggtgatgaagaaaagtacatggactacctatccacccaagttcgctacttgggtgaagaagggtctacacctggagtgctgtaagcaccaatcttaacgttgtcaggcctgctagtcagccacagcttggggaaagctgtgcagcctgtgacccccccaggagaagctgggaaaccaagcctatagtcaggccgagaacgccatggcacggaagaagccatgctgcctgtgagcccctcagaggacactgagtcaaaaaaccccacgcgcttggaggcgcaggatgggaaaagaaggtggcgaccttccccacccttcaatctggggcctgaactggagatcagctgtggatctccagaagagggactagtggttagaggagaccccccggaaaacgcaaaacagcatattgacgctgggaaagaccagagactccatgagtttccaccacgctggccgccaggcacagatcgccgaatagcggcggccggtgtggggaaatccatgggtct

SEQ ID NO: 8 - protein, 3423 aa, Zika virus strain R103451
MKNPKKKSGGFRIVNMLKRGVARVSPFGGLKRLPAGLLLGHGPIRMVLAILAFLRFTAIKPSLGLINRWGSVGKKEAMEIIKKFKKDLAAMLRIINARKEKKRRGADTSVGIVGLLLTTAMAAEVTRRGSAYYMYLDRNDAGEAISFPTTLGMNKCYIQIMDLGHMCDATMSYECPMLDEGVEPDDVDCWCNTTSTWVVYGTCHHKKGEARRSRRAVTLPSHSTRKLQTRSQTWLESREYTKHLIRVENWIFRNPGFALAAAAIAWLLGSSTSQKVIYLVMILLIAPAYSIRCIGVSNRDFVEGMSGGTWVDVVLEHGGCVTVMAQDKPTVDIELVTTTVSNMAEVRSYCYEASISDMASDSRCPTQGEAYLDKQSDTQYVCKRTLVDRGWGNGCGLFGKGSLVTCAKFACSKKMTGKSIQPENLEYRIMLSVHGSQHSGMIVNDTGHETDENRAKVEITPNSPRAEATLGGFGSLGLDCEPRTGLDFSDLYYLTMNNKHWLVHKEWFHDIPLPWHAGADTGTPHWNNKEALVEFKDAHAKRQTVVVLGSQEGAVHTALAGALEAEMDGAKGRLSSGHLKCRLKMDKLRLKGVSYSLCTAAFTFTKIPAETLHGTVTVEVQYAGTDGPCKVPAQMAVDMQTLTPVGRLITANPVITESTENSKMMLELDPPFGDSYIVIGVGEKKITHHWHRSGSTIGKAFEATVRGAKRMAVLGDTAWDFGSVGGALNSLGKGIHQIFGAAFKSLFGGMSWFSQILIGTLLMWLGLNTKNGSISLMCLALGGVLIFLSTAVSADVGCSVDFSKKETRCGTGVFVYNDVEAWRDRYKYHPDSPRRLAAAVKQAWEDGICGISSVSRMENIMWRSVEGELNAILEENGVQLTVVVGSVKNPMWRAPQRLPVPVNELPHGWKAWGKSYFVRAAKTNNSFVVDGDTLKECPLKHRAWNSFLVEDHGFGVFHTSVWLKVREDYSLECDPAVIGTAVKGKEAVHSDLGYWIESEKNDTWRLKRAHLIEMKTCEWPKSHTLWTDGIEESDLIIPKSLAGPLSHHNTREGYRTQMKGPWHSEELEIRFEECPGTKVHVEETCGTRGPSLRSTTASGRVIEEWCCRECTMPPLSFRAKDGCWYGMEIRPRKEPESNLVRSMVTAGSTDHMDHFSLGVLVILLMVQEGLKKRMTTKIIISTSMAVLVAMILGGFSMSDLAKLAILMGATFAEMNTGGDVAHLALIAAFKVRPALLVSFIFRANWTPRESMLLALASCLLQTAISALEGDLMVLINGFALAWLAIRAMVVPRTDNITLAILAALTPLARGTLLVAWRAGLATCGGFMLLSLKGKGSVKKNLPFVMALGLTAVRLVDPINVVGLLLLTRSGKRSWPPSEVLTAVGLICALAGGFAKADIEMAGPMAAVGLLIVSYVVSGKSVDMYIERAGDITWEKDAEVTGNSPRLDVALDESGDFSLVEDDGPPMREIILKVVLMTICGMNPIAIPFAAGAWYVYVKTGKRSGALWDVPAPKEVKKGETTDGVYRVMTRRLLGSTQVGVGVMQEGVFHTMWHVTKGSALRSGEGRLDPYWGDVKQDLVSYCGPWKLDAAWDGHSEVQLLAVPPGERARNIQTLPGIFKTKDGDIGAVALDYPAGTSGSPILDKCGRVIGLYGNGVVIKNGSYVSAITQGRREEETPVECFEPSMLKKKQLTVLDLHPGAGKTRRVLPEIVREAIKTRLRTVILAPTRVVAAEMEEALRGLPVRYMTTAVNVTHSGTEIVDLMCHATFTSRLLQPIRVPNYNLYIMDEAHFTDPSSIAARGYISTRVEMGEAAAIFMTATPPGTRDAFPDSNSPIMDTEVEVPERAWSSGFDWVTDHSGKTVWFVPSVRNGNEIAACLTKAGKRVIQLSRKTFETEFQKTKHQEWDFVVTTDISEMGANFKADRVIDSRRCLKPVILDGERVILAGPMPVTHASAAQRRGRIGRNPNKPGDEYLYGGGCAETDEDHAHWLEARMLLDNIYLQDGLIASLYRPEADKVAAIEGEFKLRTEQRKTFVELMKRGDLPVWLAYQVASAGITYTDRRWCFDGTTNNTILEDSVPAEVWTRHGEKRVLKPRWMDARVCSDHAALKSFKEFAAGKRGAAFGVMEALGTLPGHMTERFQEAIDNLAVLMRAETGSRPYKAAAAQLPETLETIMLLGLLGTVSLGIFFVLMRNKGIGKMGFGMVTLGASAWLMWLSEIEPARIACVLIVVFLLLVVLIPEPEKQRSPQDNQMAIIIMVAVGLLGLITANELGWLERTKSDLSHLMGRREEGATIGFSMDIDLRPASAWAIYAALTTFITPAVQHAVTTSYNNYSLMAMATQAGVLFGMGKGMPFYAWDFGVPLLMIGCYSQLTPLTLIVAIILLVAHYMYLIPGLQAAAARAAQKRTAAGIMKNPVVDGIVVTDIDTMTIDPQVEKKMGQVLLIAVAVSSAILSRTAWGWGEAGALITAATSTLWEGSPNKYWNSSTATSLCNIFRGSYLAGASLIYTVTRNAGLVKRRGGGTGETLGEKWKARLNQMSALEFYSYKKSGITEVCREEARRALKDGVATGGHAVSRGSAKLRWLVERGYLQPYGKVIDLGCGRGGWSYYAATIRKVQEVKGYTKGGPGHEEPVLVQSYGWNIVRLKSGVDVFHMAAEPCDTLLCDIGESSSSPEVEEARTLRVLSMVGDWLEKRPGAFCIKVLCPYTSTMMETLERLQRRYGGGLVRVPLSRNSTHEMYWVSGAKSNTIKSVSTTSQLLLGRMDGPRRPVKYEEDVNLGSGTRAVVSCAEAPNMKIIGNRIERIRSEHAETWFFDENHPYRTWAYHGSYEAPTQGSASSLINGVVRLLSKPWDVVTGVTGIAMTDTTPYGQQRVFKEKVDTRVPDPQEGTRQVMSMVSSWLWKELGKHKRPRVCTKEEFINKVRSNAALGAIFEEEKEWKTAVEAVNDPRFWALVDKEREHHLRGECQSCVYNMMGKREKKQGEFGKAKGSRAIWYMWLGARFLEFEALGFLNEDHWMGRENSGGGVEGLGLQRLGYVLEEMSCIPGGRMYADDTAGWDTRISRFDLENEALITNQMEKGHRALALAIIKYTYQNKVVKVLRPAEKGKTVMDIISRQDQRGSGQVVTYALNTFTNLVVQLIRNMEAEEVLEMQDLWLLRRSEKVTNWLQSNGWDRLKRMAVSGDDCVVKPIDDRFAHALRFLNDMGKVRKDTQEWKPSTGWDNWEEVPFCSHHFNKLHLKDGRSIVVPCRHQDELIGRARVSPGAGWSIRETACLAKSYAQMWQLLYFHRRDLRLMANAICSSVPVDWVPTGRTTWSIHGKGEWMTTEDMLVVWNRVWIEENDHMEDKTPVTKWTDIPYLGKREDLWCGSLIGHRPRTTWAENIKNTVNMVRRIIGDEEKYMDYLSTQVRYLGEEGSTPGVL

SEQ ID NO: 9 - DNA, 10723 bp, Dengue virus type 2 strain 16681
agttgttagtctacgtggaccgacaaagacagattctttgagggagctaagctcaacgtagttctaacagttttttaattagagagcagatctctgatgaataaccaacggaaaaaggcgaaaaacacgcctttcaatatgctgaaacgcgagagaaaccgcgtgtcgactgtgcaacagctgacaaagagattctcacttggaatgctgcagggacgaggaccattaaaactgttcatggccctggtggcgttccttcgtttcctaacaatcccaccaacagcagggatattgaagagatggggaacaattaaaaaatcaaaagctattaatgttttgagagggttcaggaaagagattggaaggatgctgaacatcttgaataggagacgcagatctgcaggcatgatcattatgctgattccaacagtgatggcgttccatttaaccacacgtaacggagaaccacacatgatcgtcagcagacaagagaaagggaaaagtcttctgtttaaaacagaggatggcgtgaacatgtgtaccctcatggccatggaccttggtgaattgtgtgaagacacaatcacgtacaagtgtccccttctcaggcagaatgagccagaagacatagactgttggtgcaactctacgtccacgtgggtaacttatgggacgtgtaccaccatgggagaacatagaagagaaaaaagatcagtggcactcgttccacatgtgggaatgggactggagacacgaactgaaacatggatgtcatcagaaggggcctggaaacatgtccagagaattgaaacttggatcttgagacatccaggcttcaccatgatggcagcaatcctggcatacaccataggaacgacacatttccaaagagccctgattttcatcttactgacagctgtcactccttcaatgacaatgcgttgcataggaatgtcaaatagagactttgtggaaggggtttcaggaggaagctgggttgacatagtcttagaacatggaagctgtgtgacgacgatggcaaaaaacaaaccaacattggattttgaactgataaaaacagaagccaaacagcctgccaccctaaggaagtactgtatagaggcaaagctaaccaacacaacaacagaatctcgctgcccaacacaaggggaacccagcctaaatgaagagcaggacaaaaggttcgtctgcaaacactccatggtagacagaggatggggaaatggatgtggactatttggaaagggaggcattgtgacctgtgctatgttcagatgcaaaaagaacatggaaggaaaagttgtgcaaccagaaaacttggaatacaccattgtgataacacctcactcaggggaagagcatgcagtcggaaatgacacaggaaaacatggcaaggaaatcaaaataacaccacagagttccatcacagaagcagaattgacaggttatggcactgtcacaatggagtgctctccaagaacgggcctcgacttcaatgagatggtgttgctgcagatggaaaataaagcttggctggtgcacaggcaatggttcctagacctgccgttaccatggttgcccggagcggacacacaagggtcaaattggatacagaaagagacattggtcactttcaaaaatccccatgcgaagaaacaggatgttgttgttttaggatcccaagaaggggccatgcacacagcacttacaggggccacagaaatccaaatgtcatcaggaaacttactcttcacaggacatctcaagtgcaggctgagaatggacaagctacagctcaaaggaatgtcatactctatgtgcacaggaaagtttaaagttgtgaaggaaatagcagaaacacaacatggaacaatagttatcagagtgcaatatgaaggggacggctctccatgcaagatcccttttgagataatggatttggaaaaaagacatgtcttaggtcgcctgattacagtcaacccaattgtgacagaaaaagatagcccagtcaacatagaagcagaacctccattcggagacagctacatcatcataggagtagagccgggacaactgaagctcaactggtttaagaaaggaagttctatcggccaaatgtttgagacaacaatgaggggggcgaagagaatggccattttaggtgacacagcctgggattttggatccttgggaggagtgtttacatctataggaaaggctctccaccaagtctttggagcaatctatggagctgccttcagtggggtttcatggactatgaaaatcctcataggagtcattatcacatggataggaatgaattcacgcagcacctcactgtctgtgacactagtattggtgggaattgtgacactgtatttgggagtcatggtgcaggccgatagtggttgcgttgtgagctggaaaaacaaagaactgaaatgtggcagtgggattttcatcacagacaacgtgcacacatggacagaacaatacaagttccaaccagaatccccttcaaaactagcttcagctatccagaaagcccatgaagagggcatttgtggaatccgctcagtaacaagactggagaatctgatgtggaaacaaataacaccagaattgaatcacattctatcagaaaatgaggtgaagttaactattatgacaggagacatcaaaggaatcatgcaggcaggaaaacgatctctgcggcctcagcccactgagctgaagtattcatggaaaacatggggcaaagcaaaaatgctctctacagagtctcataaccagacctttctcattgatggccccgaaacagcagaatgccccaacacaaatagagcttggaattcgttggaagttgaagactatggctttggagtattcaccaccaatatatggctaaaattgaaagaaaaacaggatgtattctgcgactcaaaactcatgtcagcggccataaaagacaacagagccgtccatgccgatatgggttattggatagaaagtgcactcaatgacacatggaagatagagaaagcctctttcattgaagttaaaaactgccactggccaaaatcacacaccctctggagcaatggagtgctagaaagtgagatgataattccaaagaatctcgctggaccagtgtctcaacacaactatagaccaggctaccatacacaaataacaggaccatggcatctaggtaagcttgagatggactttgatttctgtgatggaacaacagtggtagtgactgaggactgcggaaatagaggaccctctttgagaacaaccactgcctctggaaaactcataacagaatggtgctgccgatcttgcacattaccaccgctaagatacagaggtgaggatgggtgctggtacgggatggaaatcagaccattgaaggagaaagaagagaatttggtcaactccttggtcacagctggacatgggcaggtcgacaacttttcactaggagtcttgggaatggcattgttcctggaggaaatgcttaggacccgagtaggaacgaaacatgcaatactactagttgcagtttcttttgtgacattgatcacagggaacatgtcctttagagacctgggaagagtgatggttatggtaggcgccactatgacggatgacataggtatgggcgtgacttatcttgccctactagcagccttcaaagtcagaccaacttttgcagctggactactcttgagaaagctgacctccaaggaattgatgatgactactataggaattgtactcctctcccagagcaccataccagagaccattcttgagttgactgatgcgttagccttaggcatgatggtcctcaaaatggtgagaaatatggaaaagtatcaattggcagtgactatcatggctatcttgtgcgtcccaaacgcagtgatattacaaaacgcatggaaagtgagttgcacaatattggcagtggtgtccgtttccccactgctcttaacatcctcacagcaaaaaacagattggataccattagcattgacgatcaaaggtctcaatccaacagctatttttctaacaaccctctcaagaaccagcaagaaaaggagctggccattaaatgaggctatcatggcagtcgggatggtgagcattttagccagttctctcctaaaaaatgatattcccatgacaggaccattagtggctggagggctcctcactgtgtgctacgtgctcactggacgatcggccgatttggaactggagagagcagccgatgtcaaatgggaagaccaggcagagatatcaggaagcagtccaatcctgtcaataacaatatcagaagatggtagcatgtcgataaaaaatgaagaggaagaacaaacactgaccatactcattagaacaggattgctggtgatctcaggactttttcctgtatcaataccaatcacggcagcagcatggtacctgtgggaagtgaagaaacaacgggccggagtattgtgggatgttccttcacccccacccatgggaaaggctgaactggaagatggagcctatagaattaagcaaaaagggattcttggatattcccagatcggagccggagtttacaaagaaggaacattccatacaatgtggcatgtcacacgtggcgctgttctaatgcataaaggaaagaggattgaaccatcatgggcggacgtcaagaaagacctaatatcatatggaggaggctggaagttagaaggagaatggaaggaaggagaagaagtccaggtattggcactggagcctggaaaaaatccaagagccgtccaaacgaaacctggtcttttcaaaaccaacgccggaacaataggtgctgtatctctggacttttctcctggaacgtcaggatctccaattatcgacaaaaaaggaaaagttgtgggtctttatggtaatggtgttgttacaaggagtggagcatatgtgagtgctatagcccagactgaaaaaagcattgaagacaacccagagatcgaagatgacattttccgaaagagaagactgaccatcatggacctccacccaggagcgggaaagacgaagagataccttccggccatagtcagagaagctataaaacggggtttgagaacattaatcttggcccccactagagttgtggcagctgaaatggaggaagcccttagaggacttccaataagataccagaccccagccatcagagctgagcacaccgggcgggagattgtggacctaatgtgtcatgccacatttaccatgaggctgctatcaccagttagagtgccaaactacaacctgattatcatggacgaagcccatttcacagacccagcaagtatagcagctagaggatacatctcaactcgagtggagatgggtgaggcagctgggatttttatgacagccactcccccgggaagcagagacccatttcctcagagcaatgcaccaatcatagatgaagaaagagaaatccctgaacgttcgtggaattccggacatgaatgggtcacggattttaaagggaagactgtttggttcgttccaagtataaaagcaggaaatgatatagcagcttgcctgaggaaaaatggaaagaaagtgatacaactcagtaggaagacctttgattctgagtatgtcaagactagaaccaatgattgggacttcgtggttacaactgacatttcagaaatgggtgccaatttcaaggctgagagggttatagaccccagacgctgcatgaaaccagtcatactaacagatggtgaagagcgggtgattctggcaggacctatgccagtgacccactctagtgcagcacaaagaagagggagaataggaagaaatccaaaaaatgagaatgaccagtacatatacatgggggaacctctggaaaatgatgaagactgtgcacactggaaagaagctaaaatgctcctagataacatcaacacgccagaaggaatcattcctagcatgttcgaaccagagcgtgaaaaggtggatgccattgatggcgaataccgcttgagaggagaagcaaggaaaacctttgtagacttaatgagaagaggagacctaccagtctggttggcctacagagtggcagctgaaggcatcaactacgcagacagaaggtggtgttttgatggagtcaagaacaaccaaatcctagaagaaaacgtggaagttgaaatctggacaaaagaaggggaaaggaagaaattgaaacccagatggttggatgctaggatctattctgacccactggcgctaaaagaatttaaggaatttgcagccggaagaaagtctctgaccctgaacctaatcacagaaatgggtaggctcccaaccttcatgactcagaaggcaagagacgcactggacaacttagcagtgctgcacacggctgaggcaggtggaagggcgtacaaccatgctctcagtgaactgccggagaccctggagacattgcttttactgacacttctggctacagtcacgggagggatctttttattcttgatgagcggaaggggcatagggaagatgaccctgggaatgtgctgcataatcacggctagcatcctcctatggtacgcacaaatacagccacactggatagcagcttcaataatactggagttttttctcatagttttgcttattccagaacctgaaaaacagagaacaccccaagacaaccaactgacctacgttgtcatagccatcctcacagtggtggccgcaaccatggcaaacgagatgggtttcctagaaaaaacgaagaaagatctcggattgggaagcattgcaacccagcaacccgagagcaacatcctggacatagatctacgtcctgcatcagcatggacgctgtatgccgtggccacaacatttgttacaccaatgttgagacatagcattgaaaattcctcagtgaatgtgtccctaacagctatagccaaccaagccacagtgttaatgggtctcgggaaaggatggccattgtcaaagatggacatcggagttccccttctcgccattggatgctactcacaagtcaaccccataactctcacagcagctcttttcttattggtagcacattatgccatcatagggccaggactccaagcaaaagcaaccagagaagctcagaaaagagcagcggcgggcatcatgaaaaacccaactgtcgatggaataacagtgattgacctagatccaataccttatgatccaaagtttgaaaagcagttgggacaagtaatgctcctagtcctctgcgtgactcaagtattgatgatgaggactacatgggctctgtgtgaggctttaaccttagctaccgggcccatctccacattgtgggaaggaaatccagggaggttttggaacactaccattgcggtgtcaatggctaacatttttagagggagttacttggccggagctggacttctcttttctattatgaagaacacaaccaacacaagaaggggaactggcaacataggagagacgcttggagagaaatggaaaagccgattgaacgcattgggaaaaagtgaattccagatctacaagaaaagtggaatccaggaagtggatagaaccttagcaaaagaaggcattaaaagaggagaaacggaccatcacgctgtgtcgcgaggctcagcaaaactgagatggttcgttgagagaaacatggtcacaccagaagggaaagtagtggacctcggttgtggcagaggaggctggtcatactattgtggaggactaaagaatgtaagagaagtcaaaggcctaacaaaaggaggaccaggacacgaagaacccatccccatgtcaacatatgggtggaatctagtgcgtcttcaaagtggagttgacgttttcttcatcccgccagaaaagtgtgacacattattgtgtgacataggggagtcatcaccaaatcccacagtggaagcaggacgaacactcagagtccttaacttagtagaaaattggttgaacaacaacactcaattttgcataaaggttctcaacccatatatgccctcagtcatagaaaaaatggaagcactacaaaggaaatatggaggagccttagtgaggaatccactctcacgaaactccacacatgagatgtactgggtatccaatgcttccgggaacatagtgtcatcagtgaacatgatttcaaggatgttgatcaacagatttacaatgagatacaagaaagccacttacgagccggatgttgacctcggaagcggaacccgtaacatcgggattgaaagtgagataccaaacctagatataattgggaaaagaatagaaaaaataaagcaagagcatgaaacatcatggcactatgaccaagaccacccatacaaaacgtgggcataccatggtagctatgaaacaaaacagactggatcagcatcatccatggtcaacggagtggtcaggctgctgacaaaaccttgggacgtcgtccccatggtgacacagatggcaatgacagacacgactccatttggacaacagcgcgtttttaaagagaaagtggacacgagaacccaagaaccgaaagaaggcacgaagaaactaatgaaaataacagcagagtggctttggaaagaattagggaagaaaaagacacccaggatgtgcaccagagaagaattcacaagaaaggtgagaagcaatgcagccttgggggccatattcactgatgagaacaagtggaagtcggcacgtgaggctgttgaagatagtaggttttgggagctggttgacaaggaaaggaatctccatcttgaaggaaagtgtgaaacatgtgtgtacaacatgatgggaaaaagagagaagaagctaggggaattcggcaaggcaaaaggcagcagagccatatggtacatgtggcttggagcacgcttcttagagtttgaagccctaggattcttaaatgaagatcactggttctccagagagaactccctgagtggagtggaaggagaagggctgcacaagctaggttacattctaagagacgtgagcaagaaagagggaggagcaatgtatgccgatgacaccgcaggatgggatacaagaatcacactagaagacctaaaaaatgaagaaatggtaacaaaccacatggaaggagaacacaagaaactagccgaggccattttcaaactaacgtaccaaaacaaggtggtgcgtgtgcaaagaccaacaccaagaggcacagtaatggacatcatatcgagaagagaccaaagaggtagtggacaagttggcacctatggactcaatactttcaccaatatggaagcccaactaatcagacagatggagggagaaggagtctttaaaagcattcagcacctaacaatcacagaagaaatcgctgtgcaaaactggttagcaagagtggggcgcgaaaggttatcaagaatggccatcagtggagatgattgtgttgtgaaacctttagatgacaggttcgcaagcgctttaacagctctaaatgacatgggaaagattaggaaagacatacaacaatgggaaccttcaagaggatggaatgattggacacaagtgcccttctgttcacaccatttccatgagttaatcatgaaagacggtcgcgtactcgttgttccatgtagaaaccaagatgaactgattggcagagcccgaatctcccaaggagcagggtggtctttgcgggagacggcctgtttggggaagtcttacgcccaaatgtggagcttgatgtacttccacagacgcgacctcaggctggcggcaaatgctatttgctcggcagtaccatcacattgggttccaacaagtcgaacaacctggtccatacatgctaaacatgaatggatgacaacggaagacatgctgacagtctggaacagggtgtggattcaagaaaacccatggatggaagacaaaactccagtggaatcatgggaggaaatcccatacttggggaaaagagaagaccaatggtgcggctcattgattgggttaacaagcagggccacctgggcaaagaacatccaagcagcaataaatcaagttagatcccttataggcaatgaagaatacacagattacatgccatccatgaaaagattcagaagagaagaggaagaagcaggagttctgtggtagaaagcaaaactaacatgaaacaaggctagaagtcaggtcggattaagccatagtacggaaaaaactatgctacctgtgagccccgtccaaggacgttaaaagaagtcaggccatcataaatgccatagcttgagtaaactatgcagcctgtagctccacctgagaaggtgtaaaaaatccgggaggccacaaaccatggaagctgtacgcatggcgtagtggactagcggttagaggagacccctcccttacaaatcgcagcaacaatgggggcccaaggcgagatgaagctgtagtctcgctggaaggactagaggttagaggagacccccccgaaacaaaaaacagcatattgacgctgggaaagaccagagatcctgctgtctcctcagcatcattccaggcacagaacgccagaaaatggaatggtgctgttgaatcaacaggttct

SEQ ID NO: 10 - protein, 3391 aa, Dengue virus type 2 strain 16681
MNNQRKKAKNTPFNMLKRERNRVSTVQQLTKRFSLGMLQGRGPLKLFMALVAFLRFLTIPPTAGILKRWGTIKKSKAINVLRGFRKEIGRMLNILNRRRSSAGMIIMLIPTVMAFHLTTRDGEPLMIVAKHERGRPLLFKTTEGINKCTLIAMDLGEMCEDTVTYKCPLLVNTEPEDIDCWCNLTSTWVMYGTCTQSGERRREKRSVALTPHSGMGLETRAETWMSSEGAWKHAQRVESWILRNPGFALLAGFMAYMIGQTGIQRTVFFVLMMLVAPSYGMRCVGVGNRDFVEGVSGGAWVDLVLEHGGCVTTMAQGKPTLDFELTKTTAKEVALLRTYCIEASISNITTATRCPTQGEPYLKEEQDQQYICRRDVVDRGWGNGCGLFGKGGVVTCAKFSCSGKITGNLVQIENLEYTVVVTVHNGDTHAVGNDTSNHGVTATITPRSPSVEVKLPDYGELTLDCEPRSGIDFNEMILMKMKKKTWLVHKQWFLDLPLPWTAGADTSEVHWNYKERMVTFKVPHAKRQDVTVLGSQEGAMHSALAGATEVDSGDGNHMFAGHLKCKVRMEKLRIKGMSYTMCSGKFSIDKEMAETQHGTTVVKVKYEGAGAPCKVPIEIRDVNKEKVVGRIISSTPLAENTNSVTNIELEPPFGDSYIVIGVGNSALTLHWFRKGSSIGKMFESTYRGAKRMAILGETAWDFGSVGGLFTSLGKAVHQVFGSVYTTLFGGVSWMIRILIGFLVLWIGTNSRNTSMAMTCIAAGIVTLYLGVMVQADSGCVVSWKNKELKCGSGIFITDNVHTWTEQYKFQPESPSKLASAIQKAHEEDICGIRSVTRLENLMWKQITPELNHILSENEVKLTIMTGDIKGIMQAGKRSLRPQPTELKYSWKTWGKAKMLSTESHNQTFLIDGPETAECPNTNRAWNSLEVEDYGFGVFTTNIWLKLKEKQDVFCDSKLMSAAIKDNRAVHADMGYWIESALNDTWKIEKASFIEVKNCHWPKSHTLWSNGVLESEMIIPKNLAGPVSQHNYRPGYHTQITGPWHLGKLEMDFDFCDGTTVVVTEDCGNRGPSLRTTTASGKLITEWCCRSCTLPPLRYRGEDGCWYGMEIRPLKEKEENLVNSLVTAGHGQVDNFSLGVLGMALFLEEMLRTRVGTKHAILLVAVSFVTLITGNMSFRDLGRVMVMVGATMTDDIGMGVTYLALLAAFKVRPTFAAGLLLRKLTSKELMMTTIGIVLLSQSTIPETILELTDALALGMMVLKMVRNMEKYQLAVTIMAILCVPNAVILQNAWKVSCTILAVVSVSPLFLTSSQQKTDWIPLALTIKGLNPTAIFLTTLSRTSKKRSWPLNEAIMAVGMVSILASSLLKNDIPMTGPLVAGGLLTVCYVLTGRSADLELERAADVKWEDQAEISGSSPILSITISEDGSMSIKNEEEEQTLTILIRTGLLVISGLFPVSIPITAAAWYLWEVKKQRAGVLWDVPSPPPMGKAELEDGAYRIKQKGILGYSQIGAGVYKEGTFHTMWHVTRGAVLMHKGKRIEPSWADVKKDLISYGGGWKLEGEWKEGEEVQVLALEPGKNPRAVQTKPGLFKTNAGTIGAVSLDFSPGTSGSPIIDKKGKVVGLYGNGVVTRSGAYVSAIAQTEKSIEDNPEIEDDIFRKRRLTIMDLHPGAGKTKRYLPAIVREAIKRGLRTLILAPTRVVAAEMEEALRGLPIRYQTPAIRAVHTGREIVDLMCHATFTMRLLSPVRVPNYNLIIMDEAHFTDPASIAARGYISTRVEMGEAAGIFMTATPPGSRDPFPQSNAPIIDEEREIPERSWNSGHEWVTDFKGKTVWFVPSIKAGNDIAACLRKNGKKVIQLSRKTFDSEYVKTRTNDWDFVVTTDISEMGANFKAERVIDPRRCMKPVILTDGEERVILAGPMPVTHSSAAQRRGRIGRNPKNENDQYIYMGEPLENDEDCAHWKEAKMLLDNINTPEGIIPSMFEPEREKVDAIDGEYRLRGEARKTFVDLMRRGDLPVWLAYRVAAEGINYADRRWCFDGVKNNQILEENVEVEIWTKEGERKKLKPRWLDARIYSDPLALKEFKEFAAGRKSLTLNLITEMGRLPTFMTQKARDALDNLAVLHTAEAGGRAYNHALSELPETLETLLLLTLLATVTGGIFLFLMSARGIGKMTLGMCCIITASILLWYAQIQPHWIAASIILEFFLIVLLIPEPEKQRTPQDNQLTYVVIAILTVVAATMANEMGFLEKTKKDLGLGSIATQQPESNILDIDLRPASAWTLYAVATTFVTPMLRHSIENSSVNVSLTAIANQATVLMGLGKGWPLSKMDIGVPLLAIGCYSQVNPITLTAALFLLVAHYAIIGPGLQAKATREAQKRAAAGIMKNPTVDGITVIDLDPIPYDPKFEKQLGQVMLLVLCVTQVLMMRTTWALCEALTLATGPISTLWEGNPGRFWNTTIAVSMANIFRGSYLAGAGLLFSIMKNTTNTRRGTGNIGETLGEKWKSRLNALGKSEFQIYKKSGIQEVDRTLAKEGIKRGETDHHAVSRGSAKLRWFVERNMVTPEGKVVDLGCGRGGWSYYCGGLKNVREVKGLTKGGPGHEEPIPMSTYGWNLVRLQSGVDVFFIPPEKCDTLLCDIGESSPNPTVEAGRTLRVLNLVENWLNNNTQFCIKVLNPYMPSVIEKMEALQRKYGGALVRNPLSRNSTHEMYWVSNASGNIVSSVNMISRMLINRFTMRYKKATYEPDVDLGSGTRNIGIESEIPNLDIIGKRIEKIKQEHETSWHYDQDHPYKTWAYHGSYETKQTGSASSMVNGVVRLLTKPWDVVPMVTQMAMTDTTPFGQQRVFKEKVDTRTQEPKEGTKKLMKITAEWLWKELGKKKTPRMCTREEFTRKVRSNAALGAIFTDENKWKSAREAVEDSRFWELVDKERNLHLEGKCETCVYNMMGKREKKLGEFGKAKGSRAIWYMWLGARFLEFEALGFLNEDHWFSRENSLSGVEGEGLHKLGYILRDVSKKEGGAMYADDTAGWDTRITLEDLKNEEMVTNHMEGEHKKLAEAIFKLTYQNKVVRVQRPTPRGTVMDIISRRDQRGSGQVGTYGLNTFTNMEAQLIRQMEGEGVFKSIQHLTITEEIAVQNWLARVGRERLSRMAISGDDCVVKPLDDRFASALTALNDMGKIRKDIQQWEPSRGWNDWTQVPFCSHHFHELIMKDGRVLVVPCRNQDELIGRARISQGAGWSLRETACLGKSYAQMWSLMYFHRRDLRLAANAICSAVPSHWVPTSRTTWSIHAKHEWMTTEDMLTVWNRVWIQENPWMEDKTPVESWEEIPYLGKREDQWCGSLIGLTSRATWAKNIQAAINQVRSLIGNEEYTDYMPSMKRFRREEEEAGVLW

SEQ ID NO: 11 - DNA, 10723 bp, Dengue virus type 2 strain PDK-53
agttgttagtctacgtggaccgacaaagacagattctttgagggagctaagctcaatgtagttctaacagttttttaattagagagcagatctctgatgaataaccaacggaaaaaggcgaaaaacacgcctttcaatatgctgaaacgcgagagaaaccgcgtgtcgactgtgcaacagctgacaaagagattctcacttggaatgctgcagggacgaggaccattaaaactgttcatggccctggtggcgttccttcgtttcctaacaatcccaccaacagcagggatattgaagagatggggaacaattaaaaaatcaaaagctattaatgttttgagagggttcaggaaagagattggaaggatgctgaacatcttgaataggagacgcagatctgcaggcatgatcattatgctgattccaacagtgatggcgttccatttaaccacacgtaacggagaaccacacatgatcgtcagcagacaagagaaagggaaaagtcttctgtttaaaacagaggttggcgtgaacatgtgtaccctcatggccatggaccttggtgaattgtgtgaagacacaatcacgtacaagtgtccccttctcaggcagaatgagccagaagacatagactgttggtgcaactctacgtccacgtgggtaacttatgggacgtgtaccaccatgggagaacatagaagagaaaaaagatcagtggcactcgttccacatgtgggaatgggactggagacacgaactgaaacatggatgtcatcagaaggggcctggaaacatgtccagagaattgaaacttggatcttgagacatccaggcttcaccatgatggcagcaatcctggcatacaccataggaacgacacatttccaaagagccctgattttcatcttactgacagctgtcactccttcaatgacaatgcgttgcataggaatgtcaaatagagactttgtggaaggggtttcaggaggaagctgggttgacatagtcttagaacatggaagctgtgtgacgacgatggcaaaaaacaaaccaacattggattttgaactgataaaaacagaagccaaacagcctgccaccctaaggaagtactgtatagaggcaaagctaaccaacacaacaacagaatctcgctgcccaacacaaggggaacccagcctaaatgaagagcaggacaaaaggttcgtctgcaaacactccatggtagacagaggatggggaaatggatgtggactatttggaaagggaggcattgtgacctgtgctatgttcagatgcaaaaagaacatggaaggaaaagttgtgcaaccagaaaacttggaatacaccattgtgataacacctcactcaggggaagagcatgcagtcggaaatgacacaggaaaacatggcaaggaaatcaaaataacaccacagagttccatcacagaagcagaattgacaggttatggcactgtcacaatggagtgctctccaagaacgggcctcgacttcaatgagatggtgttgctgcagatggaaaataaagcttggctggtgcacaggcaatggttcctagacctgccgttaccatggttgcccggagcggacacacaagggtcaaattggatacagaaagagacattggtcactttcaaaaatccccatgcgaagaaacaggatgttgttgttttaggatcccaagaaggggccatgcacacagcacttacaggggccacagaaatccaaatgtcatcaggaaacttactcttcacaggacatctcaagtgcaggctgagaatggacaagctacagctcaaaggaatgtcatactctatgtgcacaggaaagtttaaagttgtgaaggaaatagcagaaacacaacatggaacaatagttatcagagtgcaatatgaaggggacggctctccatgcaagatcccttttgagataatggatttggaaaaaagacatgtcttaggtcgcctgattacagtcaacccaattgtgacagaaaaagatagcccagtcaacatagaagcagaacctccatttggagacagctacatcatcataggagtagagccgggacaactgaagctcaactggtttaagaaaggaagttctatcggccaaatgtttgagacaacaatgaggggggcgaagagaatggccattttaggtgacacagcctgggattttggatccttgggaggagtgtttacatctataggaaaggctctccaccaagtctttggagcaatctatggagctgccttcagtggggtttcatggactatgaaaatcctcataggagtcattatcacatggataggaatgaattcacgcagcacctcactgtctgtgacactagtattggtgggaattgtgacactgtatttgggagtcatggtgcaggccgatagtggttgcgttgtgagctggaaaaacaaagaactgaaatgtggcagtgggattttcatcacagacaacgtgcacacatggacagaacaatacaagttccaaccagaatccccttcaaaactagcttcagctatccagaaagcccatgaagaggacatttgtggaatccgctcagtaacaagactggagaatctgatgtggaaacaaataacaccagaattgaatcacattctatcagaaaatgaggtgaagttaactattatgacaggagacatcaaaggaatcatgcaggcaggaaaacgatctctgcggcctcagcccactgagctgaagtattcatggaaaacatggggcaaagcaaaaatgctctctacagagtctcataaccagacctttctcattgatggccccgaaacagcagaatgccccaacacaaatagagcttggaattcgttggaagttgaagactatggctttggagtattcaccaccaatatatggctaaaattgaaagaaaaacaggatgtattctgcgactcaaaactcatgtcagcggccataaaagacaacagagccgtccatgccgatatgggttattggatagaaagtgcactcaatgacacatggaagatagagaaagcctctttcattgaagttaaaaactgccactggccaaaatcacacaccctctggagcaatggagtgctagaaagtgagatgataattccaaagaatctcgctggaccagtgtctcaacacaactatagaccaggctaccatacacaaataacaggaccatggcatctaggtaagcttgagatggactttgatttctgtgatggaacaacagtggtagtgactgaggactgcggaaatagaggaccctctttgagaacaaccactgcctctggaaaactcataacagaatggtgctgccgatcttgcacattaccaccgctaagatacagaggtgaggatgggtgctggtacgggatggaaatcagaccattgaaggagaaagaagagaatttggtcaactccttggtcacagctggacatgggcaggtcgacaacttttcactaggagtcttgggaatggcattgttcctggaggaaatgcttaggacccgagtaggaacgaaacatgcaatactactagttgcagtttcttttgtgacattgatcacagggaacatgtcctttagagacctgggaagagtgatggttatggtaggcgccactatgacggatgacataggtatgggcgtgacttatcttgccctactagcagccttcaaagtcagaccaacttttgcagctggactactcttgagaaagctgacctccaaggaattgatgatgactactataggaattgtactcctctcccagagcaccataccagagaccattcttgagttgactgatgcgttagccttaggcatgatggtcctcaaaatggtgagaaatatggaaaagtatcaattggcagtgactatcatggctatcttgtgcgtcccaaacgcagtgatattacaaaacgcatggaaagtgagttgcacaatattggcagtggtgtccgtttccccactgttcttaacatcctcacagcaaaaaacagattggataccattagcattgacgatcaaaggtctcaatccaacagctatttttctaacaaccctctcaagaaccagcaagaaaaggagctggccattaaatgaggctatcatggcagtcgggatggtgagcattttagccagttctctcctaaaaaatgatattcccatgacaggaccattagtggctggagggctcctcactgtgtgctacgtgctcactggacgatcggccgatttggaactggagagagcagccgatgtcaaatgggaagaccaggcagagatatcaggaagcagtccaatcctgtcaataacaatatcagaagatggtagcatgtcgataaaaaatgaagaggaagaacaaacactgaccatactcattagaacaggattgctggtgatctcaggactttttcctgtatcaataccaatcacggcagcagcatggtacctgtgggaagtgaagaaacaacgggccggagtattgtgggatgttccttcacccccacccatgggaaaggctgaactggaagatggagcctatagaattaagcaaaaagggattcttggatattcccagatcggagccggagtttacaaagaaggaacattccatacaatgtggcatgtcacacgtggcgctgttctaatgcataaaggaaagaggattgaaccatcatgggcggacgtcaagaaagacctaatatcatatggaggaggctggaagttagaaggagaatggaaggaaggagaagaagtccaggtattggcactggagcctggaaaaaatccaagagccgtccaaacgaaacctggtcttttcaaaaccaacgccggaacaataggtgctgtatctctggacttttctcctggaacgtcaggatctccaattatcgacaaaaaaggaaaagttgtgggtctttatggtaatggtgttgttacaaggagtggagcatatgtgagtgctatagcccagactgaaaaaagcattgaagacaacccagagatcgaagatgacattttccgaaagagaagactgaccatcatggacctccacccaggagcgggaaagacgaagagataccttccggccatagtcagagaagctataaaacggggtttgagaacattaatcttggcccccactagagttgtggcagctgaaatggaggaagcccttagaggacttccaataagataccagaccccagccatcagagctgtgcacaccgggcgggagattgtggacctaatgtgtcatgccacatttaccatgaggctgctatcaccagttagagtgccaaactacaacctgattatcatggacgaagcccatttcacagacccagcaagtatagcagctagaggatacatctcaactcgagtggagatgggtgaggcagctgggatttttatgacagccactcccccgggaagcagagacccatttcctcagagcaatgcaccaatcatagatgaagaaagagaaatccctgaacgctcgtggaattccggacatgaatgggtcacggattttaaagggaagactgtttggttcgttccaagtataaaagcaggaaatgatatagcagcttgcctgaggaaaaatggaaagaaagtgatacaactcagtaggaagacctttgattctgagtatgtcaagactagaaccaatgattgggacttcgtggttacaactgacatttcagaaatgggtgccaatttcaaggctgagagggttatagaccccagacgctgcatgaaaccagtcatactaacagatggtgaagagcgggtgattctggcaggacctatgccagtgacccactctagtgcagcacaaagaagagggagaataggaagaaatccaaaaaatgagaatgaccagtacatatacatgggggaacctctggaaaatgatgaagactgtgcacactggaaagaagctaaaatgctcctagataacatcaacacgccagaaggaatcattcctagcatgttcgaaccagagcgtgaaaaggtggatgccattgatggcgaataccgcttgagaggagaagcaaggaaaacctttgtagacttaatgagaagaggagacctaccagtctggttggcctacagagtggcagctgaaggcatcaactacgcagacagaaggtggtgttttgatggagtcaagaacaaccaaatcctagaagaaaacgtggaagttgaaatctggacaaaagaaggggaaaggaagaaattgaaacccagatggttggatgctaggatctattctgacccactggcgctaaaagaatttaaggaatttgcagccggaagaaagtctctgaccctgaacctaatcacagaaatgggtaggctcccaaccttcatgactcagaaggcaagagacgcactggacaacttagcagtgctgcacacggctgaggcaggtggaagggcgtacaaccatgctctcagtgaactgccggagaccctggagacattgcttttactgacacttctggctacagtcacgggagggatctttttattcttgatgagcgcaaggggcatagggaagatgaccctgggaatgtgctgcataatcacggctagcatcctcctatggtacgcacaaatacagccacactggatagcagcttcaataatactggagttttttctcatagttttgcttattccagaacctgaaaaacagagaacaccccaagacaaccaactgacctacgttgtcatagccatcctcacagtggtggccgcaaccatggcaaacgagatgggtttcctagaaaaaacgaagaaagatctcggattgggaagcattgcaacccagcaacccgagagcaacatcctggacatagatctacgtcctgcatcagcatggacgctgtatgccgtggccacaacatttgttacaccaatgttgagacatagcattgaaaattcctcagtgaatgtgtccctaacagctatagccaaccaagccacagtgttaatgggtctcgggaaaggatggccattgtcaaagatggacatcggagttccccttctcgccattggatgctactcacaagtcaaccccataactctcacagcagctcttttcttattggtagcacattatgccatcatagggccaggactccaagcaaaagcaaccagagaagctcagaaaagagcagcggcgggcatcatgaaaaacccaactgtcgatggaataacagtgattgacctagatccaataccttatgatccaaagtttgaaaagcagttgggacaagtaatgctcctagtcctctgcgtgactcaagtattgatgatgaggactacatgggctctgtgtgaggctttaaccttagctaccgggcccatctccacattgtgggaaggaaatccagggaggttttggaacactaccattgcggtgtcaatggctaacatttttagagggagttacttggccggagctggacttctcttttctattatgaagaacacaaccaacacaagaaggggaactggcaacataggagagacgcttggagagaaatggaaaagccgattgaacgcattgggaaaaagtgaattccagatctacaagaaaagtggaatccaggaagtggatagaaccttagcaaaagaaggcattaaaagaggagaaacggaccatcacgctgtgtcgcgaggctcagcaaaactgagatggttcgttgagagaaacatggtcacaccagaagggaaagtagtggacctcggttgtggcagaggaggctggtcatactattgtggaggactaaagaatgtaagagaagtcaaaggcctaacaaaaggaggaccaggacacgaagaacccatccccatgtcaacatatgggtggaatctagtgcgtcttcaaagtggagttgacgttttcttcatcccgccagaaaagtgtgacacattattgtgtgacataggggagtcatcaccaaatcccacagtggaagcaggacgaacactcagagtccttaacttagtagaaaattggttgaacaacaacactcaattttgcataaaggttctcaacccatatatgccctcagtcatagaaaaaatggaagcactacaaaggaaatatggaggagccttagtgaggaatccactctcacgaaactccacacatgagatgtactgggtatccaatgcttccgggaacatagtgtcatcagtgaacatgatttcaaggatgttgatcaacagatttacaatgagatacaagaaagccacttacgagccggatgttgacctcggaagcggaacccgtaacatcgggattgaaagtgagataccaaacctagatataattgggaaaagaatagaaaaaataaagcaagagcatgaaacatcatggcactatgaccaagaccacccatacaaaacgtgggcataccatggtagctatgaaacaaaacagactggatcagcatcatccatggtcaacggagtggtcaggctgctgacaaaaccttgggacgttgtccccatggtgacacagatggcaatgacagacacgactccatttggacaacagcgcgtttttaaagagaaagtggacacgagaacccaagaaccgaaagaaggcacgaagaaactaatgaaaataacagcagagtggctttggaaagaattagggaagaaaaagacacccaggatgtgcaccagagaagaattcacaagaaaggtgagaagcaatgcagccttgggggccatattcactgatgagaacaagtggaagtcggcacgtgaggctgttgaagatagtaggttttgggagctggttgacaaggaaaggaatctccatcttgaaggaaagtgtgaaacatgtgtgtacaacatgatgggaaaaagagagaagaagctaggggaattcggcaaggcaaaaggcagcagagccatatggtacatgtggcttggagcacgcttcttagagtttgaagccctaggattcttaaatgaagatcactggttctccagagagaactccctgagtggagtggaaggagaagggctgcacaagctaggttacattctaagagacgtgagcaagaaagagggaggagcaatgtatgccgatgacaccgcaggatgggatacaagaatcacactagaagacctaaaaaatgaagaaatggtaacaaaccacatggaaggagaacacaagaaactagccgaggccattttcaaactaacgtaccaaaacaaggtggtgcgtgtgcaaagaccaacaccaagaggcacagtaatggacatcatatcgagaagagaccaaagaggtagtggacaagttggcacctatggactcaatactttcaccaatatggaagcccaactaatcagacagatggagggagaaggagtctttaaaagcattcagcacctaacaatcacagaagaaatcgctgtgcaaaactggttagcaagagtggggcgcgaaaggttatcaagaatggccatcagtggagatgattgtgttgtgaaacctttagatgacaggttcgcaagcgctttaacagctctaaatgacatgggaaagattaggaaagacatacaacaatgggaaccttcaagaggatggaatgattggacacaagtgcccttctgttcacaccatttccatgagttaatcatgaaagacggtcgcgtactcgttgttccatgtagaaaccaagatgaactgattggcagagcccgaatctcccaaggagcagggtggtctttgcgggagacggcctgtttggggaagtcttacgcccaaatgtggagcttgatgtacttccacagacgcgacctcaggctggcggcaaatgctatttgctcggcagtaccatcacattgggttccaacaagtcgaacaacctggtccatacatgctaaacatgaatggatgacaacggaagacatgctgacagtctggaacagggtgtggattcaagaaaacccatggatggaagacaaaactccagtggaatcatgggaggaaatcccatacttggggaaaagagaagaccaatggtgcggctcattgattgggttaacaagcagggccacctgggcaaagaacatccaagcagcaataaatcaagttagatcccttataggcaatgaagaatacacagattacatgccatccatgaaaagattcagaagagaagaggaagaagcaggagttctgtggtagaaagcaaaactaacatgaaacaaggctagaagtcaggtcggattaagccatagtacggaaaaaactatgctacctgtgagccccgtccaaggacgttaaaagaagtcaggccatcataaatgccatagcttgagtaaactatgcagcctgtagctccacctgagaaggtgtaaaaaatccgggaggccacaaaccatggaagctgtacgcatggcgtagtggactagcggttagaggagacccctcccttacaaatcgcagcaacaatgggggcccaaggcgagatgaagctgtagtctcgctggaaggactagaggttagaggagacccccccgaaacaaaaaacagcatattgacgctgggaaagaccagagatcctgctgtctcctcagcatcattccaggcacagaacgccagaaaatggaatggtgctgttgaatcaacaggttct

SEQ ID NO: 12 - protein, 3391 aa, Dengue virus type 2 strain PDK-53
MNNQRKKAKNTPFNMLKRERNRVSTVQQLTKRFSLGMLQGRGPLKLFMALVAFLRFLTIPPTAGILKRWGTIKKSKAINVLRGFRKEIGRMLNILNRRRRSAGMIIMLIPTVMAFHLTTRNGEPHMIVSRQEKGKSLLFKTEVGVNMCTLMAMDLGELCEDTITYKCPLLRQNEPEDIDCWCNSTSTWVTYGTCTTMGEHRREKRSVALVPHVGMGLETRTETWMSSEGAWKHVQRIETWILRHPGFTMMAAILAYTIGTTHFQRALIFILLTAVTPSMTMRCIGMSNRDFVEGVSGGSWVDIVLEHGSCVTTMAKNKPTLDFELIKTEAKQPATLRKYCIEAKLTNTTTESRCPTQGEPSLNEEQDKRFVCKHSMVDRGWGNGCGLFGKGGIVTCAMFRCKKNMEGKVVQPENLEYTIVITPHSGEEHAVGNDTGKHGKEIKITPQSSITEAELTGYGTVTMECSPRTGLDFNEMVLLQMENKAWLVHRQWFLDLPLPWLPGADTQGSNWIQKETLVTFKNPHAKKQDVVVLGSQEGAMHTALTGATEIQMSSGNLLFTGHLKCRLRMDKLQLKGMSYSMCTGKFKVVKEIAETQHGTIVIRVQYEGDGSPCKIPFEIMDLEKRHVLGRLITVNPIVTEKDSPVNIEAEPPFGDSYIIIGVEPGQLKLNWFKKGSSIGQMFETTMRGAKRMAILGDTAWDFGSLGGVFTSIGKALHQVFGAIYGAAFSGVSWTMKILIGVIITWIGMNSRSTSLSVTLVLVGIVTLYLGVMVQADSGCVVSWKNKELKCGSGIFITDNVHTWTEQYKFQPESPSKLASAIQKAHEEDICGIRSVTRLENLMWKQITPELNHILSENEVKLTIMTGDIKGIMQAGKRSLRPQPTELKYSWKTWGKAKMLSTESHNQTFLIDGPETAECPNTNRAWNSLEVEDYGFGVFTTNIWLKLKEKQDVFCDSKLMSAAIKDNRAVHADMGYWIESALNDTWKIEKASFIEVKNCHWPKSHTLWSNGVLESEMIIPKNLAGPVSQHNYRPGYHTQITGPWHLGKLEMDFDFCDGTTVVVTEDCGNRGPSLRTTTASGKLITEWCCRSCTLPPLRYRGEDGCWYGMEIRPLKEKEENLVNSLVTAGHGQVDNFSLGVLGMALFLEEMLRTRVGTKHAILLVAVSFVTLITGNMSFRDLGRVMVMVGATMTDDIGMGVTYLALLAAFKVRPTFAAGLLLRKLTSKELMMTTIGIVLLSQSTIPETILELTDALALGMMVLKMVRNMEKYQLAVTIMAILCVPNAVILQNAWKVSCTILAVVSVSPLFLTSSQQKTDWIPLALTIKGLNPTAIFLTTLSRTSKKRSWPLNEAIMAVGMVSILASSLLKNDIPMTGPLVAGGLLTVCYVLTGRSADLELERAADVKWEDQAEISGSSPILSITISEDGSMSIKNEEEEQTLTILIRTGLLVISGLFPVSIPITAAAWYLWEVKKQRAGVLWDVPSPPPMGKAELEDGAYRIKQKGILGYSQIGAGVYKEGTFHTMWHVTRGAVLMHKGKRIEPSWADVKKDLISYGGGWKLEGEWKEGEEVQVLALEPGKNPRAVQTKPGLFKTNAGTIGAVSLDFSPGTSGSPIIDKKGKVVGLYGNGVVTRSGAYVSAIAQTEKSIEDNPEIEDDIFRKRRLTIMDLHPGAGKTKRYLPAIVREAIKRGLRTLILAPTRVVAAEMEEALRGLPIRYQTPAIRAVHTGREIVDLMCHATFTMRLLSPVRVPNYNLIIMDEAHFTDPASIAARGYISTRVEMGEAAGIFMTATPPGSRDPFPQSNAPIIDEEREIPERSWNSGHEWVTDFKGKTVWFVPSIKAGNDIAACLRKNGKKVIQLSRKTFDSEYVKTRTNDWDFVVTTDISEMGANFKAERVIDPRRCMKPVILTDGEERVILAGPMPVTHSSAAQRRGRIGRNPKNENDQYIYMGEPLENDEDCAHWKEAKMLLDNINTPEGIIPSMFEPEREKVDAIDGEYRLRGEARKTFVDLMRRGDLPVWLAYRVAAEGINYADRRWCFDGVKNNQILEENVEVEIWTKEGERKKLKPRWLDARIYSDPLALKEFKEFAAGRKSLTLNLITEMGRLPTFMTQKARDALDNLAVLHTAEAGGRAYNHALSELPETLETLLLLTLLATVTGGIFLFLMSARGIGKMTLGMCCIITASILLWYAQIQPHWIAASIILEFFLIVLLIPEPEKQRTPQDNQLTYVVIAILTVVAATMANEMGFLEKTKKDLGLGSIATQQPESNILDIDLRPASAWTLYAVATTFVTPMLRHSIENSSVNVSLTAIANQATVLMGLGKGWPLSKMDIGVPLLAIGCYSQVNPITLTAALFLLVAHYAIIGPGLQAKATREAQKRAAAGIMKNPTVDGITVIDLDPIPYDPKFEKQLGQVMLLVLCVTQVLMMRTTWALCEALTLATGPISTLWEGNPGRFWNTTIAVSMANIFRGSYLAGAGLLFSIMKNTTNTRRGTGNIGETLGEKWKSRLNALGKSEFQIYKKSGIQEVDRTLAKEGIKRGETDHHAVSRGSAKLRWFVERNMVTPEGKVVDLGCGRGGWSYYCGGLKNVREVKGLTKGGPGHEEPIPMSTYGWNLVRLQSGVDVFFIPPEKCDTLLCDIGESSPNPTVEAGRTLRVLNLVENWLNNNTQFCIKVLNPYMPSVIEKMEALQRKYGGALVRNPLSRNSTHEMYWVSNASGNIVSSVNMISRMLINRFTMRYKKATYEPDVDLGSGTRNIGIESEIPNLDIIGKRIEKIKQEHETSWHYDQDHPYKTWAYHGSYETKQTGSASSMVNGVVRLLTKPWDVVPMVTQMAMTDTTPFGQQRVFKEKVDTRTQEPKEGTKKLMKITAEWLWKELGKKKTPRMCTREEFTRKVRSNAALGAIFTDENKWKSAREAVEDSRFWELVDKERNLHLEGKCETCVYNMMGKREKKLGEFGKAKGSRAIWYMWLGARFLEFEALGFLNEDHWFSRENSLSGVEGEGLHKLGYILRDVSKKEGGAMYADDTAGWDTRITLEDLKNEEMVTNHMEGEHKKLAEAIFKLTYQNKVVRVQRPTPRGTVMDIISRRDQRGSGQVGTYGLNTFTNMEAQLIRQMEGEGVFKSIQHLTITEEIAVQNWLARVGRERLSRMAISGDDCVVKPLDDRFASALTALNDMGKIRKDIQQWEPSRGWNDWTQVPFCSHHFHELIMKDGRVLVVPCRNQDELIGRARISQGAGWSLRETACLGKSYAQMWSLMYFHRRDLRLAANAICSAVPSHWVPTSRTTWSIHAKHEWMTTEDMLTVWNRVWIQENPWMEDKTPVESWEEIPYLGKREDQWCGSLIGLTSRATWAKNIQAAINQVRSLIGNEEYTDYMPSMKRFRREEEEAGVLW

SEQ ID NO: 13 - DNA, 10807 bp, Zika virus strain PRVABC59
agttgttgatctgtgtgaatcagactgcgacagttcgagtttgaagcgaaagctagcaacagtatcaacaggttttattttggatttggaaacgagagtttctggtcatgaaaaacccaaaaaagaaatccggaggattccggattgtcaatatgctaaaacgcggagtagcccgtgtgagcccctttgggggcttgaagaggctgccagccggacttctgctgggtcatgggcccatcaggatggtcttggcgattctagcctttttgagattcacggcaatcaagccatcactgggtctcatcaatagatggggttcagtggggaaaaaagaggctatggaaacaataaagaagttcaagaaagatctggctgccatgctgagaataatcaatgctaggaaggagaagaagagacgaggcgcagatactagtgtcggaattgttggcctcctgctgaccacagctatggcagcggaggtcactagacgtgggagtgcatactatatgtacttggacagaaacgatgctggggaggccatatcttttccaaccacattggggatgaataagtgttatatacagatcatggatcttggacacatgtgtgatgccaccatgagctatgaatgccctatgctggatgagggggtggaaccagatgacgtcgattgttggtgcaacacgacgtcaacttgggttgtgtacggaacctgccatcacaaaaaaggtgaagcacggagatctagaagagctgtgacgctcccctcccattccaccaggaagctgcaaacgcggtcgcaaacctggttggaatcaagagaatacacaaagcacttgattagagtcgaaaattggatattcaggaaccctggcttcgcgttagcagcagctgccatcgcttggcttttgggaagctcaacgagccaaaaagtcatatacttggtcatgatactgctgattgccccggcatacagcatcaggtgcataggagtcagcaatagggactttgtggaaggtatgtcaggtgggacttgggttgatgttgtcttggaacatggaggttgtgtcaccgtaatggcacaggacaaaccgactgtcgacatagagctggttacaacaacagtcagcaacatggcggaggtaagatcctactgctatgaggcatcaatatcagacatggcttctgacagccgctgcccaacacaaggtgaagcctaccttgacaagcaatcagacactcaatatgtctgcaaaagaacgttagtggacagaggctggggaaatggatgtggactttttggcaaagggagcctggtgacatgcgctaagtttgcatgctccaagaaaatgaccgggaagagcatccagccagagaatctggagtaccggataatgctgtcagttcatggctcccagcacagtgggatgatcgttaatgacacaggacatgaaactgatgagaatagagcgaaagttgagataacgcccaattcaccgagagccgaagccaccctggggggttttggaagcctaggacttgattgtgaaccgaggacaggccttgacttttcagatttgtattacttgactatgaataacaagcactggttggttcacaaggagtggttccacgacattccattaccttggcacgctggggcagacaccggaactccacactggaacaacaaagaagcactggtagagttcaaggacgcacatgccaaaaggcaaactgtcgtggttctagggagtcaagaaggagcagttcacacggcccttgctggagctctggaggctgagatggatggtgcaaagggaaggctgtcctctggccacttgaaatgtcgcctgaaaatggataaacttagattgaagggcgtgtcatactccttgtgtactgcagcgttcacattcaccaagatcccggctgaaacactgcacgggacagtcacagtggaggtacagtacgcagggacagatggaccttgcaaggttccagctcagatggcggtggacatgcaaactctgaccccagttgggaggttgataaccgctaaccccgtaatcactgaaagcactgagaactctaagatgatgctggaacttgatccaccatttggggactcttacattgtcataggagtcggggagaagaagatcacccaccactggcacaggagtggcagcaccattggaaaagcatttgaagccactgtgagaggtgccaagagaatggcagtcttgggagacacagcctgggactttggatcagttggaggcgctctcaactcattgggcaagggcatccatcaaatttttggagcagctttcaaatcattgtttggaggaatgtcctggttctcacaaattctcattggaacgttgctgatgtggttgggtctgaacacaaagaatggatctatttcccttatgtgcttggccttagggggagtgttgatcttcttatccacagccgtctctgctgatgtggggtgctcggtggacttctcaaagaaggagacgagatgcggtacaggggtgttcgtctataacgacgttgaagcctggagggacaggtacaagtaccatcctgactccccccgtagattggcagcagcagtcaagcaagcctgggaagatggtatctgcgggatctcctctgtttcaagaatggaaaacatcatgtggagatcagtagaaggggagctcaacgcaatcctggaagagaatggagttcaactgacggtcgttgtgggatctgtaaaaaaccccatgtggagaggtccacagagattgcccgtgcctgtgaacgagctgccccacggctggaaggcttgggggaaatcgtatttcgtcagagcagcaaagacaaataacagctttgtcgtggatggtgacacactgaaggaatgcccactcaaacatagagcatggaacagctttcttgtggaggatcatgggttcggggtatttcacactagtgtctggctcaaggttagagaagattattcattagagtgtgatccagccgttattggaacagctgttaagggaaaggaggctgtacacagtgatctaggctactggattgagagtgagaagaatgacacatggaggctgaagagggcccatctgatcgagatgaaaacatgtgaatggccaaagtcccacacattgtggacagatggaatagaagagagtgatctgatcatacccaagtctttagctgggccactcagccatcacaataccagagagggctacaggacccaaatgaaagggccatggcacagtgaagagcttgaaattcggtttgaggaatgcccaggcactaaggtccacgtggaggaaacatgtggaacaagaggaccatctctgagatcaaccactgcaagcggaagggtgatcgaggaatggtgctgcagggagtgcacaatgcccccactgtcgttccgggctaaagatggctgttggtatggaatggagataaggcccaggaaagaaccagaaagcaacttagtaaggtcaatggtgactgcaggatcaactgatcacatggaccacttctcccttggagtgcttgtgatcctgctcatggtgcaggaagggctgaagaagagaatgaccacaaagatcatcataagcacatcaatggcagtgctggtagctatgatcctgggaggattttcaatgagtgacctggctaagcttgcaattttgatgggtgccaccttcgcggaaatgaacactggaggagatgtagctcatctggcgctgatagcggcattcaaagtcagaccagcgttgctggtatctttcatcttcagagctaattggacaccccgtgaaagcatgctgctggccttggcctcgtgtcttttgcaaactgcgatctccgccttggaaggcgacctgatggttctcatcaatggttttgctttggcctggttggcaatacgagcgatggttgttccacgcactgataacatcaccttggcaatcctggctgctctgacaccactggcccggggcacactgcttgtggcgtggagagcaggccttgctacttgcggggggtttatgctcctctctctgaagggaaaaggcagtgtgaagaagaacttaccatttgtcatggccctgggactaaccgctgtgaggctggtcgaccccatcaacgtggtgggactgctgttgctcacaaggagtgggaagcggagctggccccctagcgaagtactcacagctgttggcctgatatgcgcattggctggagggttcgccaaggcagatatagagatggctgggcccatggccgcggtcggtctgctaattgtcagttacgtggtctcaggaaagagtgtggacatgtacattgaaagagcaggtgacatcacatgggaaaaagatgcggaagtcactggaaacagtccccggctcgatgtggcgctagatgagagtggtgatttctccctggtggaggatgacggtccccccatgagagagatcatactcaaggtggtcctgatgaccatctgtggcatgaacccaatagccataccctttgcagctggagcgtggtacgtatacgtgaagactggaaaaaggagtggtgctctatgggatgtgcctgctcccaaggaagtaaaaaagggggagaccacagatggagtgtacagagtaatgactcgtagactgctaggttcaacacaagttggagtgggagttatgcaagagggggtctttcacactatgtggcacgtcacaaaaggatccgcgctgagaagcggtgaagggagacttgatccatactggggagatgtcaagcaggatctggtgtcatactgtggtccatggaagctagatgccgcctgggatgggcacagcgaggtgcagctcttggccgtgccccccggagagagagcgaggaacatccagactctgcccggaatatttaagacaaaggatggggacattggagcggttgcgctggattacccagcaggaacttcaggatctccaatcctagacaagtgtgggagagtgataggactttatggcaatggggtcgtgatcaaaaacgggagttatgttagtgccatcacccaagggaggagggaggaagagactcctgttgagtgcttcgagccctcgatgctgaagaagaagcagctaactgtcttagacttgcatcctggagctgggaaaaccaggagagttcttcctgaaatagtccgtgaagccataaaaacaagactccgtactgtgatcttagctccaaccagggttgtcgctgctgaaatggaggaggcccttagagggcttccagtgcgttatatgacaacagcagtcaatgtcacccactctggaacagaaatcgtcgacttaatgtgccatgccaccttcacttcacgtctactacagccaatcagagtccccaactataatctgtatattatggatgaggcccacttcacagatccctcaagtatagcagcaagaggatacatttcaacaagggttgagatgggcgaggcggctgccatcttcatgaccgccacgccaccaggaacccgtgacgcatttccggactccaactcaccaattatggacaccgaagtggaagtcccagagagagcctggagctcaggctttgattgggtgacggatcattctggaaaaacagtttggtttgttccaagcgtgaggaacggcaatgagatcgcagcttgtctgacaaaggctggaaaacgggtcatacagctcagcagaaagacttttgagacagagttccagaaaacaaaacatcaagagtgggactttgtcgtgacaactgacatttcagagatgggcgccaactttaaagctgaccgtgtcatagattccaggagatgcctaaagccggtcatacttgatggcgagagagtcattctggctggacccatgcctgtcacacatgccagcgctgcccagaggagggggcgcataggcaggaatcccaacaaacctggagatgagtatctgtatggaggtgggtgcgcagagactgacgaagaccatgcacactggcttgaagcaagaatgctccttgacaatatttacctccaagatggcctcatagcctcgctctatcgacctgaggccgacaaagtagcagccattgagggagagttcaagcttaggacggagcaaaggaagacctttgtggaactcatgaaaagaggagatcttcctgtttggctggcctatcaggttgcatctgccggaataacctacacagatagaagatggtgctttgatggcacgaccaacaacaccataatggaagacagtgtgccggcagaggtgtggaccagacacggagagaaaagagtgctcaaaccgaggtggatggacgccagagtttgttcagatcatgcggccctgaagtcattcaaggagtttgccgctgggaaaagaggagcggcttttggagtgatggaagccctgggaacactgccaggacacatgacagagagattccaggaagccattgacaacctcgctgtgctcatgcgggcagagactggaagcaggccttacaaagccgcggcggcccaattgccggagaccctagagaccataatgcttttggggttgctgggaacagtctcgctgggaatcttcttcgtcttgatgaggaacaagggcatagggaagatgggctttggaatggtgactcttggggccagcgcatggctcatgtggctctcggaaattgagccagccagaattgcatgtgtcctcattgttgtgttcctattgctggtggtgctcatacctgagccagaaaagcaaagatctccccaggacaaccaaatggcaatcatcatcatggtagcagtaggtcttctgggcttgattaccgccaatgaactcggatggttggagagaacaaagagtgacctaagccatctaatgggaaggagagaggagggggcaaccataggattctcaatggacattgacctgcggccagcctcagcttgggccatctatgctgccttgacaactttcattaccccagccgtccaacatgcagtgaccacctcatacaacaactactccttaatggcgatggccacgcaagctggagtgttgtttggcatgggcaaagggatgccattctacgcatgggactttggagtcccgctgctaatgataggttgctactcacaattaacacccctgaccctaatagtggccatcattttgctcgtggcgcactacatgtacttgatcccagggctgcaggcagcagctgcgcgtgctgcccagaagagaacggcagctggcatcatgaagaaccctgttgtggatggaatagtggtgactgacattgacacaatgacaattgacccccaagtggagaaaaagatgggacaggtgctactcatagcagtagccgtctccagcgccatactgtcgcggaccgcctgggggtggggggaggctggggctctgatcacagccgcaacttccactttgtgggaaggctctccgaacaagtactggaactcctctacagccacttcactgtgtaacatttttaggggaagttacttggctggagcttctctaatctacacagtaacaagaaacgctggcttggtcaagagacgtgggggtggaacaggagagaccctgggagagaaatggaaggcccgcttgaaccagatgtcggccctggagttctactcctacaaaaagtcaggcatcaccgaggtgtgcagagaagaggcccgccgcgccctcaaggacggtgtggcaacgggaggccatgctgtgtcccgaggaagtgcaaagctgagatggttggtggagcggggatacctgcagccctatggaaaggtcattgatcttggatgtggcagagggggctggagttactacgtcgccaccatccgcaaagttcaagaagtgaaaggatacacaaaaggaggccctggtcatgaagaacccgtgttggtgcaaagctatgggtggaacatagtccgtcttaagagtggggtggacgtctttcatatggcggctgagccgtgtgacacgttgctgtgtgacataggtgagtcatcatctagtcctgaagtggaagaagcacggacgctcagagtcctctccatggtgggggattggcttgaaaaaagaccaggagccttttgtataaaagtgttgtgcccatacaccagcactatgatggaaaccctggagcgactgcagcgtaggtatgggggaggactggtcagagtgccactctcccgcaactctacacatgagatgtactgggtctctggagcgaaaagcaacaccataaaaagtgtgtccaccacgagccagctcctcttggggcgcatggacgggcctaggaggccagtgaaatatgaggaggatgtgaatctcggctctggcacgcgggctgtggtaagctgcgctgaagctcccaacatgaagatcattggtaaccgcattgaaaggatccgcagtgagcacgcggaaacgtggttctttgacgagaaccacccatataggacatgggcttaccatggaagctatgaggcccccacacaagggtcagcgtcctctctaataaacggggttgtcaggctcctgtcaaaaccctgggatgtggtgactggagtcacaggaatagccatgaccgacaccacaccgtatggtcagcaaagagttttcaaggaaaaagtggacactagggtgccagacccccaagaaggcactcgtcaggttatgagcatggtctcttcctggttgtggaaagagctaggcaaacacaaacggccacgagtctgcaccaaagaagagttcatcaacaaggttcgtagcaatgcagcattaggggcaatatttgaagaggaaaaagagtggaagactgcagtggaagctgtgaacgatccaaggttctgggctctagtggacaaggaaagagagcaccacctgagaggagagtgccagagctgtgtgtacaacatgatgggaaaaagagaaaagaaacaaggggaatttggaaaggccaagggcagccgcgccatctggtatatgtggctaggggctagatttctagagttcgaagcccttggattcttgaacgaggatcactggatggggagagagaactcaggaggtggtgttgaagggctgggattacaaagactcggatatgtcctagaagagatgagtcgtataccaggaggaaggatgtatgcagatgacactgctggctgggacacccgcattagcaggtttgatctggagaatgaagctctaatcaccaaccaaatggagaaagggcacagggccttggcattggccataatcaagtacacataccaaaacaaagtggtaaaggtccttagaccagctgaaaaagggaaaacagttatggacattatttcgagacaagaccaaagggggagcggacaagttgtcacttacgctcttaacacatttaccaacctagtggtgcaactcattcggaatatggaggctgaggaagttctagagatgcaagacttgtggctgctgcggaggtcagagaaagtgaccaactggttgcagagcaacggatgggataggctcaaacgaatggcagtcagtggagatgattgcgttgtgaagccaattgatgataggtttgcacatgccctcaggttcttgaatgatatgggaaaagttaggaaggacacacaagagtggaaaccctcaactggatgggacaactgggaagaagttccgttttgctcccaccacttcaacaagctccatctcaaggacgggaggtccattgtggttccctgccgccaccaagatgaactgattggccgggcccgcgtctctccaggggcgggatggagcatccgggagactgcttgcctagcaaaatcatatgcgcaaatgtggcagctcctttatttccacagaagggacctccgactgatggccaatgccatttgttcatctgtgccagttgactgggttccaactgggagaactacctggtcaatccatggaaagggagaatggatgaccactgaagacatgcttgtggtgtggaacagagtgtggattgaggagaacgaccacatggaagacaagaccccagttacgaaatggacagacattccctatttgggaaaaagggaagacttgtggtgtggatctctcatagggcacagaccgcgcaccacctgggctgagaacattaaaaacacagtcaacatggtgcgcaggatcataggtgatgaagaaaagtacatggactacctatccacccaagttcgctacttgggtgaagaagggtctacacctggagtgctgtaagcaccaatcttaatgttgtcaggcctgctagtcagccacagcttggggaaagctgtgcagcctgtgacccccccaggagaagctgggaaaccaagcctatagtcaggccgagaacgccatggcacggaagaagccatgctgcctgtgagcccctcagaggacactgagtcaaaaaaccccacgcgcttggaggcgcaggatgggaaaagaaggtggcgaccttccccacccttcaatctggggcctgaactggagatcagctgtggatctccagaagagggactagtggttagaggagaccccccggaaaacgcaaaacagcatattgacgctgggaaagaccagagactccatgagtttccaccacgctggccgccaggcacagatcgccgaatagcggcggccggtgtggggaaatccatgggtct

SEQ ID NO: 14 - protein, 3423 aa, Zika virus strain PRVABC59
MKNPKKKSGGFRIVNMLKRGVARVSPFGGLKRLPAGLLLGHGPIRMVLAILAFLRFTAIKPSLGLINRWGSVGKKEAMETIKKFKKDLAAMLRIINARKEKKRRGADTSVGIVGLLLTTAMAAEVTRRGSAYYMYLDRNDAGEAISFPTTLGMNKCYIQIMDLGHMCDATMSYECPMLDEGVEPDDVDCWCNTTSTWVVYGTCHHKKGEARRSRRAVTLPSHSTRKLQTRSQTWLESREYTKHLIRVENWIFRNPGFALAAAAIAWLLGSSTSQKVIYLVMILLIAPAYSIRCIGVSNRDFVEGMSGGTWVDVVLEHGGCVTVMAQDKPTVDIELVTTTVSNMAEVRSYCYEASISDMASDSRCPTQGEAYLDKQSDTQYVCKRTLVDRGWGNGCGLFGKGSLVTCAKFACSKKMTGKSIQPENLEYRIMLSVHGSQHSGMIVNDTGHETDENRAKVEITPNSPRAEATLGGFGSLGLDCEPRTGLDFSDLYYLTMNNKHWLVHKEWFHDIPLPWHAGADTGTPHWNNKEALVEFKDAHAKRQTVVVLGSQEGAVHTALAGALEAEMDGAKGRLSSGHLKCRLKMDKLRLKGVSYSLCTAAFTFTKIPAETLHGTVTVEVQYAGTDGPCKVPAQMAVDMQTLTPVGRLITANPVITESTENSKMMLELDPPFGDSYIVIGVGEKKITHHWHRSGSTIGKAFEATVRGAKRMAVLGDTAWDFGSVGGALNSLGKGIHQIFGAAFKSLFGGMSWFSQILIGTLLMWLGLNTKNGSISLMCLALGGVLIFLSTAVSADVGCSVDFSKKETRCGTGVFVYNDVEAWRDRYKYHPDSPRRLAAAVKQAWEDGICGISSVSRMENIMWRSVEGELNAILEENGVQLTVVVGSVKNPMWRGPQRLPVPVNELPHGWKAWGKSYFVRAAKTNNSFVVDGDTLKECPLKHRAWNSFLVEDHGFGVFHTSVWLKVREDYSLECDPAVIGTAVKGKEAVHSDLGYWIESEKNDTWRLKRAHLIEMKTCEWPKSHTLWTDGIEESDLIIPKSLAGPLSHHNTREGYRTQMKGPWHSEELEIRFEECPGTKVHVEETCGTRGPSLRSTTASGRVIEEWCCRECTMPPLSFRAKDGCWYGMEIRPRKEPESNLVRSMVTAGSTDHMDHFSLGVLVILLMVQEGLKKRMTTKIIISTSMAVLVAMILGGFSMSDLAKLAILMGATFAEMNTGGDVAHLALIAAFKVRPALLVSFIFRANWTPRESMLLALASCLLQTAISALEGDLMVLINGFALAWLAIRAMVVPRTDNITLAILAALTPLARGTLLVAWRAGLATCGGFMLLSLKGKGSVKKNLPFVMALGLTAVRLVDPINVVGLLLLTRSGKRSWPPSEVLTAVGLICALAGGFAKADIEMAGPMAAVGLLIVSYVVSGKSVDMYIERAGDITWEKDAEVTGNSPRLDVALDESGDFSLVEDDGPPMREIILKVVLMTICGMNPIAIPFAAGAWYVYVKTGKRSGALWDVPAPKEVKKGETTDGVYRVMTRRLLGSTQVGVGVMQEGVFHTMWHVTKGSALRSGEGRLDPYWGDVKQDLVSYCGPWKLDAAWDGHSEVQLLAVPPGERARNIQTLPGIFKTKDGDIGAVALDYPAGTSGSPILDKCGRVIGLYGNGVVIKNGSYVSAITQGRREEETPVECFEPSMLKKKQLTVLDLHPGAGKTRRVLPEIVREAIKTRLRTVILAPTRVVAAEMEEALRGLPVRYMTTAVNVTHSGTEIVDLMCHATFTSRLLQPIRVPNYNLYIMDEAHFTDPSSIAARGYISTRVEMGEAAAIFMTATPPGTRDAFPDSNSPIMDTEVEVPERAWSSGFDWVTDHSGKTVWFVPSVRNGNEIAACLTKAGKRVIQLSRKTFETEFQKTKHQEWDFVVTTDISEMGANFKADRVIDSRRCLKPVILDGERVILAGPMPVTHASAAQRRGRIGRNPNKPGDEYLYGGGCAETDEDHAHWLEARMLLDNIYLQDGLIASLYRPEADKVAAIEGEFKLRTEQRKTFVELMKRGDLPVWLAYQVASAGITYTDRRWCFDGTTNNTIMEDSVPAEVWTRHGEKRVLKPRWMDARVCSDHAALKSFKEFAAGKRGAAFGVMEALGTLPGHMTERFQEAIDNLAVLMRAETGSRPYKAAAAQLPETLETIMLLGLLGTVSLGIFFVLMRNKGIGKMGFGMVTLGASAWLMWLSEIEPARIACVLIVVFLLLVVLIPEPEKQRSPQDNQMAIIIMVAVGLLGLITANELGWLERTKSDLSHLMGRREEGATIGFSMDIDLRPASAWAIYAALTTFITPAVQHAVTTSYNNYSLMAMATQAGVLFGMGKGMPFYAWDFGVPLLMIGCYSQLTPLTLIVAIILLVAHYMYLIPGLQAAAARAAQKRTAAGIMKNPVVDGIVVTDIDTMTIDPQVEKKMGQVLLIAVAVSSAILSRTAWGWGEAGALITAATSTLWEGSPNKYWNSSTATSLCNIFRGSYLAGASLIYTVTRNAGLVKRRGGGTGETLGEKWKARLNQMSALEFYSYKKSGITEVCREEARRALKDGVATGGHAVSRGSAKLRWLVERGYLQPYGKVIDLGCGRGGWSYYVATIRKVQEVKGYTKGGPGHEEPVLVQSYGWNIVRLKSGVDVFHMAAEPCDTLLCDIGESSSSPEVEEARTLRVLSMVGDWLEKRPGAFCIKVLCPYTSTMMETLERLQRRYGGGLVRVPLSRNSTHEMYWVSGAKSNTIKSVSTTSQLLLGRMDGPRRPVKYEEDVNLGSGTRAVVSCAEAPNMKIIGNRIERIRSEHAETWFFDENHPYRTWAYHGSYEAPTQGSASSLINGVVRLLSKPWDVVTGVTGIAMTDTTPYGQQRVFKEKVDTRVPDPQEGTRQVMSMVSSWLWKELGKHKRPRVCTKEEFINKVRSNAALGAIFEEEKEWKTAVEAVNDPRFWALVDKEREHHLRGECQSCVYNMMGKREKKQGEFGKAKGSRAIWYMWLGARFLEFEALGFLNEDHWMGRENSGGGVEGLGLQRLGYVLEEMSRIPGGRMYADDTAGWDTRISRFDLENEALITNQMEKGHRALALAIIKYTYQNKVVKVLRPAEKGKTVMDIISRQDQRGSGQVVTYALNTFTNLVVQLIRNMEAEEVLEMQDLWLLRRSEKVTNWLQSNGWDRLKRMAVSGDDCVVKPIDDRFAHALRFLNDMGKVRKDTQEWKPSTGWDNWEEVPFCSHHFNKLHLKDGRSIVVPCRHQDELIGRARVSPGAGWSIRETACLAKSYAQMWQLLYFHRRDLRLMANAICSSVPVDWVPTGRTTWSIHGKGEWMTTEDMLVVWNRVWIEENDHMEDKTPVTKWTDIPYLGKREDLWCGSLIGHRPRTTWAENIKNTVNMVRRIIGDEEKYMDYLSTQVRYLGEEGSTPGVL

SEQ ID NO: 15 - DNA, 10768 bp, Artificial Sequence
  Synthetic construct
agttgttagtctacgtggaccgacaaagacagattctttgagggagctaagctcaacgtagttctaacagttttttaattagagagcagatctctgatgaataaccaacggaaaaaggcgaaaaacacgcctttcaatatgctgaaacgcgagagaaaccgcgtgtcgactgtgcaacagctgacaaagagattctcacttggaatgctgcagggacgaggaccattaaaactgttcatggccctggtggcgttccttcgtttcctaacaatcccaccaacagcagggatattgaagagatggggaacaattaaaaaatcaaaagctattaatgttttgagagggttcaggaaagagattggaaggatgctgaacatcttgaataggagacgcagatccgcgggtactagtgtcggaattgttggcctcctgctgaccacagctatggcagcggaggtcactagacgtgggagtgcatactatatgtacttggacagaaacgatgctggggaggccatatcttttccaaccacattggggatgaataagtgttatatacagatcatggatcttggacacatgtgtgatgccaccatgagctatgaatgccctatgctggatgagggggtggaaccagatgacgtcgattgttggtgcaacacgacgtcaacttgggttgtgtacggaacctgccatcacaaaaaaggtgaagcacggagaagtagaagagctgtgacgctcccctcccattccactaggaagctgcaaacgcggtcgcaaacctggttggaatcaagagaatacacaaagcacttgattagagtcgaaaattggatattcaggaaccctggcttcgcgttagcagcagctgccatcgcttggcttttgggaagctcaacgagccaaaaagtcatatacttggtcatgatactgctgattgccccggcatacagcatcaggtgcataggagtcagcaatagggactttgtggaaggtatgtcaggtgggacttgggttgatattgtcttggaacatggaggttgtgtcaccgtaatggcacaggacaaaccgactgtcgacatagagctggttacaacaacagtcagcaacatggcggaggtaagatcctactgctatgaggcatcaatatcagacatggcttcggacagccgctgcccaacacaaggtgaagcctaccttgacaagcaatcagacactcaatatgtctgcaaaagaacgttagtggacagaggctggggaaatggatgtggactttttggcaaagggagtctggtgacatgcgctaagtttgcatgctccaagaaaatgaccgggaagagcatccagccagagaatctggagtaccggataatgctgtcagttcatggctcccagcacagtgggatgatcgttaatgacacaggacatgaaactgatgagaatagagcgaaggttgagataacgcccaattcaccaagagccgaagccaccctggggggttttggaagcctaggacttgattgtgaaccgaggacaggccttgacttttcagatttgtattacttgactatgaataacaagcactggttggttcacaaggagtggttccacgacattccattaccttggcacgctggggcagacaccggaactccacactggaacaacaaagaagcactggtagagttcaaggacgcacatgccaaaaggcaaactgtcgtggttctagggagtcaagaaggagcagttcacacggcccttgctggagctctggaggctgagatggatggtgcaaagggaaggctgtcctctggccacttgaaatgtcgcctgaaaatggataaacttagattgaagggcgtgtcatactccttgtgtaccgcagcgttcacattcaccaagatcccggctgaaacactgcacgggacagtcacagtggaggtacagtacgcagggacagatggaccttgcaaggttccagctcagatggcggtggacatgcaaactctgaccccagttgggaggttgataaccgctaaccccgtaatcactgaaagcactgagaactctaagatgatgctggaacttgatccaccatttggggactcttacattgtcataggagtcggggagaagaagatcacccaccactggcacaggagtggcagcaccattggaaaagcatttgaagccactgtgagaggtgccaagagaatggcagtcttgggagacacagcctgggactttggatcagttggaggcgctctcaactcattgggcaagggcatccatcaaatttttggagcagctttcaaatcattgtttggaggaatgtcctggttctcaagaattctcattggaacgttgctgatgtggttgggtctgaacacaaagaatggatctatttcccttatgtgcttggccgccggctttgtgacactgtatttgggggtcatggtgcaggccgatagtggttgcgttgtgagctggaaaaacaaagaactgaaatgtggcagtgggattttcatcacagacaacgtgcacacatggacagaacaatacaagttccaaccagaatccccttcaaaactagcttcagctatccagaaagcccatgaagagggcatttgtggaatccgctcagtaacaagactggagaatctgatgtggaaacaaataacaccagaattgaatcacattctatcagaaaatgaggtgaagttaactattatgacaggagacatcaaaggaatcatgcaggcaggaaaacgatctctgcggcctcagcccactgagctgaagtattcatggaaaacatggggcaaagcaaaaatgctctctacagagtctcataaccagacctttctcattgatggccccgaaacagcagaatgccccaacacaaatagagcttggaattcgttggaagttgaagactatggctttggagtattcaccaccaatatatggctaaaattgaaagaaaaacaggatgtattctgcgactcaaaactcatgtcagcggccataaaagacaacagagccgtccatgccgatatgggttattggatagaaagtgcactcaatgacacatggaagatagagaaagcctctttcattgaagttaaaaactgccactggccaaaatcacacaccctctggagcaatggagtgctagaaagtgagatgataattccaaagaatctcgctggaccagtgtctcaacacaactatagaccaggctaccatacacaaataacaggaccatggcatctaggtaagcttgagatggactttgatttctgtgatggaacaacagtggtagtgactgaggactgcggaaatagaggaccctctttgagaacaaccactgcctctggaaaactcataacagaatggtgctgccgatcttgcacattaccaccgctaagatacagaggtgaggatgggtgctggtacgggatggaaatcagaccattgaaggagaaagaagagaatttggtcaactccttggtcacagctggacatgggcaggtcgacaacttttcactaggagtcttgggaatggcattgttcctggaggaaatgcttaggacccgagtaggaacgaaacatgcaatactactagttgcagtttcttttgtgacattgatcacagggaacatgtcctttagagacctgggaagagtgatggttatggtaggcgccactatgacggatgacataggtatgggcgtgacttatcttgccctactagcagccttcaaagtcagaccaacttttgcagctggactactcttgagaaagctgacctccaatgaattgatgatgactactataggaattgtactcctctcccagagcaccataccagagaccattcttgagttgactgatgcgttagccttaggcatgatggtcctcaaaatggtgagaaatatggaaaagtatcaattggcagtgactatcatggctatcttgtgcgtcccaaacgcagtgatattacaaaacgcatggaaagtgagttgcacaatattggcagtggtgtccgtttccccactgctcttaacatcctcacagcaaaaaacagattggataccattagcattgacgatcaaaggtctcaatccaacagctatttttctaacaaccctctcaagaaccagcaagaaaaggagctggccattaaatgaggctatcatggcagtcgggatggtgagcattttagccagttctctcctaaaaaatgatattcccatgacaggaccattagtggctggagggctcctcactgtgtgctacgtgctcactggacgatcggccgatttggaactggagagagcagccgatgtcaaatgggaagaccaggcagagatatcaggaagcagtccaatcctgtcaataacaatatcagaagatggtagcatgtcgataaaaaatgaagaggaagaacaaacactgaccatactcattagaacaggattgctggtgatctcaggactttttcctgtatcaataccaatcacggcagcagcatggtacctgtgggaagtgaagaaacaacgggccggagtattgtgggatgttccttcacccccacccatgggaaaggctgaactggaagatggagcctatagaattaagcaaaaagggattcttggatattcccagatcggagccggagtttacaaagaaggaacattccatacaatgtggcatgtcacacgtggcgctgttctaatgcataaaggaaagaggattgaaccatcatgggcggacgtcaagaaagacctaatatcatatggaggaggctggaagttagaaggagaatggaaggaaggagaagaagtccaggtattggcactggagcctggaaaaaatccaagagccgtccaaacgaaacctggtcttttcaaaaccaacgccggaacaataggtgctgtatctctggacttttctcctggaacgtcaggatctccaattatcgacaaaaaaggaaaagttgtgggtctttatggtaatggtgttgttacaaggagtggagcatatgtgagtgctatagcccagactgaaaaaagcattgaagacaacccagagatcgaagatgacattttccgaaagagaagactgaccatcatggacctccacccaggagcgggaaagacgaagagataccttccggccatagtcagagaagctataaaacggggtttgagaacattaatcttggcccccactagagttgtggcagctgaaatggaggaagcccttagaggacttccaataagataccagaccccagccatcagagctgagcacaccgggcgggagattgtggacctaatgtgtcatgccacatttaccatgaggctgctatcaccagttagagtgccaaactacaacctgattatcatggacgaagcccatttcacagacccagcaagtatagcagctagaggatacatctcaactcgagtggagatgggtgaggcagctgggatttttatgacagccactcccccgggaagcagagacccatttcctcagagcaatgcaccaatcatagatgaagaaagagaaatccctgaacgttcgtggaattccggacatgaatgggtcacggattttaaagggaagactgtttggttcgttccaagtataaaagcaggaaatgatatagcagcttgcctgaggaaaaatggaaagaaagtgatacaactcagtaggaagacctttgattctgagtatgtcaagactagaaccaatgattgggacttcgtggttacaactgacatttcagaaatgggtgccaatttcaaggctgagagggttatagaccccagacgctgcatgaaaccagtcatactaacagatggtgaagagcgggtgattctggcaggacctatgccagtgacccactctagtgcagcacaaagaagagggagaataggaagaaatccaaaaaatgagaatgaccagtacatatacatgggggaacctctggaaaatgatgaagactgtgcacactggaaagaagctaaaatgctcctagataacatcaacacgccagaaggaatcattcctagcatgttcgaaccagagcgtgaaaaggtggatgccattgatggcgaataccgcttgagaggagaagcaaggaaaacctttgtagacttaatgagaagaggagacctaccagtctggttggcctacagagtggcagctgaaggcatcaactacgcagacagaaggtggtgttttgatggagtcaagaacaaccaaatcctagaagaaaacgtggaagttgaaatctggacaaaagaaggggaaaggaagaaattgaaacccagatggttggatgctaggatctattctgacccactggcgctaaaagaatttaaggaatttgcagccggaagaaagtctctgaccctgaacctaatcacagaaatgggtaggctcccaaccttcatgactcagaaggcaagaaacgcactggacaacttagcagtgctgcacacggctgaggcaggtggaagggcgtacaaccatgctctcagtgaactgccggagaccctggagacattgcttttactgacacttctggctacagtcacgggagggatctttttattcttgatgagcggaaggggcatagggaagatgaccctgggaatgtgctgcataatcacggctagcatcctcctatggtacgcacaaatacagccacactggatagcagcttcaataatactggagttttttctcatagttttgcttattccagaacctgaaaaacagagaacaccccaagacaaccaactgacctacgttgtcatagccatcctcacagtggtggccgcaaccatggcaaacgagatgggtttcctagaaaaaacgaagaaagatctcggattgggaagcattgcaacccagcaacccgagagcaacatcctggacatagatctacgtcctgcatcagcatggacgctgtatgccgtggccacaacatttgttacaccaatgttgagacatagcattgaaaattcctcagtgaatgtgtccctaacagctatagccaaccaagccacagtgttaatgggtctcgggaaaggatggccattgtcaaagatggacatcggagttccccttctcgccattggatgctactcacaagtcaaccccataactctcacagcagctcttttcttattggtagcacattatgccatcatagggccaggactccaagcaaaagcaaccagagaagctcagaaaagagcagcggcgggcatcatgaaaaacccaactgtcgatggaataacagtgattgacctagatccaataccttatgatccaaagtttgaaaagcagttgggacaagtaatgctcctagtcctctgcgtgactcaagtattgatgatgaggactacatgggctctgtgtgaggctttaaccttagctaccgggcccatctccacattgtgggaaggaaatccagggaggttttggaacactaccattgcggtgtcaatggctaacatttttagagggagttacttggccggagctggacttctcttttctattatgaagaacacaaccaacacaagaaggggaactggcaacataggagagacgcttggagagaaatggaaaagccgattgaacgcattgggaaaaagtgaattccagatctacaagaaaagtggaatccaggaagtggatagaaccttagcaaaagaaggcattaaaagaggagaaacggaccatcacgctgtgtcgcgaggctcagcaaaactgagatggttcgttgagagaaacatggtcacaccagaagggaaagtagtggacctcggttgtggcagaggaggctggtcatactattgtggaggactaaagaatgtaagagaagtcaaaggcctaacaaaaggaggaccaggacacgaagaacccatccccatgtcaacatatgggtggaatctagtgcgtcttcaaagtggagttgacgttttcttcatcccgccagaaaagtgtgacacattattgtgtgacataggggagtcatcaccaaatcccacagtggaagcaggacgaacactcagagtccttaacttagtagaaaattggttgaacaacaacactcaattttgcataaaggttctcaacccatatatgccctcagtcatagaaaaaatggaagcactacaaaggaaatatggaggagccttagtgaggaatccactctcacgaaactccacacatgagatgtactgggtatccaatgcttccgggaacatagtgtcatcagtgaacatgatttcaaggatgttgatcaacagatttacaatgagatacaagaaagccacttacgagccggatgttgacctcggaagcggaacccgtaacatcgggattgaaagtgagataccaaacctagatataattgggaaaagaatagaaaaaataaagcaagagcatgaaacatcatggcactatgaccaagaccacccatacaaaacgtgggcataccatggtagctatgaaacaaaacagactggatcagcatcatccatggtcaacggagtggtcaggctgctgacaaaaccttgggacgtcgtccccatggtgacacagatggcaatgacagacacgactccatttggacaacagcgcgtttttaaagagaaagtggacacgagaacccaagaaccgaaagaaggcacgaagaaactaatgaaaataacagcagagtggctttggaaagaattagggaagaaaaagacacccaggatgtgcaccagagaagaattcacaagaaaggtgagaagcaatgcagccttgggggccatattcactgatgagaacaagtggaagtcggcacgtgaggctgttgaagatagtaggttttgggagctggttgacaaggaaaggaatctccatcttgaaggaaagtgtgaaacatgtgtgtacaacatgatgggaaaaagagagaagaagctaggggaattcggcaaggcaaaaggcagcagagccatatggtacatgtggcttggagcacgcttcttagagtttgaagccctaggattcttaaatgaagatcactggttctccagagagaactccctgagtggagtggaaggagaagggctgcacaagctaggttacattctaagagacgtgagcaagaaagagggaggagcaatgtatgccgatgacaccgcaggatgggatacaagaatcacactagaagacctaaaaaatgaagaaatggtaacaaaccacatggaaggagaacacaagaaactagccgaggccattttcaaactaacgtaccaaaacaaggtggtgcgtgtgcaaagaccaacaccaagaggcacagtaatggacatcatatcgagaagagaccaaagaggtagtggacaagttggcacctatggactcaatactttcaccaatatggaagcccaactaatcagacagatggagggagaaggagtctttaaaagcattcagcacctaacaatcacagaagaaatcgctgtgcaaaactggttagcaagagtggggcgcgaaaggttatcaagaatggccatcagtggagatgattgtgttgtgaaacctttagatgacaggttcgcaagcgctttaacagctctaaatgacatgggaaagattaggaaagacatacaacaatgggaaccttcaagaggatggaatgattggacacaagtgcccttctgttcacaccatttccatgagttaatcatgaaagacggtcgcgtactcgttgttccatgtagaaaccaagatgaactgattggcagagcccgaatctcccaaggagcagggtggtctttgcgggagacggcctgtttggggaagtcttacgcccaaatgtggagcttgatgtacttccacagacgcgacctcaggctggcggcaaatgctatttgctcggcagtaccatcacattgggttccaacaagtcgaacaacctggtccatacatgctaaacatgaatggatgacaacggaagacatgctgacagtctggaacagggtgtggattcaagaaaacccatggatggaagacaaaactccagtggaatcatgggaggaaatcccatacttggggaaaagagaagaccaatggtgcggctcattgattgggttaacaagcagggccacctgggcaaagaacatccaagcagcaataaatcaagttagatcccttataggcaatgaagaatacacagattacatgccatccatgaaaagattcagaagagaagaggaagaagcaggagttctgtggtagaaagcaaaactaacatgaaacaaggctagaagtcaggtcggattaagccatagtacggaaaaaactatgctacctgtgagccccgtccaaggacgttaaaagaagtcaggccatcataaatgccatagcttgagtaaactatgcagcctgtagctccacctgagaaggtgtaaaaaatccgggaggccacaaaccatggaagctgtacgcatggcgtagtggactagcggttagaggagacccctcccttacaaatcgcagcaacaatgggggcccaaggcgagatgaagctgtagtctcgctggaaggactagaggttagaggagacccccccgaaacaaaaaacagcatattgacgctgggaaagaccagagatcctgctgtctcctcagcatcattccaggcacagaacgccagaaaatggaatggtgctgttgaatcaacaggttct

SEQ ID NO: 16 - protein, 3406 aa, Artificial Sequence
  Synthetic polypeptide
MNNQRKKAKNTPFNMLKRERNRVSTVQQLTKRFSLGMLQGRGPLKLFMALVAFLRFLTIPPTAGILKRWGTIKKSKAINVLRGFRKEIGRMLNILNRRRRSAGTSVGIVGLLLTTAMAAEVTRRGSAYYMYLDRNDAGEAISFPTTLGMNKCYIQIMDLGHMCDATMSYECPMLDEGVEPDDVDCWCNTTSTWVVYGTCHHKKGEARRSRRAVTLPSHSTRKLQTRSQTWLESREYTKHLIRVENWIFRNPGFALAAAAIAWLLGSSTSQKVIYLVMILLIAPAYSIRCIGVSNRDFVEGMSGGTWVDIVLEHGGCVTVMAQDKPTVDIELVTTTVSNMAEVRSYCYEASISDMASDSRCPTQGEAYLDKQSDTQYVCKRTLVDRGWGNGCGLFGKGSLVTCAKFACSKKMTGKSIQPENLEYRIMLSVHGSQHSGMIVNDTGHETDENRAKVEITPNSPRAEATLGGFGSLGLDCEPRTGLDFSDLYYLTMNNKHWLVHKEWFHDIPLPWHAGADTGTPHWNNKEALVEFKDAHAKRQTVVVLGSQEGAVHTALAGALEAEMDGAKGRLSSGHLKCRLKMDKLRLKGVSYSLCTAAFTFTKIPAETLHGTVTVEVQYAGTDGPCKVPAQMAVDMQTLTPVGRLITANPVITESTENSKMMLELDPPFGDSYIVIGVGEKKITHHWHRSGSTIGKAFEATVRGAKRMAVLGDTAWDFGSVGGALNSLGKGIHQIFGAAFKSLFGGMSWFSRILIGTLLMWLGLNTKNGSISLMCLAAGFVTLYLGVMVQADSGCVVSWKNKELKCGSGIFITDNVHTWTEQYKFQPESPSKLASAIQKAHEEGICGIRSVTRLENLMWKQITPELNHILSENEVKLTIMTGDIKGIMQAGKRSLRPQPTELKYSWKTWGKAKMLSTESHNQTFLIDGPETAECPNTNRAWNSLEVEDYGFGVFTTNIWLKLKEKQDVFCDSKLMSAAIKDNRAVHADMGYWIESALNDTWKIEKASFIEVKNCHWPKSHTLWSNGVLESEMIIPKNLAGPVSQHNYRPGYHTQITGPWHLGKLEMDFDFCDGTTVVVTEDCGNRGPSLRTTTASGKLITEWCCRSCTLPPLRYRGEDGCWYGMEIRPLKEKEENLVNSLVTAGHGQVDNFSLGVLGMALFLEEMLRTRVGTKHAILLVAVSFVTLITGNMSFRDLGRVMVMVGATMTDDIGMGVTYLALLAAFKVRPTFAAGLLLRKLTSNELMMTTIGIVLLSQSTIPETILELTDALALGMMVLKMVRNMEKYQLAVTIMAILCVPNAVILQNAWKVSCTILAVVSVSPLLLTSSQQKTDWIPLALTIKGLNPTAIFLTTLSRTSKKRSWPLNEAIMAVGMVSILASSLLKNDIPMTGPLVAGGLLTVCYVLTGRSADLELERAADVKWEDQAEISGSSPILSITISEDGSMSIKNEEEEQTLTILIRTGLLVISGLFPVSIPITAAAWYLWEVKKQRAGVLWDVPSPPPMGKAELEDGAYRIKQKGILGYSQIGAGVYKEGTFHTMWHVTRGAVLMHKGKRIEPSWADVKKDLISYGGGWKLEGEWKEGEEVQVLALEPGKNPRAVQTKPGLFKTNAGTIGAVSLDFSPGTSGSPIIDKKGKVVGLYGNGVVTRSGAYVSAIAQTEKSIEDNPEIEDDIFRKRRLTIMDLHPGAGKTKRYLPAIVREAIKRGLRTLILAPTRVVAAEMEEALRGLPIRYQTPAIRAEHTGREIVDLMCHATFTMRLLSPVRVPNYNLIIMDEAHFTDPASIAARGYISTRVEMGEAAGIFMTATPPGSRDPFPQSNAPIIDEEREIPERSWNSGHEWVTDFKGKTVWFVPSIKAGNDIAACLRKNGKKVIQLSRKTFDSEYVKTRTNDWDFVVTTDISEMGANFKAERVIDPRRCMKPVILTDGEERVILAGPMPVTHSSAAQRRGRIGRNPKNENDQYIYMGEPLENDEDCAHWKEAKMLLDNINTPEGIIPSMFEPEREKVDAIDGEYRLRGEARKTFVDLMRRGDLPVWLAYRVAAEGINYADRRWCFDGVKNNQILEENVEVEIWTKEGERKKLKPRWLDARIYSDPLALKEFKEFAAGRKSLTLNLITEMGRLPTFMTQKARDALDNLAVLHTAEAGGRAYNHALSELPETLETLLLLTLLATVTGGIFLFLMSGRGIGKMTLGMCCIITASILLWYAQIQPHWIAASIILEFFLIVLLIPEPEKQRTPQDNQLTYVVIAILTVVAATMANEMGFLEKTKKDLGLGSIATQQPESNILDIDLRPASAWTLYAVATTFVTPMLRHSIENSSVNVSLTAIANQATVLMGLGKGWPLSKMDIGVPLLAIGCYSQVNPITLTAALFLLVAHYAIIGPGLQAKATREAQKRAAAGIMKNPTVDGITVIDLDPIPYDPKFEKQLGQVMLLVLCVTQVLMMRTTWALCEALTLATGPISTLWEGNPGRFWNTTIAVSMANIFRGSYLAGAGLLFSIMKNTTNTRRGTGNIGETLGEKWKSRLNALGKSEFQIYKKSGIQEVDRTLAKEGIKRGETDHHAVSRGSAKLRWFVERNMVTPEGKVVDLGCGRGGWSYYCGGLKNVREVKGLTKGGPGHEEPIPMSTYGWNLVRLQSGVDVFFIPPEKCDTLLCDIGESSPNPTVEAGRTLRVLNLVENWLNNNTQFCIKVLNPYMPSVIEKMEALQRKYGGALVRNPLSRNSTHEMYWVSNASGNIVSSVNMISRMLINRFTMRYKKATYEPDVDLGSGTRNIGIESEIPNLDIIGKRIEKIKQEHETSWHYDQDHPYKTWAYHGSYETKQTGSASSMVNGVVRLLTKPWDVVPMVTQMAMTDTTPFGQQRVFKEKVDTRTQEPKEGTKKLMKITAEWLWKELGKKKTPRMCTREEFTRKVRSNAALGAIFTDENKWKSAREAVEDSRFWELVDKERNLHLEGKCETCVYNMMGKREKKLGEFGKAKGSRAIWYMWLGARFLEFEALGFLNEDHWFSRENSLSGVEGEGLHKLGYILRDVSKKEGGAMYADDTAGWDTRITLEDLKNEEMVTNHMEGEHKKLAEAIFKLTYQNKVVRVQRPTPRGTVMDIISRRDQRGSGQVGTYGLNTFTNMEAQLIRQMEGEGVFKSIQHLTITEEIAVQNWLARVGRERLSRMAISGDDCVVKPLDDRFASALTALNDMGKIRKDIQQWEPSRGWNDWTQVPFCSHHFHELIMKDGRVLVVPCRNQDELIGRARISQGAGWSLRETACLGKSYAQMWSLMYFHRRDLRLAANAICSAVPSHWVPTSRTTWSIHAKHEWMTTEDMLTVWNRVWIQENPWMEDKTPVESWEEIPYLGKREDQWCGSLIGLTSRATWAKNIQAAINQVRSLIGNEEYTDYMPSMKRFRREEEEAGVLW

SEQ ID NO: 17 - DNA, 10768 bp, Artificial Sequence
  Synthetic construct
agttgttagtctacgtggaccgacaaagacagattctttgagggagctaagctcaatgtagttctaacagttttttaattagagagcagatctctgatgaataaccaacggaaaaaggcgaaaaacacgcctttcaatatgctgaaacgcgagagaaaccgcgtgtcgactgtgcaacagctgacaaagagattctcacttggaatgctgcagggacgaggaccattaaaactgttcatggccctggtggcgttccttcgtttcctaacaatcccaccaacagcagggatattgaagagatggggaacaattaaaaaatcaaaagctattaatgttttgagagggttcaggaaagagattggaaggatgctgaacatcttgaataggagacgcagatccgcgggtactagtgtcggaattgttggcctcctgctgaccacagctatggcagcggaggtcactagacgtgggagtgcatactatatgtacttggacagaaacgatgctggggaggccatatcttttccaaccacattggggatgaataagtgttatatacagatcatggatcttggacacatgtgtgatgccaccatgagctatgaatgccctatgctggatgagggggtggaaccagatgacgtcgattgttggtgcaacacgacgtcaacttgggttgtgtacggaacctgccatcacaaaaaaggtgaagcacggagaagtagaagagctgtgacgctcccctcccattccactaggaagctgcaaacgcggtcgcaaacctggttggaatcaagagaatacacaaagcacttgattagagtcgaaaattggatattcaggaaccctggcttcgcgttagcagcagctgccatcgcttggcttttgggaagctcaacgagccaaaaagtcatatacttggtcatgatactgctgattgccccggcatacagcatcaggtgcataggagtcagcaatagggactttgtggaaggtatgtcaggtgggacttgggttgatattgtcttggaacatggaggttgtgtcaccgtaatggcacaggacaaaccgactgtcgacatagagctggttacaacaacagtcagcaacatggcggaggtaagatcctactgctatgaggcatcaatatcagacatggcttcggacagccgctgcccaacacaaggtgaagcctaccttgacaagcaatcagacactcaatatgtctgcaaaagaacgttagtggacagaggctggggaaatggatgtggactttttggcaaagggagtctggtgacatgcgctaagtttgcatgctccaagaaaatgaccgggaagagcatccagccagagaatctggagtaccggataatgctgtcagttcatggctcccagcacagtgggatgatcgttaatgacacaggacatgaaactgatgagaatagagcgaaggttgagataacgcccaattcaccaagagccgaagccaccctggggggttttggaagcctaggacttgattgtgaaccgaggacaggccttgacttttcagatttgtattacttgactatgaataacaagcactggttggttcacaaggagtggttccacgacattccattaccttggcacgctggggcagacaccggaactccacactggaacaacaaagaagcactggtagagttcaaggacgcacatgccaaaaggcaaactgtcgtggttctagggagtcaagaaggagcagttcacacggcccttgctggagctctggaggctgagatggatggtgcaaagggaaggctgtcctctggccacttgaaatgtcgcctgaaaatggataaacttagattgaagggcgtgtcatactccttgtgtaccgcagcgttcacattcaccaagatcccggctgaaacactgcacgggacagtcacagtggaggtacagtacgcagggacagatggaccttgcaaggttccagctcagatggcggtggacatgcaaactctgaccccagttgggaggttgataaccgctaaccccgtaatcactgaaagcactgagaactctaagatgatgctggaacttgatccaccatttggggactcttacattgtcataggagtcggggagaagaagatcacccaccactggcacaggagtggcagcaccattggaaaagcatttgaagccactgtgagaggtgccaagagaatggcagtcttgggagacacagcctgggactttggatcagttggaggcgctctcaactcattgggcaagggcatccatcaaatttttggagcagctttcaaatcattgtttggaggaatgtcctggttctcaagaattctcattggaacgttgctgatgtggttgggtctgaacacaaagaatggatctatttcccttatgtgcttggccgccggctttgtgacactgtatttgggagtcatggtgcaggccgatagtggttgcgttgtgagctggaaaaacaaagaactgaaatgtggcagtgggattttcatcacagacaacgtgcacacatggacagaacaatacaagttccaaccagaatccccttcaaaactagcttcagctatccagaaagcccatgaagaggacatttgtggaatccgctcagtaacaagactggagaatctgatgtggaaacaaataacaccagaattgaatcacattctatcagaaaatgaggtgaagttaactattatgacaggagacatcaaaggaatcatgcaggcaggaaaacgatctctgcggcctcagcccactgagctgaagtattcatggaaaacatggggcaaagcaaaaatgctctctacagagtctcataaccagacctttctcattgatggccccgaaacagcagaatgccccaacacaaatagagcttggaattcgttggaagttgaagactatggctttggagtattcaccaccaatatatggctaaaattgaaagaaaaacaggatgtattctgcgactcaaaactcatgtcagcggccataaaagacaacagagccgtccatgccgatatgggttattggatagaaagtgcactcaatgacacatggaagatagagaaagcctctttcattgaagttaaaaactgccactggccaaaatcacacaccctctggagcaatggagtgctagaaagtgagatgataattccaaagaatctcgctggaccagtgtctcaacacaactatagaccaggctaccatacacaaataacaggaccatggcatctaggtaagcttgagatggactttgatttctgtgatggaacaacagtggtagtgactgaggactgcggaaatagaggaccctctttgagaacaaccactgcctctggaaaactcataacagaatggtgctgccgatcttgcacattaccaccgctaagatacagaggtgaggatgggtgctggtacgggatggaaatcagaccattgaaggagaaagaagagaatttggtcaactccttggtcacagctggacatgggcaggtcgacaacttttcactaggagtcttgggaatggcattgttcctggaggaaatgcttaggacccgagtaggaacgaaacatgcaatactactagttgcagtttcttttgtgacattgatcacagggaacatgtcctttagagacctgggaagagtgatggttatggtaggcgccactatgacggatgacataggtatgggcgtgacttatcttgccctactagcagccttcaaagtcagaccaacttttgcagctggactactcttgagaaagctgacctccaatgaattgatgatgactactataggaattgtactcctctcccagagcaccataccagagaccattcttgagttgactgatgcgttagccttaggcatgatggtcctcaaaatggtgagaaatatggaaaagtatcaattggcagtgactatcatggctatcttgtgcgtcccaaacgcagtgatattacaaaacgcatggaaagtgagttgcacaatattggcagtggtgtccgtttccccactgttcttaacatcctcacagcaaaaaacagattggataccattagcattgacgatcaaaggtctcaatccaacagctatttttctaacaaccctctcaagaaccagcaagaaaaggagctggccattaaatgaggctatcatggcagtcgggatggtgagcattttagccagttctctcctaaaaaatgatattcccatgacaggaccattagtggctggagggctcctcactgtgtgctacgtgctcactggacgatcggccgatttggaactggagagagcagccgatgtcaaatgggaagaccaggcagagatatcaggaagcagtccaatcctgtcaataacaatatcagaagatggtagcatgtcgataaaaaatgaagaggaagaacaaacactgaccatactcattagaacaggattgctggtgatctcaggactttttcctgtatcaataccaatcacggcagcagcatggtacctgtgggaagtgaagaaacaacgggccggagtattgtgggatgttccttcacccccacccatgggaaaggctgaactggaagatggagcctatagaattaagcaaaaagggattcttggatattcccagatcggagccggagtttacaaagaaggaacattccatacaatgtggcatgtcacacgtggcgctgttctaatgcataaaggaaagaggattgaaccatcatgggcggacgtcaagaaagacctaatatcatatggaggaggctggaagttagaaggagaatggaaggaaggagaagaagtccaggtattggcactggagcctggaaaaaatccaagagccgtccaaacgaaacctggtcttttcaaaaccaacgccggaacaataggtgctgtatctctggacttttctcctggaacgtcaggatctccaattatcgacaaaaaaggaaaagttgtgggtctttatggtaatggtgttgttacaaggagtggagcatatgtgagtgctatagcccagactgaaaaaagcattgaagacaacccagagatcgaagatgacattttccgaaagagaagactgaccatcatggacctccacccaggagcgggaaagacgaagagataccttccggccatagtcagagaagctataaaacggggtttgagaacattaatcttggcccccactagagttgtggcagctgaaatggaggaagcccttagaggacttccaataagataccagaccccagccatcagagctgtgcacaccgggcgggagattgtggacctaatgtgtcatgccacatttaccatgaggctgctatcaccagttagagtgccaaactacaacctgattatcatggacgaagcccatttcacagacccagcaagtatagcagctagaggatacatctcaactcgagtggagatgggtgaggcagctgggatttttatgacagccactcccccgggaagcagagacccatttcctcagagcaatgcaccaatcatagatgaagaaagagaaatccctgaacgctcgtggaattccggacatgaatgggtcacggattttaaagggaagactgtttggttcgttccaagtataaaagcaggaaatgatatagcagcttgcctgaggaaaaatggaaagaaagtgatacaactcagtaggaagacctttgattctgagtatgtcaagactagaaccaatgattgggacttcgtggttacaactgacatttcagaaatgggtgccaatttcaaggctgagagggttatagaccccagacgctgcatgaaaccagtcatactaacagatggtgaagagcgggtgattctggcaggacctatgccagtgacccactctagtgcagcacaaagaagagggagaataggaagaaatccaaaaaatgagaatgaccagtacatatacatgggggaacctctggaaaatgatgaagactgtgcacactggaaagaagctaaaatgctcctagataacatcaacacgccagaaggaatcattcctagcatgttcgaaccagagcgtgaaaaggtggatgccattgatggcgaataccgcttgagaggagaagcaaggaaaacctttgtagacttaatgagaagaggagacctaccagtctggttggcctacagagtggcagctgaaggcatcaactacgcagacagaaggtggtgttttgatggagtcaagaacaaccaaatcctagaagaaaacgtggaagttgaaatctggacaaaagaaggggaaaggaagaaattgaaacccagatggttggatgctaggatctattctgacccactggcgctaaaagaatttaaggaatttgcagccggaagaaagtctctgaccctgaacctaatcacagaaatgggtaggctcccaaccttcatgactcagaaggcaagaaacgcactggacaacttagcagtgctgcacacggctgaggcaggtggaagggcgtacaaccatgctctcagtgaactgccggagaccctggagacattgcttttactgacacttctggctacagtcacgggagggatctttttattcttgatgagcgcaaggggcatagggaagatgaccctgggaatgtgctgcataatcacggctagcatcctcctatggtacgcacaaatacagccacactggatagcagcttcaataatactggagttttttctcatagttttgcttattccagaacctgaaaaacagagaacaccccaagacaaccaactgacctacgttgtcatagccatcctcacagtggtggccgcaaccatggcaaacgagatgggtttcctagaaaaaacgaagaaagatctcggattgggaagcattgcaacccagcaacccgagagcaacatcctggacatagatctacgtcctgcatcagcatggacgctgtatgccgtggccacaacatttgttacaccaatgttgagacatagcattgaaaattcctcagtgaatgtgtccctaacagctatagccaaccaagccacagtgttaatgggtctcgggaaaggatggccattgtcaaagatggacatcggagttccccttctcgccattggatgctactcacaagtcaaccccataactctcacagcagctcttttcttattggtagcacattatgccatcatagggccaggactccaagcaaaagcaaccagagaagctcagaaaagagcagcggcgggcatcatgaaaaacccaactgtcgatggaataacagtgattgacctagatccaataccttatgatccaaagtttgaaaagcagttgggacaagtaatgctcctagtcctctgcgtgactcaagtattgatgatgaggactacatgggctctgtgtgaggctttaaccttagctaccgggcccatctccacattgtgggaaggaaatccagggaggttttggaacactaccattgcggtgtcaatggctaacatttttagagggagttacttggccggagctggacttctcttttctattatgaagaacacaaccaacacaagaaggggaactggcaacataggagagacgcttggagagaaatggaaaagccgattgaacgcattgggaaaaagtgaattccagatctacaagaaaagtggaatccaggaagtggatagaaccttagcaaaagaaggcattaaaagaggagaaacggaccatcacgctgtgtcgcgaggctcagcaaaactgagatggttcgttgagagaaacatggtcacaccagaagggaaagtagtggacctcggttgtggcagaggaggctggtcatactattgtggaggactaaagaatgtaagagaagtcaaaggcctaacaaaaggaggaccaggacacgaagaacccatccccatgtcaacatatgggtggaatctagtgcgtcttcaaagtggagttgacgttttcttcatcccgccagaaaagtgtgacacattattgtgtgacataggggagtcatcaccaaatcccacagtggaagcaggacgaacactcagagtccttaacttagtagaaaattggttgaacaacaacactcaattttgcataaaggttctcaacccatatatgccctcagtcatagaaaaaatggaagcactacaaaggaaatatggaggagccttagtgaggaatccactctcacgaaactccacacatgagatgtactgggtatccaatgcttccgggaacatagtgtcatcagtgaacatgatttcaaggatgttgatcaacagatttacaatgagatacaagaaagccacttacgagccggatgttgacctcggaagcggaacccgtaacatcgggattgaaagtgagataccaaacctagatataattgggaaaagaatagaaaaaataaagcaagagcatgaaacatcatggcactatgaccaagaccacccatacaaaacgtgggcataccatggtagctatgaaacaaaacagactggatcagcatcatccatggtcaacggagtggtcaggctgctgacaaaaccttgggacgtcgtccccatggtgacacagatggcaatgacagacacgactccatttggacaacagcgcgtttttaaagagaaagtggacacgagaacccaagaaccgaaagaaggcacgaagaaactaatgaaaataacagcagagtggctttggaaagaattagggaagaaaaagacacccaggatgtgcaccagagaagaattcacaagaaaggtgagaagcaatgcagccttgggggccatattcactgatgagaacaagtggaagtcggcacgtgaggctgttgaagatagtaggttttgggagctggttgacaaggaaaggaatctccatcttgaaggaaagtgtgaaacatgtgtgtacaacatgatgggaaaaagagagaagaagctaggggaattcggcaaggcaaaaggcagcagagccatatggtacatgtggcttggagcacgcttcttagagtttgaagccctaggattcttaaatgaagatcactggttctccagagagaactccctgagtggagtggaaggagaagggctgcacaagctaggttacattctaagagacgtgagcaagaaagagggaggagcaatgtatgccgatgacaccgcaggatgggatacaagaatcacactagaagacctaaaaaatgaagaaatggtaacaaaccacatggaaggagaacacaagaaactagccgaggccattttcaaactaacgtaccaaaacaaggtggtgcgtgtgcaaagaccaacaccaagaggcacagtaatggacatcatatcgagaagagaccaaagaggtagtggacaagttggcacctatggactcaatactttcaccaatatggaagcccaactaatcagacagatggagggagaaggagtctttaaaagcattcagcacctaacaatcacagaagaaatcgctgtgcaaaactggttagcaagagtggggcgcgaaaggttatcaagaatggccatcagtggagatgattgtgttgtgaaacctttagatgacaggttcgcaagcgctttaacagctctaaatgacatgggaaagattaggaaagacatacaacaatgggaaccttcaagaggatggaatgattggacacaagtgcccttctgttcacaccatttccatgagttaatcatgaaagacggtcgcgtactcgttgttccatgtagaaaccaagatgaactgattggcagagcccgaatctcccaaggagcagggtggtctttgcgggagacggcctgtttggggaagtcttacgcccaaatgtggagcttgatgtacttccacagacgcgacctcaggctggcggcaaatgctatttgctcggcagtaccatcacattgggttccaacaagtcgaacaacctggtccatacatgctaaacatgaatggatgacaacggaagacatgctgacagtctggaacagggtgtggattcaagaaaacccatggatggaagacaaaactccagtggaatcatgggaggaaatcccatacttggggaaaagagaagaccaatggtgcggctcattgattgggttaacaagcagggccacctgggcaaagaacatccaagcagcaataaatcaagttagatcccttataggcaatgaagaatacacagattacatgccatccatgaaaagattcagaagagaagaggaagaagcaggagttctgtggtagaaagcaaaactaacatgaaacaaggctagaagtcaggtcggattaagccatagtacggaaaaaactatgctacctgtgagccccgtccaaggacgttaaaagaagtcaggccatcataaatgccatagcttgagtaaactatgcagcctgtagctccacctgagaaggtgtaaaaaatccgggaggccacaaaccatggaagctgtacgcatggcgtagtggactagcggttagaggagacccctcccttacaaatcgcagcaacaatgggggcccaaggcgagatgaagctgtagtctcgctggaaggactagaggttagaggagacccccccgaaacaaaaaacagcatattgacgctgggaaagaccagagatcctgctgtctcctcagcatcattccaggcacagaacgccagaaaatggaatggtgctgttgaatcaacaggttct

SEQ ID NO: 18 - protein, 3406 aa, Artificial Sequence
  Synthetic polypeptide
MNNQRKKAKNTPFNMLKRERNRVSTVQQLTKRFSLGMLQGRGPLKLFMALVAFLRFLTIPPTAGILKRWGTIKKSKAINVLRGFRKEIGRMLNILNRRRRSAGTSVGIVGLLLTTAMAAEVTRRGSAYYMYLDRNDAGEAISFPTTLGMNKCYIQIMDLGHMCDATMSYECPMLDEGVEPDDVDCWCNTTSTWVVYGTCHHKKGEARRSRRAVTLPSHSTRKLQTRSQTWLESREYTKHLIRVENWIFRNPGFALAAAAIAWLLGSSTSQKVIYLVMILLIAPAYSIRCIGVSNRDFVEGMSGGTWVDIVLEHGGCVTVMAQDKPTVDIELVTTTVSNMAEVRSYCYEASISDMASDSRCPTQGEAYLDKQSDTQYVCKRTLVDRGWGNGCGLFGKGSLVTCAKFACSKKMTGKSIQPENLEYRIMLSVHGSQHSGMIVNDTGHETDENRAKVEITPNSPRAEATLGGFGSLGLDCEPRTGLDFSDLYYLTMNNKHWLVHKEWFHDIPLPWHAGADTGTPHWNNKEALVEFKDAHAKRQTVVVLGSQEGAVHTALAGALEAEMDGAKGRLSSGHLKCRLKMDKLRLKGVSYSLCTAAFTFTKIPAETLHGTVTVEVQYAGTDGPCKVPAQMAVDMQTLTPVGRLITANPVITESTENSKMMLELDPPFGDSYIVIGVGEKKITHHWHRSGSTIGKAFEATVRGAKRMAVLGDTAWDFGSVGGALNSLGKGIHQIFGAAFKSLFGGMSWFSRILIGTLLMWLGLNTKNGSISLMCLAAGFVTLYLGVMVQADSGCVVSWKNKELKCGSGIFITDNVHTWTEQYKFQPESPSKLASAIQKAHEEDICGIRSVTRLENLMWKQITPELNHILSENEVKLTIMTGDIKGIMQAGKRSLRPQPTELKYSWKTWGKAKMLSTESHNQTFLIDGPETAECPNTNRAWNSLEVEDYGFGVFTTNIWLKLKEKQDVFCDSKLMSAAIKDNRAVHADMGYWIESALNDTWKIEKASFIEVKNCHWPKSHTLWSNGVLESEMIIPKNLAGPVSQHNYRPGYHTQITGPWHLGKLEMDFDFCDGTTVVVTEDCGNRGPSLRTTTASGKLITEWCCRSCTLPPLRYRGEDGCWYGMEIRPLKEKEENLVNSLVTAGHGQVDNFSLGVLGMALFLEEMLRTRVGTKHAILLVAVSFVTLITGNMSFRDLGRVMVMVGATMTDDIGMGVTYLALLAAFKVRPTFAAGLLLRKLTSNELMMTTIGIVLLSQSTIPETILELTDALALGMMVLKMVRNMEKYQLAVTIMAILCVPNAVILQNAWKVSCTILAVVSVSPLFLTSSQQKTDWIPLALTIKGLNPTAIFLTTLSRTSKKRSWPLNEAIMAVGMVSILASSLLKNDIPMTGPLVAGGLLTVCYVLTGRSADLELERAADVKWEDQAEISGSSPILSITISEDGSMSIKNEEEEQTLTILIRTGLLVISGLFPVSIPITAAAWYLWEVKKQRAGVLWDVPSPPPMGKAELEDGAYRIKQKGILGYSQIGAGVYKEGTFHTMWHVTRGAVLMHKGKRIEPSWADVKKDLISYGGGWKLEGEWKEGEEVQVLALEPGKNPRAVQTKPGLFKTNAGTIGAVSLDFSPGTSGSPIIDKKGKVVGLYGNGVVTRSGAYVSAIAQTEKSIEDNPEIEDDIFRKRRLTIMDLHPGAGKTKRYLPAIVREAIKRGLRTLILAPTRVVAAEMEEALRGLPIRYQTPAIRAVHTGREIVDLMCHATFTMRLLSPVRVPNYNLIIMDEAHFTDPASIAARGYISTRVEMGEAAGIFMTATPPGSRDPFPQSNAPIIDEEREIPERSWNSGHEWVTDFKGKTVWFVPSIKAGNDIAACLRKNGKKVIQLSRKTFDSEYVKTRTNDWDFVVTTDISEMGANFKAERVIDPRRCMKPVILTDGEERVILAGPMPVTHSSAAQRRGRIGRNPKNENDQYIYMGEPLENDEDCAHWKEAKMLLDNINTPEGIIPSMFEPEREKVDAIDGEYRLRGEARKTFVDLMRRGDLPVWLAYRVAAEGINYADRRWCFDGVKNNQILEENVEVEIWTKEGERKKLKPRWLDARIYSDPLALKEFKEFAAGRKSLTLNLITEMGRLPTFMTQKARNALDNLAVLHTAEAGGRAYNHALSELPETLETLLLLTLLATVTGGIFLFLMSARGIGKMTLGMCCIITASILLWYAQIQPHWIAASIILEFFLIVLLIPEPEKQRTPQDNQLTYVVIAILTVVAATMANEMGFLEKTKKDLGLGSIATQQPESNILDIDLRPASAWTLYAVATTFVTPMLRHSIENSSVNVSLTAIANQATVLMGLGKGWPLSKMDIGVPLLAIGCYSQVNPITLTAALFLLVAHYAIIGPGLQAKATREAQKRAAAGIMKNPTVDGITVIDLDPIPYDPKFEKQLGQVMLLVLCVTQVLMMRTTWALCEALTLATGPISTLWEGNPGRFWNTTIAVSMANIFRGSYLAGAGLLFSIMKNTTNTRRGTGNIGETLGEKWKSRLNALGKSEFQIYKKSGIQEVDRTLAKEGIKRGETDHHAVSRGSAKLRWFVERNMVTPEGKVVDLGCGRGGWSYYCGGLKNVREVKGLTKGGPGHEEPIPMSTYGWNLVRLQSGVDVFFIPPEKCDTLLCDIGESSPNPTVEAGRTLRVLNLVENWLNNNTQFCIKVLNPYMPSVIEKMEALQRKYGGALVRNPLSRNSTHEMYWVSNASGNIVSSVNMISRMLINRFTMRYKKATYEPDVDLGSGTRNIGIESEIPNLDIIGKRIEKIKQEHETSWHYDQDHPYKTWAYHGSYETKQTGSASSMVNGVVRLLTKPWDVVPMVTQMAMTDTTPFGQQRVFKEKVDTRTQEPKEGTKKLMKITAEWLWKELGKKKTPRMCTREEFTRKVRSNAALGAIFTDENKWKSAREAVEDSRFWELVDKERNLHLEGKCETCVYNMMGKREKKLGEFGKAKGSRAIWYMWLGARFLEFEALGFLNEDHWFSRENSLSGVEGEGLHKLGYILRDVSKKEGGAMYADDTAGWDTRITLEDLKNEEMVTNHMEGEHKKLAEAIFKLTYQNKVVRVQRPTPRGTVMDIISRRDQRGSGQVGTYGLNTFTNMEAQLIRQMEGEGVFKSIQHLTITEEIAVQNWLARVGRERLSRMAISGDDCVVKPLDDRFASALTALNDMGKIRKDIQQWEPSRGWNDWTQVPFCSHHFHELIMKDGRVLVVPCRNQDELIGRARISQGAGWSLRETACLGKSYAQMWSLMYFHRRDLRLAANAICSAVPSHWVPTSRTTWSIHAKHEWMTTEDMLTVWNRVWIQENPWMEDKTPVESWEEIPYLGKREDQWCGSLIGLTSRATWAKNIQAAINQVRSLIGNEEYTDYMPSMKRFRREEEEAGVLW

SEQ ID NO: 19 - DNA, 10768 bp, Artificial Sequence
  Synthetic construct
agttgttagtctacgtggaccgacaaagacagattctttgagggagctaagctcaacgtagttctaacagttttttaattagagagcagatctctgatgaataaccaacggaaaaaggcgaaaaacacgcctttcaatatgctgaaacgcgagagaaaccgcgtgtcgactgtgcaacagctgacaaagagattctcacttggaatgctgcagggacgaggaccattaaaactgttcatggccctggtggcgttccttcgtttcctaacaatcccaccaacagcagggatattgaagagatggggaacaattaaaaaatcaaaagctattaatgttttgagagggttcaggaaagagattggaaggatgctgaacatcttgaataggagacgcagatccgcgggtactagtgtcggaattgttggcctcctgctgaccacagctatggcagcggaggtcactagacgtgggagtgcatactatatgtacttggacagaaacgatgctggggaggccatatcttttccaaccacattggggatgaataagtgttatatacagatcatggatcttggacacatgtgtgatgccaccatgagctatgaatgccctatgctggatgagggggtggaaccagatgacgtcgattgttggtgcaacacgacgtcaacttgggttgtgtacggaacctgccatcacaaaaaaggtgaagcacggagaagtagaagagctgtgacgctcccctcccattccactaggaagctgcaaacgcggtcgcaaacctggttggaatcaagagaatacacaaagcacttgattagagtcgaaaattggatattcaggaaccctggcttcgcgttagcagcagctgccatcgcttggcttttgggaagctcaacgagccaaaaagtcatatacttggtcatgatactgctgattgccccggcatacagcatcaggtgcataggagtcagcaatagggactttgtggaaggtatgtcaggtgggacttgggttgatattgtcttggaacatggaggttgtgtcaccgtaatggcacaggacaaaccgactgtcgacatagagctggttacaacaacagtcagcaacatggcggaggtaagatcctactgctatgaggcatcaatatcagacatggcttcggacagccgctgcccaacacaaggtgaagcctaccttgacaagcaatcagacactcaatatgtctgcaaaagaacgttagtggacagaggctggggaaatggatgtggactttttggcaaagggagtctggtgacatgcgctaagtttgcatgctccaagaaaatgaccgggaagagcatccagccagagaatctggagtaccggataatgctgtcagttcatggctcccagcacagtgggatgatcgttaatgacacaggacatgaaactgatgagaatagagcgaaggttgagataacgcccaattcaccaagagccgaagccaccctggggggttttggaagcctaggacttgattgtgaaccgaggacaggccttgacttttcagatttgtattacttgactatgaataacaagcactggttggttcacaaggagtggttccacgacattccattaccttggcacgctggggcagacaccggaactccacactggaacaacaaagaagcactggtagagttcaaggacgcacatgccaaaaggcaaactgtcgtggttctagggagtcaagaaggagcagttcacacggcccttgctggagctctggaggctgagatggatggtgcaaagggaaggctgtcctctggccacttgaaatgtcgcctgaaaatggataaacttagattgaagggcgtgtcatactccttgtgtaccgcagcgttcacattcaccaagatcccggctgaaacactgcacgggacagtcacagtggaggtacagtacgcagggacagatggaccttgcaaggttccagctcagatggcggtggacatgcaaactctgaccccagttgggaggttgataaccgctaaccccgtaatcactgaaagcactgagaactctaagatgatgctggaacttgatccaccatttggggactcttacattgtcataggagtcggggagaagaagatcacccaccactggcacaggagtggcagcaccattggaaaagcatttgaagccactgtgagaggtgccaagagaatggcagtcttgggagacacagcctgggactttggatcagttggaggcgctctcaactcattgggcaagggcatccatcaaatttttggagcagctttcaaatcattgtttggaggaatgtcctggttctcaagaattctcattggaacgttgctgatgtggttgggtctgaacacaaagaatggatctacttcccttatgtgcttggccgccggctttgtgacactgtatttgggggtcatggtgcaggccgatagtggttgcgttgtgagctggaaaaacaaagaactgaaatgtggcagtgggattttcatcacagacaacgtgcacacatggacagaacaatacaagttccaaccagaatccccttcaaaactagcttcagctatccagaaagcccatgaagagggcatttgtggaatccgctcagtaacaagactggagaatctgatgtggaaacaaataacaccagaattgaatcacattctatcagaaaatgaggtgaagttaactattatgacaggagacatcaaaggaatcatgcaggcaggaaaacgatctctgcggcctcagcccactgagctgaagtattcatggaaaacatggggcaaagcaaaaatgctctctacagagtctcataaccagacctttctcattgatggccccgaaacagcagaatgccccaacacaaatagagcttggaattcgttggaagttgaagactatggctttggagtattcaccaccaatatatggctaaaattgaaagaaaaacaggatgtattctgcgactcaaaactcatgtcagcggccataaaagacaacagagccgtccatgccgatatgggttattggatagaaagtgcactcaatgacacatggaagatagagaaagcctctttcattgaagttaaaaactgccactggccaaaatcacacaccctctggagcaatggagtgctagaaagtgagatgataattccaaagaatctcgctggaccagtgtctcaacacaactatagaccaggctaccatacacaaataacaggaccatggcatctaggtaagcttgagatggactttgatttctgtgatggaacaacagtggtagtgactgaggactgcggaaatagaggaccctctttgagaacaaccactgcctctggaaaactcataacagaatggtgctgccgatcttgcacattaccaccgctaagatacagaggtgaggatgggtgctggtacgggatggaaatcagaccattgaaggagaaagaagagaatttggtcaactccttggtcacagctggacatgggcaggtcgacaacttttcactaggagtcttgggaatggcattgttcctggaggaaatgcttaggacccgagtaggaacgaaacatgcaatactactagttgcagtttcttttgtgacattgatcacagggaacatgtcctttagagacctgggaagagtgatggttatggtaggcgccactatgacggatgacataggtatgggcgtgacttatcttgccctactagcagccttcaaagtcagaccaacttttgcagctggactactcttgagaaagctgacctccaatgaattgatgatgactactataggaattgtactcctctcccagagcaccataccagagaccattcttgagttgactgatgcgttagccttaggcatgatggtcctcaaaatggtgagaaatatggaaaagtatcaattggcagtgactatcatggctatcttgtgcgtcccaaacgcagtgatattacaaaacgcatggaaagtgagttgcacaatattggcagtggtgtccgtttccccactgctcttaacatcctcacagcaaaaaacagattggataccattagcattgacgatcaaaggtctcaatccaacagctatttttctaacaaccctctcaagaaccagcaagaaaaggagctggccattaaatgaggctatcatggcagtcgggatggtgagcattttagccagttctctcctaaaaaatgatattcccatgacaggaccattagtggctggagggctcctcactgtgtgctacgtgctcactggacgatcggccgatttggaactggagagagcagccgatgtcaaatgggaagaccaggcagagatatcaggaagcagtccaatcctgtcaataacaatatcagaagatggtagcatgtcgataaaaaatgaagaggaagaacaaacactgaccatactcattagaacaggattgctggtgatctcaggactttttcctgtatcaataccaatcacggcagcagcatggtacctgtgggaagtgaagaaacaacgggccggagtattgtgggatgttccttcacccccacccatgggaaaggctgaactggaagatggagcctatagaattaagcaaaaagggattcttggatattcccagatcggagccggagtttacaaagaaggaacattccatacaatgtggcatgtcacacgtggcgctgttctaatgcataaaggaaagaggattgaaccatcatgggcggacgtcaagaaagacctaatatcatatggaggaggctggaagttagaaggagaatggaaggaaggagaagaagtccaggtattggcactggagcctggaaaaaatccaagagccgtccaaacgaaacctggtcttttcaaaaccaacgccggaacaataggtgctgtatctctggacttttctcctggaacgtcaggatctccaattatcgacaaaaaaggaaaagttgtgggtctttatggtaatggtgttgttacaaggagtggagcatatgtgagtgctatagcccagactgaaaaaagcattgaagacaacccagagatcgaagatgacattttccgaaagagaagactgaccatcatggacctccacccaggagcgggaaagacgaagagataccttccggccatagtcagagaagctataaaacggggtttgagaacattaatcttggcccccactagagttgtggcagctgaaatggaggaagcccttagaggacttccaataagataccagaccccagccatcagagctgagcacaccgggcgggagattgtggacctaatgtgtcatgccacatttaccatgaggctgctatcaccagttagagtgccaaactacaacctgattatcatggacgaagcccatttcacagacccagcaagtatagcagctagaggatacatctcaactcgagtggagatgggtgaggcagctgggatttttatgacagccactcccccgggaagcagagacccatttcctcagagcaatgcaccaatcatagatgaagaaagagaaatccctgaacgttcgtggaattccggacatgaatgggtcacggattttaaagggaagactgtttggttcgttccaagtataaaagcaggaaatgatatagcagcttgcctgaggaaaaatggaaagaaagtgatacaactcagtaggaagacctttgattctgagtatgtcaagactagaaccaatgattgggacttcgtggttacaactgacatttcagaaatgggtgccaatttcaaggctgagagggttatagaccccagacgctgcatgaaaccagtcatactaacagatggtgaagagcgggtgattctggcaggacctatgccagtgacccactctagtgcagcacaaagaagagggagaataggaagaaatccaaaaaatgagaatgaccagtacatatacatgggggaacctctggaaaatgatgaagactgtgcacactggaaagaagctaaaatgctcctagataacatcaacacgccagaaggaatcattcctagcatgttcgaaccagagcgtgaaaaggtggatgccattgatggcgaataccgcttgagaggagaagcaaggaaaacctttgtagacttaatgagaagaggagacctaccagtctggttggcctacagagtggcagctgaaggcatcaactacgcagacagaaggtggtgttttgatggagtcaagaacaaccaaatcctagaagaaaacgtggaagttgaaatctggacaaaagaaggggaaaggaagaaattgaaacccagatggttggatgctaggatctattctgacccactggcgctaaaagaatttaaggaatttgcagccggaagaaagtctctgaccctgaacctaatcacagaaatgggtaggctcccaaccttcatgactcagaaggcaagagacgcactggacaacttagcagtgctgcacacggctgaggcaggtggaagggcgtacaaccatgctctcagtgaactgccggagaccctggagacattgcttttactgacacttctggctacagtcacgggagggatctttttattcttgatgagcggaaggggcatagggaagatgaccctgggaatgtgctgcataatcacggctagcatcctcctatggtacgcacaaatacagccacactggatagcagcttcaataatactggagttttttctcatagttttgcttattccagaacctgaaaaacagagaacaccccaagacaaccaactgacctacgttgtcatagccatcctcacagtggtggccgcaaccatggcaaacgagatgggtttcctagaaaaaacgaagaaagatctcggattgggaagcattgcaacccagcaacccgagagcaacatcctggacatagatctacgtcctgcatcagcatggacgctgtatgccgtggccacaacatttgttacaccaatgttgagacatagcattgaaaattcctcagtgaatgtgtccctaacagctatagccaaccaagccacagtgttaatgggtctcgggaaaggatggccattgtcaaagatggacatcggagttccccttctcgccattggatgctactcacaagtcaaccccataactctcacagcagctcttttcttattggtagcacattatgccatcatagggccaggactccaagcaaaagcaaccagagaagctcagaaaagagcagcggcgggcatcatgaaaaacccaactgtcgatggaataacagtgattgacctagatccaataccttatgatccaaagtttgaaaagcagttgggacaagtaatgctcctagtcctctgcgtgactcaagtattgatgatgaggactacatgggctctgtgtgaggctttaaccttagctaccgggcccatctccacattgtgggaaggaaatccagggaggttttggaacactaccattgcggtgtcaatggctaacatttttagagggagttacttggccggagctggacttctcttttctattatgaagaacacaaccaacacaagaaggggaactggcaacataggagagacgcttggagagaaatggaaaagccgattgaacgcattgggaaaaagtgaattccagatctacaagaaaagtggaatccaggaagtggatagaaccttagcaaaagaaggcattaaaagaggagaaacggaccatcacgctgtgtcgcgaggctcagcaaaactgagatggttcgttgagagaaacatggtcacaccagaagggaaagtagtggacctcggttgtggcagaggaggctggtcatactattgtggaggactaaagaatgtaagagaagtcaaaggcctaacaaaaggaggaccaggacacgaagaacccatccccatgtcaacatatgggtggaatctagtgcgtcttcaaagtggagttgacgttttcttcatcccgccagaaaagtgtgacacattattgtgtgacataggggagtcatcaccaaatcccacagtggaagcaggacgaacactcagagtccttaacttagtagaaaattggttgaacaacaacactcaattttgcataaaggttctcaacccatatatgccctcagtcatagaaaaaatggaagcactacaaaggaaatatggaggagccttagtgaggaatccactctcacgaaactccacacatgagatgtactgggtatccaatgcttccgggaacatagtgtcatcagtgaacatgatttcaaggatgttgatcaacagatttacaatgagatacaagaaagccacttacgagccggatgttgacctcggaagcggaacccgtaacatcgggattgaaagtgagataccaaacctagatataattgggaaaagaatagaaaaaataaagcaagagcatgaaacatcatggcactatgaccaagaccacccatacaaaacgtgggcataccatggtagctatgaaacaaaacagactggatcagcatcatccatggtcaacggagtggtcaggctgctgacaaaaccttgggacgtcgtccccatggtgacacagatggcaatgacagacacgactccatttggacaacagcgcgtttttaaagagaaagtggacacgagaacccaagaaccgaaagaaggcacgaagaaactaatgaaaataacagcagagtggctttggaaagaattagggaagaaaaagacacccaggatgtgcaccagagaagaattcacaagaaaggtgagaagcaatgcagccttgggggccatattcactgatgagaacaagtggaagtcggcacgtgaggctgttgaagatagtaggttttgggagctggttgacaaggaaaggaatctccatcttgaaggaaagtgtgaaacatgtgtgtacaacatgatgggaaaaagagagaagaagctaggggaattcggcaaggcaaaaggcagcagagccatatggtacatgtggcttggagcacgcttcttagagtttgaagccctaggattcttaaatgaagatcactggttctccagagagaactccctgagtggagtggaaggagaagggctgcacaagctaggttacattctaagagacgtgagcaagaaagagggaggagcaatgtatgccgatgacaccgcaggatgggatacaagaatcacactagaagacctaaaaaatgaagaaatggtaacaaaccacatggaaggagaacacaagaaactagccgaggccattttcaaactaacgtaccaaaacaaggtggtgcgtgtgcaaagaccaacaccaagaggcacagtaatggacatcatatcgagaagagaccaaagaggtagtggacaagttggcacctatggactcaatactttcaccaatatggaagcccaactaatcagacagatggagggagaaggagtctttaaaagcattcagcacctaacaatcacagaagaaatcgctgtgcaaaactggttagcaagagtggggcgcgaaaggttatcaagaatggccatcagtggagatgattgtgttgtgaaacctttagatgacaggttcgcaagcgctttaacagctctaaatgacatgggaaagattaggaaagacatacaacaatgggaaccttcaagaggatggaatgattggacacaagtgcccttctgttcacaccatttccatgagttaatcatgaaagacggtcgcgtactcgttgttccatgtagaaaccaagatgaactgattggcagagcccgaatctcccaaggagcagggtggtctttgcgggagacggcctgtttggggaagtcttacgcccaaatgtggagcttgatgtacttccacagacgcgacctcaggctggcggcaaatgctatttgctcggcagtaccatcacattgggttccaacaagtcgaacaacctggtccatacatgctaaacatgaatggatgacaacggaagacatgctgacagtctggaacagggtgtggattcaagaaaacccatggatggaagacaaaactccagtggaatcatgggaggaaatcccatacttggggaaaagagaagaccaatggtgcggctcattgattgggttaacaagcagggccacctgggcaaagaacatccaagcagcaataaatcaagttagatcccttataggcaatgaagaatacacagattacatgccatccatgaaaagattcagaagagaagaggaagaagcaggagttctgtggtagaaagcaaaactaacatgaaacaaggctagaagtcaggtcggattaagccatagtacggaaaaaactatgctacctgtgagccccgtccaaggacgttaaaagaagtcaggccatcataaatgccatagcttgagtaaactatgcagcctgtagctccacctgagaaggtgtaaaaaatccgggaggccacaaaccatggaagctgtacgcatggcgtagtggactagcggttagaggagacccctcccttacaaatcgcagcaacaatgggggcccaaggcgagatgaagctgtagtctcgctggaaggactagaggttagaggagacccccccgaaacaaaaaacagcatattgacgctgggaaagaccagagatcctgctgtctcctcagcatcattccaggcacagaacgccagaaaatggaatggtgctgttgaatcaacaggttct

SEQ ID NO: 20 - protein, 3406 aa, Artificial Sequence
  Synthetic polypeptide
MNNQRKKAKNTPFNMLKRERNRVSTVQQLTKRFSLGMLQGRGPLKLFMALVAFLRFLTIPPTAGILKRWGTIKKSKAINVLRGFRKEIGRMLNILNRRRRSAGTSVGIVGLLLTTAMAAEVTRRGSAYYMYLDRNDAGEAISFPTTLGMNKCYIQIMDLGHMCDATMSYECPMLDEGVEPDDVDCWCNTTSTWVVYGTCHHKKGEARRSRRAVTLPSHSTRKLQTRSQTWLESREYTKHLIRVENWIFRNPGFALAAAAIAWLLGSSTSQKVIYLVMILLIAPAYSIRCIGVSNRDFVEGMSGGTWVDIVLEHGGCVTVMAQDKPTVDIELVTTTVSNMAEVRSYCYEASISDMASDSRCPTQGEAYLDKQSDTQYVCKRTLVDRGWGNGCGLFGKGSLVTCAKFACSKKMTGKSIQPENLEYRIMLSVHGSQHSGMIVNDTGHETDENRAKVEITPNSPRAEATLGGFGSLGLDCEPRTGLDFSDLYYLTMNNKHWLVHKEWFHDIPLPWHAGADTGTPHWNNKEALVEFKDAHAKRQTVVVLGSQEGAVHTALAGALEAEMDGAKGRLSSGHLKCRLKMDKLRLKGVSYSLCTAAFTFTKIPAETLHGTVTVEVQYAGTDGPCKVPAQMAVDMQTLTPVGRLITANPVITESTENSKMMLELDPPFGDSYIVIGVGEKKITHHWHRSGSTIGKAFEATVRGAKRMAVLGDTAWDFGSVGGALNSLGKGIHQIFGAAFKSLFGGMSWFSRILIGTLLMWLGLNTKNGSTSLMCLAAGFVTLYLGVMVQADSGCVVSWKNKELKCGSGIFITDNVHTWTEQYKFQPESPSKLASAIQKAHEEGICGIRSVTRLENLMWKQITPELNHILSENEVKLTIMTGDIKGIMQAGKRSLRPQPTELKYSWKTWGKAKMLSTESHNQTFLIDGPETAECPNTNRAWNSLEVEDYGFGVFTTNIWLKLKEKQDVFCDSKLMSAAIKDNRAVHADMGYWIESALNDTWKIEKASFIEVKNCHWPKSHTLWSNGVLESEMIIPKNLAGPVSQHNYRPGYHTQITGPWHLGKLEMDFDFCDGTTVVVTEDCGNRGPSLRTTTASGKLITEWCCRSCTLPPLRYRGEDGCWYGMEIRPLKEKEENLVNSLVTAGHGQVDNFSLGVLGMALFLEEMLRTRVGTKHAILLVAVSFVTLITGNMSFRDLGRVMVMVGATMTDDIGMGVTYLALLAAFKVRPTFAAGLLLRKLTSNELMMTTIGIVLLSQSTIPETILELTDALALGMMVLKMVRNMEKYQLAVTIMAILCVPNAVILQNAWKVSCTILAVVSVSPLLLTSSQQKTDWIPLALTIKGLNPTAIFLTTLSRTSKKRSWPLNEAIMAVGMVSILASSLLKNDIPMTGPLVAGGLLTVCYVLTGRSADLELERAADVKWEDQAEISGSSPILSITISEDGSMSIKNEEEEQTLTILIRTGLLVISGLFPVSIPITAAAWYLWEVKKQRAGVLWDVPSPPPMGKAELEDGAYRIKQKGILGYSQIGAGVYKEGTFHTMWHVTRGAVLMHKGKRIEPSWADVKKDLISYGGGWKLEGEWKEGEEVQVLALEPGKNPRAVQTKPGLFKTNAGTIGAVSLDFSPGTSGSPIIDKKGKVVGLYGNGVVTRSGAYVSAIAQTEKSIEDNPEIEDDIFRKRRLTIMDLHPGAGKTKRYLPAIVREAIKRGLRTLILAPTRVVAAEMEEALRGLPIRYQTPAIRAEHTGREIVDLMCHATFTMRLLSPVRVPNYNLIIMDEAHFTDPASIAARGYISTRVEMGEAAGIFMTATPPGSRDPFPQSNAPIIDEEREIPERSWNSGHEWVTDFKGKTVWFVPSIKAGNDIAACLRKNGKKVIQLSRKTFDSEYVKTRTNDWDFVVTTDISEMGANFKAERVIDPRRCMKPVILTDGEERVILAGPMPVTHSSAAQRRGRIGRNPKNENDQYIYMGEPLENDEDCAHWKEAKMLLDNINTPEGIIPSMFEPEREKVDAIDGEYRLRGEARKTFVDLMRRGDLPVWLAYRVAAEGINYADRRWCFDGVKNNQILEENVEVEIWTKEGERKKLKPRWLDARIYSDPLALKEFKEFAAGRKSLTLNLITEMGRLPTFMTQKARDALDNLAVLHTAEAGGRAYNHALSELPETLETLLLLTLLATVTGGIFLFLMSGRGIGKMTLGMCCIITASILLWYAQIQPHWIAASIILEFFLIVLLIPEPEKQRTPQDNQLTYVVIAILTVVAATMANEMGFLEKTKKDLGLGSIATQQPESNILDIDLRPASAWTLYAVATTFVTPMLRHSIENSSVNVSLTAIANQATVLMGLGKGWPLSKMDIGVPLLAIGCYSQVNPITLTAALFLLVAHYAIIGPGLQAKATREAQKRAAAGIMKNPTVDGITVIDLDPIPYDPKFEKQLGQVMLLVLCVTQVLMMRTTWALCEALTLATGPISTLWEGNPGRFWNTTIAVSMANIFRGSYLAGAGLLFSIMKNTTNTRRGTGNIGETLGEKWKSRLNALGKSEFQIYKKSGIQEVDRTLAKEGIKRGETDHHAVSRGSAKLRWFVERNMVTPEGKVVDLGCGRGGWSYYCGGLKNVREVKGLTKGGPGHEEPIPMSTYGWNLVRLQSGVDVFFIPPEKCDTLLCDIGESSPNPTVEAGRTLRVLNLVENWLNNNTQFCIKVLNPYMPSVIEKMEALQRKYGGALVRNPLSRNSTHEMYWVSNASGNIVSSVNMISRMLINRFTMRYKKATYEPDVDLGSGTRNIGIESEIPNLDIIGKRIEKIKQEHETSWHYDQDHPYKTWAYHGSYETKQTGSASSMVNGVVRLLTKPWDVVPMVTQMAMTDTTPFGQQRVFKEKVDTRTQEPKEGTKKLMKITAEWLWKELGKKKTPRMCTREEFTRKVRSNAALGAIFTDENKWKSAREAVEDSRFWELVDKERNLHLEGKCETCVYNMMGKREKKLGEFGKAKGSRAIWYMWLGARFLEFEALGFLNEDHWFSRENSLSGVEGEGLHKLGYILRDVSKKEGGAMYADDTAGWDTRITLEDLKNEEMVTNHMEGEHKKLAEAIFKLTYQNKVVRVQRPTPRGTVMDIISRRDQRGSGQVGTYGLNTFTNMEAQLIRQMEGEGVFKSIQHLTITEEIAVQNWLARVGRERLSRMAISGDDCVVKPLDDRFASALTALNDMGKIRKDIQQWEPSRGWNDWTQVPFCSHHFHELIMKDGRVLVVPCRNQDELIGRARISQGAGWSLRETACLGKSYAQMWSLMYFHRRDLRLAANAICSAVPSHWVPTSRTTWSIHAKHEWMTTEDMLTVWNRVWIQENPWMEDKTPVESWEEIPYLGKREDQWCGSLIGLTSRATWAKNIQAAINQVRSLIGNEEYTDYMPSMKRFRREEEEAGVLW

SEQ ID NO: 21 - DNA, 10768 bp, Artificial Sequence
  Synthetic construct
agttgttagtctacgtggaccgacaaagacagattctttgagggagctaagctcaatgtagttctaacagttttttaattagagagcagatctctgatgaataaccaacggaaaaaggcgaaaaacacgcctttcaatatgctgaaacgcgagagaaaccgcgtgtcgactgtgcaacagctgacaaagagattctcacttggaatgctgcagggacgaggaccattaaaactgttcatggccctggtggcgttccttcgtttcctaacaatcccaccaacagcagggatattgaagagatggggaacaattaaaaaatcaaaagctattaatgttttgagagggttcaggaaagagattggaaggatgctgaacatcttgaataggagacgcagatccgcgggtactagtgtcggaattgttggcctcctgctgaccacagctatggcagcggaggtcactagacgtgggagtgcatactatatgtacttggacagaaacgatgctggggaggccatatcttttccaaccacattggggatgaataagtgttatatacagatcatggatcttggacacatgtgtgatgccaccatgagctatgaatgccctatgctggatgagggggtggaaccagatgacgtcgattgttggtgcaacacgacgtcaacttgggttgtgtacggaacctgccatcacaaaaaaggtgaagcacggagaagtagaagagctgtgacgctcccctcccattccactaggaagctgcaaacgcggtcgcaaacctggttggaatcaagagaatacacaaagcacttgattagagtcgaaaattggatattcaggaaccctggcttcgcgttagcagcagctgccatcgcttggcttttgggaagctcaacgagccaaaaagtcatatacttggtcatgatactgctgattgccccggcatacagcatcaggtgcataggagtcagcaatagggactttgtggaaggtatgtcaggtgggacttgggttgatattgtcttggaacatggaggttgtgtcaccgtaatggcacaggacaaaccgactgtcgacatagagctggttacaacaacagtcagcaacatggcggaggtaagatcctactgctatgaggcatcaatatcagacatggcttcggacagccgctgcccaacacaaggtgaagcctaccttgacaagcaatcagacactcaatatgtctgcaaaagaacgttagtggacagaggctggggaaatggatgtggactttttggcaaagggagtctggtgacatgcgctaagtttgcatgctccaagaaaatgaccgggaagagcatccagccagagaatctggagtaccggataatgctgtcagttcatggctcccagcacagtgggatgatcgttaatgacacaggacatgaaactgatgagaatagagcgaaggttgagataacgcccaattcaccaagagccgaagccaccctggggggttttggaagcctaggacttgattgtgaaccgaggacaggccttgacttttcagatttgtattacttgactatgaataacaagcactggttggttcacaaggagtggttccacgacattccattaccttggcacgctggggcagacaccggaactccacactggaacaacaaagaagcactggtagagttcaaggacgcacatgccaaaaggcaaactgtcgtggttctagggagtcaagaaggagcagttcacacggcccttgctggagctctggaggctgagatggatggtgcaaagggaaggctgtcctctggccacttgaaatgtcgcctgaaaatggataaacttagattgaagggcgtgtcatactccttgtgtaccgcagcgttcacattcaccaagatcccggctgaaacactgcacgggacagtcacagtggaggtacagtacgcagggacagatggaccttgcaaggttccagctcagatggcggtggacatgcaaactctgaccccagttgggaggttgataaccgctaaccccgtaatcactgaaagcactgagaactctaagatgatgctggaacttgatccaccatttggggactcttacattgtcataggagtcggggagaagaagatcacccaccactggcacaggagtggcagcaccattggaaaagcatttgaagccactgtgagaggtgccaagagaatggcagtcttgggagacacagcctgggactttggatcagttggaggcgctctcaactcattgggcaagggcatccatcaaatttttggagcagctttcaaatcattgtttggaggaatgtcctggttctcaagaattctcattggaacgttgctgatgtggttgggtctgaacacaaagaatggatctacttcccttatgtgcttggccgccggctttgtgacactgtatttgggagtcatggtgcaggccgatagtggttgcgttgtgagctggaaaaacaaagaactgaaatgtggcagtgggattttcatcacagacaacgtgcacacatggacagaacaatacaagttccaaccagaatccccttcaaaactagcttcagctatccagaaagcccatgaagaggacatttgtggaatccgctcagtaacaagactggagaatctgatgtggaaacaaataacaccagaattgaatcacattctatcagaaaatgaggtgaagttaactattatgacaggagacatcaaaggaatcatgcaggcaggaaaacgatctctgcggcctcagcccactgagctgaagtattcatggaaaacatggggcaaagcaaaaatgctctctacagagtctcataaccagacctttctcattgatggccccgaaacagcagaatgccccaacacaaatagagcttggaattcgttggaagttgaagactatggctttggagtattcaccaccaatatatggctaaaattgaaagaaaaacaggatgtattctgcgactcaaaactcatgtcagcggccataaaagacaacagagccgtccatgccgatatgggttattggatagaaagtgcactcaatgacacatggaagatagagaaagcctctttcattgaagttaaaaactgccactggccaaaatcacacaccctctggagcaatggagtgctagaaagtgagatgataattccaaagaatctcgctggaccagtgtctcaacacaactatagaccaggctaccatacacaaataacaggaccatggcatctaggtaagcttgagatggactttgatttctgtgatggaacaacagtggtagtgactgaggactgcggaaatagaggaccctctttgagaacaaccactgcctctggaaaactcataacagaatggtgctgccgatcttgcacattaccaccgctaagatacagaggtgaggatgggtgctggtacgggatggaaatcagaccattgaaggagaaagaagagaatttggtcaactccttggtcacagctggacatgggcaggtcgacaacttttcactaggagtcttgggaatggcattgttcctggaggaaatgcttaggacccgagtaggaacgaaacatgcaatactactagttgcagtttcttttgtgacattgatcacagggaacatgtcctttagagacctgggaagagtgatggttatggtaggcgccactatgacggatgacataggtatgggcgtgacttatcttgccctactagcagccttcaaagtcagaccaacttttgcagctggactactcttgagaaagctgacctccaatgaattgatgatgactactataggaattgtactcctctcccagagcaccataccagagaccattcttgagttgactgatgcgttagccttaggcatgatggtcctcaaaatggtgagaaatatggaaaagtatcaattggcagtgactatcatggctatcttgtgcgtcccaaacgcagtgatattacaaaacgcatggaaagtgagttgcacaatattggcagtggtgtccgtttccccactgttcttaacatcctcacagcaaaaaacagattggataccattagcattgacgatcaaaggtctcaatccaacagctatttttctaacaaccctctcaagaaccagcaagaaaaggagctggccattaaatgaggctatcatggcagtcgggatggtgagcattttagccagttctctcctaaaaaatgatattcccatgacaggaccattagtggctggagggctcctcactgtgtgctacgtgctcactggacgatcggccgatttggaactggagagagcagccgatgtcaaatgggaagaccaggcagagatatcaggaagcagtccaatcctgtcaataacaatatcagaagatggtagcatgtcgataaaaaatgaagaggaagaacaaacactgaccatactcattagaacaggattgctggtgatctcaggactttttcctgtatcaataccaatcacggcagcagcatggtacctgtgggaagtgaagaaacaacgggccggagtattgtgggatgttccttcacccccacccatgggaaaggctgaactggaagatggagcctatagaattaagcaaaaagggattcttggatattcccagatcggagccggagtttacaaagaaggaacattccatacaatgtggcatgtcacacgtggcgctgttctaatgcataaaggaaagaggattgaaccatcatgggcggacgtcaagaaagacctaatatcatatggaggaggctggaagttagaaggagaatggaaggaaggagaagaagtccaggtattggcactggagcctggaaaaaatccaagagccgtccaaacgaaacctggtcttttcaaaaccaacgccggaacaataggtgctgtatctctggacttttctcctggaacgtcaggatctccaattatcgacaaaaaaggaaaagttgtgggtctttatggtaatggtgttgttacaaggagtggagcatatgtgagtgctatagcccagactgaaaaaagcattgaagacaacccagagatcgaagatgacattttccgaaagagaagactgaccatcatggacctccacccaggagcgggaaagacgaagagataccttccggccatagtcagagaagctataaaacggggtttgagaacattaatcttggcccccactagagttgtggcagctgaaatggaggaagcccttagaggacttccaataagataccagaccccagccatcagagctgtgcacaccgggcgggagattgtggacctaatgtgtcatgccacatttaccatgaggctgctatcaccagttagagtgccaaactacaacctgattatcatggacgaagcccatttcacagacccagcaagtatagcagctagaggatacatctcaactcgagtggagatgggtgaggcagctgggatttttatgacagccactcccccgggaagcagagacccatttcctcagagcaatgcaccaatcatagatgaagaaagagaaatccctgaacgctcgtggaattccggacatgaatgggtcacggattttaaagggaagactgtttggttcgttccaagtataaaagcaggaaatgatatagcagcttgcctgaggaaaaatggaaagaaagtgatacaactcagtaggaagacctttgattctgagtatgtcaagactagaaccaatgattgggacttcgtggttacaactgacatttcagaaatgggtgccaatttcaaggctgagagggttatagaccccagacgctgcatgaaaccagtcatactaacagatggtgaagagcgggtgattctggcaggacctatgccagtgacccactctagtgcagcacaaagaagagggagaataggaagaaatccaaaaaatgagaatgaccagtacatatacatgggggaacctctggaaaatgatgaagactgtgcacactggaaagaagctaaaatgctcctagataacatcaacacgccagaaggaatcattcctagcatgttcgaaccagagcgtgaaaaggtggatgccattgatggcgaataccgcttgagaggagaagcaaggaaaacctttgtagacttaatgagaagaggagacctaccagtctggttggcctacagagtggcagctgaaggcatcaactacgcagacagaaggtggtgttttgatggagtcaagaacaaccaaatcctagaagaaaacgtggaagttgaaatctggacaaaagaaggggaaaggaagaaattgaaacccagatggttggatgctaggatctattctgacccactggcgctaaaagaatttaaggaatttgcagccggaagaaagtctctgaccctgaacctaatcacagaaatgggtaggctcccaaccttcatgactcagaaggcaagagacgcactggacaacttagcagtgctgcacacggctgaggcaggtggaagggcgtacaaccatgctctcagtgaactgccggagaccctggagacattgcttttactgacacttctggctacagtcacgggagggatctttttattcttgatgagcgcaaggggcatagggaagatgaccctgggaatgtgctgcataatcacggctagcatcctcctatggtacgcacaaatacagccacactggatagcagcttcaataatactggagttttttctcatagttttgcttattccagaacctgaaaaacagagaacaccccaagacaaccaactgacctacgttgtcatagccatcctcacagtggtggccgcaaccatggcaaacgagatgggtttcctagaaaaaacgaagaaagatctcggattgggaagcattgcaacccagcaacccgagagcaacatcctggacatagatctacgtcctgcatcagcatggacgctgtatgccgtggccacaacatttgttacaccaatgttgagacatagcattgaaaattcctcagtgaatgtgtccctaacagctatagccaaccaagccacagtgttaatgggtctcgggaaaggatggccattgtcaaagatggacatcggagttccccttctcgccattggatgctactcacaagtcaaccccataactctcacagcagctcttttcttattggtagcacattatgccatcatagggccaggactccaagcaaaagcaaccagagaagctcagaaaagagcagcggcgggcatcatgaaaaacccaactgtcgatggaataacagtgattgacctagatccaataccttatgatccaaagtttgaaaagcagttgggacaagtaatgctcctagtcctctgcgtgactcaagtattgatgatgaggactacatgggctctgtgtgaggctttaaccttagctaccgggcccatctccacattgtgggaaggaaatccagggaggttttggaacactaccattgcggtgtcaatggctaacatttttagagggagttacttggccggagctggacttctcttttctattatgaagaacacaaccaacacaagaaggggaactggcaacataggagagacgcttggagagaaatggaaaagccgattgaacgcattgggaaaaagtgaattccagatctacaagaaaagtggaatccaggaagtggatagaaccttagcaaaagaaggcattaaaagaggagaaacggaccatcacgctgtgtcgcgaggctcagcaaaactgagatggttcgttgagagaaacatggtcacaccagaagggaaagtagtggacctcggttgtggcagaggaggctggtcatactattgtggaggactaaagaatgtaagagaagtcaaaggcctaacaaaaggaggaccaggacacgaagaacccatccccatgtcaacatatgggtggaatctagtgcgtcttcaaagtggagttgacgttttcttcatcccgccagaaaagtgtgacacattattgtgtgacataggggagtcatcaccaaatcccacagtggaagcaggacgaacactcagagtccttaacttagtagaaaattggttgaacaacaacactcaattttgcataaaggttctcaacccatatatgccctcagtcatagaaaaaatggaagcactacaaaggaaatatggaggagccttagtgaggaatccactctcacgaaactccacacatgagatgtactgggtatccaatgcttccgggaacatagtgtcatcagtgaacatgatttcaaggatgttgatcaacagatttacaatgagatacaagaaagccacttacgagccggatgttgacctcggaagcggaacccgtaacatcgggattgaaagtgagataccaaacctagatataattgggaaaagaatagaaaaaataaagcaagagcatgaaacatcatggcactatgaccaagaccacccatacaaaacgtgggcataccatggtagctatgaaacaaaacagactggatcagcatcatccatggtcaacggagtggtcaggctgctgacaaaaccttgggacgtcgtccccatggtgacacagatggcaatgacagacacgactccatttggacaacagcgcgtttttaaagagaaagtggacacgagaacccaagaaccgaaagaaggcacgaagaaactaatgaaaataacagcagagtggctttggaaagaattagggaagaaaaagacacccaggatgtgcaccagagaagaattcacaagaaaggtgagaagcaatgcagccttgggggccatattcactgatgagaacaagtggaagtcggcacgtgaggctgttgaagatagtaggttttgggagctggttgacaaggaaaggaatctccatcttgaaggaaagtgtgaaacatgtgtgtacaacatgatgggaaaaagagagaagaagctaggggaattcggcaaggcaaaaggcagcagagccatatggtacatgtggcttggagcacgcttcttagagtttgaagccctaggattcttaaatgaagatcactggttctccagagagaactccctgagtggagtggaaggagaagggctgcacaagctaggttacattctaagagacgtgagcaagaaagagggaggagcaatgtatgccgatgacaccgcaggatgggatacaagaatcacactagaagacctaaaaaatgaagaaatggtaacaaaccacatggaaggagaacacaagaaactagccgaggccattttcaaactaacgtaccaaaacaaggtggtgcgtgtgcaaagaccaacaccaagaggcacagtaatggacatcatatcgagaagagaccaaagaggtagtggacaagttggcacctatggactcaatactttcaccaatatggaagcccaactaatcagacagatggagggagaaggagtctttaaaagcattcagcacctaacaatcacagaagaaatcgctgtgcaaaactggttagcaagagtggggcgcgaaaggttatcaagaatggccatcagtggagatgattgtgttgtgaaacctttagatgacaggttcgcaagcgctttaacagctctaaatgacatgggaaagattaggaaagacatacaacaatgggaaccttcaagaggatggaatgattggacacaagtgcccttctgttcacaccatttccatgagttaatcatgaaagacggtcgcgtactcgttgttccatgtagaaaccaagatgaactgattggcagagcccgaatctcccaaggagcagggtggtctttgcgggagacggcctgtttggggaagtcttacgcccaaatgtggagcttgatgtacttccacagacgcgacctcaggctggcggcaaatgctatttgctcggcagtaccatcacattgggttccaacaagtcgaacaacctggtccatacatgctaaacatgaatggatgacaacggaagacatgctgacagtctggaacagggtgtggattcaagaaaacccatggatggaagacaaaactccagtggaatcatgggaggaaatcccatacttggggaaaagagaagaccaatggtgcggctcattgattgggttaacaagcagggccacctgggcaaagaacatccaagcagcaataaatcaagttagatcccttataggcaatgaagaatacacagattacatgccatccatgaaaagattcagaagagaagaggaagaagcaggagttctgtggtagaaagcaaaactaacatgaaacaaggctagaagtcaggtcggattaagccatagtacggaaaaaactatgctacctgtgagccccgtccaaggacgttaaaagaagtcaggccatcataaatgccatagcttgagtaaactatgcagcctgtagctccacctgagaaggtgtaaaaaatccgggaggccacaaaccatggaagctgtacgcatggcgtagtggactagcggttagaggagacccctcccttacaaatcgcagcaacaatgggggcccaaggcgagatgaagctgtagtctcgctggaaggactagaggttagaggagacccccccgaaacaaaaaacagcatattgacgctgggaaagaccagagatcctgctgtctcctcagcatcattccaggcacagaacgccagaaaatggaatggtgctgttgaatcaacaggttct

SEQ ID NO: 22 - protein, 3406 aa, Artificial Sequence
  Synthetic polypeptide
MNNQRKKAKNTPFNMLKRERNRVSTVQQLTKRFSLGMLQGRGPLKLFMALVAFLRFLTIPPTAGILKRWGTIKKSKAINVLRGFRKEIGRMLNILNRRRRSAGTSVGIVGLLLTTAMAAEVTRRGSAYYMYLDRNDAGEAISFPTTLGMNKCYIQIMDLGHMCDATMSYECPMLDEGVEPDDVDCWCNTTSTWVVYGTCHHKKGEARRSRRAVTLPSHSTRKLQTRSQTWLESREYTKHLIRVENWIFRNPGFALAAAAIAWLLGSSTSQKVIYLVMILLIAPAYSIRCIGVSNRDFVEGMSGGTWVDIVLEHGGCVTVMAQDKPTVDIELVTTTVSNMAEVRSYCYEASISDMASDSRCPTQGEAYLDKQSDTQYVCKRTLVDRGWGNGCGLFGKGSLVTCAKFACSKKMTGKSIQPENLEYRIMLSVHGSQHSGMIVNDTGHETDENRAKVEITPNSPRAEATLGGFGSLGLDCEPRTGLDFSDLYYLTMNNKHWLVHKEWFHDIPLPWHAGADTGTPHWNNKEALVEFKDAHAKRQTVVVLGSQEGAVHTALAGALEAEMDGAKGRLSSGHLKCRLKMDKLRLKGVSYSLCTAAFTFTKIPAETLHGTVTVEVQYAGTDGPCKVPAQMAVDMQTLTPVGRLITANPVITESTENSKMMLELDPPFGDSYIVIGVGEKKITHHWHRSGSTIGKAFEATVRGAKRMAVLGDTAWDFGSVGGALNSLGKGIHQIFGAAFKSLFGGMSWFSRILIGTLLMWLGLNTKNGSTSLMCLAAGFVTLYLGVMVQADSGCVVSWKNKELKCGSGIFITDNVHTWTEQYKFQPESPSKLASAIQKAHEEDICGIRSVTRLENLMWKQITPELNHILSENEVKLTIMTGDIKGIMQAGKRSLRPQPTELKYSWKTWGKAKMLSTESHNQTFLIDGPETAECPNTNRAWNSLEVEDYGFGVFTTNIWLKLKEKQDVFCDSKLMSAAIKDNRAVHADMGYWIESALNDTWKIEKASFIEVKNCHWPKSHTLWSNGVLESEMIIPKNLAGPVSQHNYRPGYHTQITGPWHLGKLEMDFDFCDGTTVVVTEDCGNRGPSLRTTTASGKLITEWCCRSCTLPPLRYRGEDGCWYGMEIRPLKEKEENLVNSLVTAGHGQVDNFSLGVLGMALFLEEMLRTRVGTKHAILLVAVSFVTLITGNMSFRDLGRVMVMVGATMTDDIGMGVTYLALLAAFKVRPTFAAGLLLRKLTSNELMMTTIGIVLLSQSTIPETILELTDALALGMMVLKMVRNMEKYQLAVTIMAILCVPNAVILQNAWKVSCTILAVVSVSPLFLTSSQQKTDWIPLALTIKGLNPTAIFLTTLSRTSKKRSWPLNEAIMAVGMVSILASSLLKNDIPMTGPLVAGGLLTVCYVLTGRSADLELERAADVKWEDQAEISGSSPILSITISEDGSMSIKNEEEEQTLTILIRTGLLVISGLFPVSIPITAAAWYLWEVKKQRAGVLWDVPSPPPMGKAELEDGAYRIKQKGILGYSQIGAGVYKEGTFHTMWHVTRGAVLMHKGKRIEPSWADVKKDLISYGGGWKLEGEWKEGEEVQVLALEPGKNPRAVQTKPGLFKTNAGTIGAVSLDFSPGTSGSPIIDKKGKVVGLYGNGVVTRSGAYVSAIAQTEKSIEDNPEIEDDIFRKRRLTIMDLHPGAGKTKRYLPAIVREAIKRGLRTLILAPTRVVAAEMEEALRGLPIRYQTPAIRAVHTGREIVDLMCHATFTMRLLSPVRVPNYNLIIMDEAHFTDPASIAARGYISTRVEMGEAAGIFMTATPPGSRDPFPQSNAPIIDEEREIPERSWNSGHEWVTDFKGKTVWFVPSIKAGNDIAACLRKNGKKVIQLSRKTFDSEYVKTRTNDWDFVVTTDISEMGANFKAERVIDPRRCMKPVILTDGEERVILAGPMPVTHSSAAQRRGRIGRNPKNENDQYIYMGEPLENDEDCAHWKEAKMLLDNINTPEGIIPSMFEPEREKVDAIDGEYRLRGEARKTFVDLMRRGDLPVWLAYRVAAEGINYADRRWCFDGVKNNQILEENVEVEIWTKEGERKKLKPRWLDARIYSDPLALKEFKEFAAGRKSLTLNLITEMGRLPTFMTQKARDALDNLAVLHTAEAGGRAYNHALSELPETLETLLLLTLLATVTGGIFLFLMSARGIGKMTLGMCCIITASILLWYAQIQPHWIAASIILEFFLIVLLIPEPEKQRTPQDNQLTYVVIAILTVVAATMANEMGFLEKTKKDLGLGSIATQQPESNILDIDLRPASAWTLYAVATTFVTPMLRHSIENSSVNVSLTAIANQATVLMGLGKGWPLSKMDIGVPLLAIGCYSQVNPITLTAALFLLVAHYAIIGPGLQAKATREAQKRAAAGIMKNPTVDGITVIDLDPIPYDPKFEKQLGQVMLLVLCVTQVLMMRTTWALCEALTLATGPISTLWEGNPGRFWNTTIAVSMANIFRGSYLAGAGLLFSIMKNTTNTRRGTGNIGETLGEKWKSRLNALGKSEFQIYKKSGIQEVDRTLAKEGIKRGETDHHAVSRGSAKLRWFVERNMVTPEGKVVDLGCGRGGWSYYCGGLKNVREVKGLTKGGPGHEEPIPMSTYGWNLVRLQSGVDVFFIPPEKCDTLLCDIGESSPNPTVEAGRTLRVLNLVENWLNNNTQFCIKVLNPYMPSVIEKMEALQRKYGGALVRNPLSRNSTHEMYWVSNASGNIVSSVNMISRMLINRFTMRYKKATYEPDVDLGSGTRNIGIESEIPNLDIIGKRIEKIKQEHETSWHYDQDHPYKTWAYHGSYETKQTGSASSMVNGVVRLLTKPWDVVPMVTQMAMTDTTPFGQQRVFKEKVDTRTQEPKEGTKKLMKITAEWLWKELGKKKTPRMCTREEFTRKVRSNAALGAIFTDENKWKSAREAVEDSRFWELVDKERNLHLEGKCETCVYNMMGKREKKLGEFGKAKGSRAIWYMWLGARFLEFEALGFLNEDHWFSRENSLSGVEGEGLHKLGYILRDVSKKEGGAMYADDTAGWDTRITLEDLKNEEMVTNHMEGEHKKLAEAIFKLTYQNKVVRVQRPTPRGTVMDIISRRDQRGSGQVGTYGLNTFTNMEAQLIRQMEGEGVFKSIQHLTITEEIAVQNWLARVGRERLSRMAISGDDCVVKPLDDRFASALTALNDMGKIRKDIQQWEPSRGWNDWTQVPFCSHHFHELIMKDGRVLVVPCRNQDELIGRARISQGAGWSLRETACLGKSYAQMWSLMYFHRRDLRLAANAICSAVPSHWVPTSRTTWSIHAKHEWMTTEDMLTVWNRVWIQENPWMEDKTPVESWEEIPYLGKREDQWCGSLIGLTSRATWAKNIQAAINQVRSLIGNEEYTDYMPSMKRFRREEEEAGVLW

SEQ ID NO: 23 - DNA, 10768 bp, Artificial Sequence
  Synthetic construct
agttgttagtctacgtggaccgacaaagacagattctttgagggagctaagctcaacgtagttctaacagttttttaattagagagcagatctctgatgaataaccaacggaaaaaggcgaaaaacacgcctttcaatatgctgaaacgcgagagaaaccgcgtgtcgactgtgcaacagctgacaaagagattctcacttggaatgctgcagggacgaggaccattaaaactgttcatggccctggtggcgttccttcgtttcctaacaatcccaccaacagcagggatattgaagagatggggaacaattaaaaaatcaaaagctattaatgttttgagagggttcaggaaagagattggaaggatgctgaacatcttgaataggagacgcagatccgcgggtactagtgtcggaattgttggcctcctgctgaccacagctatggcagcggaggtcactagacgtgggagtgcatactatatgtacttggacagaaacgatgctggggaggccatatcttttccaaccacattggggatgaataagtgttatatacagatcatggatcttggacacatgtgtgatgccaccatgagctatgaatgccctatgctggatgagggggtggaaccagatgacgtcgattgttggtgcaacacgacgtcaacttgggttgtgtacggaacctgccatcacaaaaaaggtgaagcacggagaagtagaagagctgtgacgctcccctcccattccactaggaagctgcaaacgcggtcgcaaacctggttggaatcaagagaatacacaaagcacttgattagagtcgaaaattggatattcaggaaccctggcttcgcgttagcagcagctgccatcgcttggcttttgggaagctcaacgagccaaaaagtcatatacttggtcatgatactgctgattgccccggcatacagcatcaggtgcataggagtcagcaatagggactttgtggaaggtatgtcaggtgggacttgggttgatattgtcttggaacatggaggttgtgtcaccgtaatggcacaggacaaaccgactgtcgacatagagctggttacaacaacagtcagcaacatggcggaggtaagatcctactgctatgaggcatcaatatcagacatggcttcggacagccgctgcccaacacaaggtgaagcctaccttgacaagcaatcagacactcaatatgtctgcaaaagaacgttagtggacagaggctggggaaatggatgtggactttttggcaaagggagtctggtgacatgcgctaagtttgcatgctccaagaaaatgaccgggaagagcatccagccagagaatctggagtaccggataatgctgtcagttcatggctcccagcacagtgggatgatcgttaatgacacaggacatgaaactgatgagaatagagcgaaggttgagataacgcccaattcaccaagagccgaagccaccctggggggttttggaagcctaggacttgattgtgaaccgaggacaggccttgacttttcagatttgtattacttgactatgaataacaagcactggttggttcacaaggagtggttccacgacattccattaccttggcacgctggggcagacaccggaactccacactggaacaacaaagaagcactggtagagttcaaggacgcacatgccaaaaggcaaactgtcgtggttctagggagtcaagaaggagcagttcacacggcccttgctggagctctggaggctgagatggatggtgcaaagggaaggctgtcctctggccacttgaaatgtcgcctgaaaatggataaacttagattgaagggcgtgtcatactccttgtgtaccgcagcgttcacattcaccaagatcccggctgaaacactgcacgggacagtcacagtggaggtacagtacgcagggacagatggaccttgcaaggttccagctcagatggcggtggacatgcaaactctgaccccagttgggaggttgataaccgctaaccccgtaatcactgaaagcactgagaactctaagatgatgctggaacttgatccaccatttggggactcttacattgtcataggagtcggggagaagaagatcacccaccactggcacaggagtggcagcaccattggaaaagcatttgaagccactgtgagaggtgccaagagaatggcagtcttgggagacacagcctgggactttggatcagttggaggcgctctcaactcattgggcaagggcatccatcaaatttttggagcagctttcaaatcattgtttggaggaatgtcctggttctcaagaattctcattggaacgttgctgatgtggttgggtctgaacacaaagaatggatctacttcccttatgtgcttggccgccggctttgtgacactgtatttgggggtcatggtgcaggccgatagtggttgcgttgtgagctggaaaaacaaagaactgaaatgtggcagtgggattttcatcacagacaacgtgcacacatggacagaacaatacaagttccaaccagaatccccttcaaaactagcttcagctatccagaaagcccatgaagagggcatttgtggaatccgctcagtaacaagactggagaatctgatgtggaaacaaataacaccagaattgaatcacattctatcagaaaatgaggtgaagttaactattatgacaggagacatcaaaggaatcatgcaggcaggaaaacgatctctgcggcctcagcccactgagctgaagtattcatggaaaacatggggcaaagcaaaaatgctctctacagagtctcataaccagacctttctcattgatggccccgaaacagcagaatgccccaacacaaatagagcttggaattcgttggaagttgaagactatggctttggagtattcaccaccaatatatggctaaaattgaaagaaaaacaggatgtattctgcgactcaaaactcatgtcagcggccataaaagacaacagagccgtccatgccgatatgggttattggatagaaagtgcactcaatgacacatggaagatagagaaagcctctttcattgaagttaaaaactgccactggccaaaatcacacaccctctggagcaatggagtgctagaaagtgagatgataattccaaagaatctcgctggaccagtgtctcaacacaactatagaccaggctaccatacacaaataacaggaccatggcatctaggtaagcttgagatggactttgatttctgtgatggaacaacagtggtagtgactgaggactgcggaaatagaggaccctctttgagaacaaccactgcctctggaaaactcataacagaatggtgctgccgatcttgcacattaccaccgctaagatacagaggtgaggatgggtgctggtacgggatggaaatcagaccattgaaggagaaagaagagaatttggtcaactccttggtcacagctggacatgggcaggtcgacaacttttcactaggagtcttgggaatggcattgttcctggaggaaatgcttaggacccgagtaggaacgaaacatgcaatactactagttgcagtttcttttgtgacattgatcacagggaacatgtcctttagagacctgggaagagtgatggttatggtaggcgccactatgacggatgacataggtatgggcgtgacttatcttgccctactagcagccttcaaagtcagaccaacttttgcagctggactactcttgagaaagctgacctccaatgaattgatgatgactactataggaattgtactcctctcccagagcaccataccagagaccattcttgagttgactgatgcgttagccttaggcatgatggtcctcaaaatggtgagaaatatggaaaagtatcaattggcagtgactatcatggctatcttgtgcgtcccaaacgcagtgatattacaaaacgcatggaaagtgagttgcacaatattggcagtggtgtccgtttccccactgctcttaacatcctcacagcaaaaaacagattggataccattagcattgacgatcaaaggtctcaatccaacagctatttttctaacaaccctctcaagaaccagcaagaaaaggagctggccattaaatgaggctatcatggcagtcgggatggtgagcattttagccagttctctcctaaaaaatgatattcccatgacaggaccattagtggctggagggctcctcactgtgtgctacgtgctcactggacgatcggccgatttggaactggagagagcagccgatgtcaaatgggaagaccaggcagagatatcaggaagcagtccaatcctgtcaataacaatatcagaagatggtagcatgtcgataaaaaatgaagaggaagaacaaacactgaccatactcattagaacaggattgctggtgatctcaggactttttcctgtatcaataccaatcacggcagcagcatggtacctgtgggaagtgaagaaacaacgggccggagtattgtgggatgttccttcacccccacccatgggaaaggctgaactggaagatggagcctatagaattaagcaaaaagggattcttggatattcccagatcggagccggagtttacaaagaaggaacattccatacaatgtggcatgtcacacgtggcgctgttctaatgcataaaggaaagaggattgaaccatcatgggcggacgtcaagaaagacctaatatcatatggaggaggctggaagttagaaggagaatggaaggaaggagaagaagtccaggtattggcactggagcctggaaaaaatccaagagccgtccaaacgaaacctggtcttttcaaaaccaacgccggaacaataggtgctgtatctctggacttttctcctggaacgtcaggatctccaattatcgacaaaaaaggaaaagttgtgggtctttatggtaatggtgttgttacaaggagtggagcatatgtgagtgctatagcccagactgaaaaaagcattgaagacaacccagagatcgaagatgacattttccgaaagagaagactgaccatcatggacctccacccaggagcgggaaagacgaagagataccttccggccatagtcagagaagctataaaacggggtttgagaacattaatcttggcccccactagagttgtggcagctgaaatggaggaagcccttagaggacttccaataagataccagaccccagccatcagagctgagcacaccgggcgggagattgtggacctaatgtgtcatgccacatttaccatgaggctgctatcaccagttagagtgccaaactacaacctgattatcatggacgaagcccatttcacagacccagcaagtatagcagctagaggatacatctcaactcgagtggagatgggtgaggcagctgggatttttatgacagccactcccccgggaagcagagacccatttcctcagagcaatgcaccaatcatagatgaagaaagagaaatccctgaacgttcgtggaattccggacatgaatgggtcacggattttaaagggaagactgtttggttcgttccaagtataaaagcaggaaatgatatagcagcttgcctgaggaaaaatggaaagaaagtgatacaactcagtaggaagacctttgattctgagtatgtcaagactagaaccaatgattgggacttcgtggttacaactgacatttcagaaatgggtgccaatttcaaggctgagagggttatagaccccagacgctgcatgaaaccagtcatactaacagatggtgaagagcgggtgattctggcaggacctatgccagtgacccactctagtgcagcacaaagaagagggagaataggaagaaatccaaaaaatgagaatgaccagtacatatacatgggggaacctctggaaaatgatgaagactgtgcacactggaaagaagctaaaatgctcctagataacatcaacacgccagaaggaatcattcctagcatgttcgaaccagagcgtgaaaaggtggatgccattgatggcgaataccgcttgagaggagaagcaaggaaaacctttgtagacttaatgagaagaggagacctaccagtctggttggcctacagagtggcagctgaaggcatcaactacgcagacagaaggtggtgttttgatggagtcaagaacaaccaaatcctagaagaaaacgtggaagttgaaatctggacaaaagaaggggaaaggaagaaattgaaacccagatggttggatgctaggatctattctgacccactggcgctaaaagaatttaaggaatttgcagccggaagaaagtctctgaccctgaacctaatcacagaaatgggtaggctcccaaccttcatgactcagaaggcaagaaacgcactggacaacttagcagtgctgcacacggctgaggcaggtggaagggcgtacaaccatgctctcagtgaactgccggagaccctggagacattgcttttactgacacttctggctacagtcacgggagggatctttttattcttgatgagcggaaggggcatagggaagatgaccctgggaatgtgctgcataatcacggctagcatcctcctatggtacgcacaaatacagccacactggatagcagcttcaataatactggagttttttctcatagttttgcttattccagaacctgaaaaacagagaacaccccaagacaaccaactgacctacgttgtcatagccatcctcacagtggtggccgcaaccatggcaaacgagatgggtttcctagaaaaaacgaagaaagatctcggattgggaagcattgcaacccagcaacccgagagcaacatcctggacatagatctacgtcctgcatcagcatggacgctgtatgccgtggccacaacatttgttacaccaatgttgagacatagcattgaaaattcctcagtgaatgtgtccctaacagctatagccaaccaagccacagtgttaatgggtctcgggaaaggatggccattgtcaaagatggacatcggagttccccttctcgccattggatgctactcacaagtcaaccccataactctcacagcagctcttttcttattggtagcacattatgccatcatagggccaggactccaagcaaaagcaaccagagaagctcagaaaagagcagcggcgggcatcatgaaaaacccaactgtcgatggaataacagtgattgacctagatccaataccttatgatccaaagtttgaaaagcagttgggacaagtaatgctcctagtcctctgcgtgactcaagtattgatgatgaggactacatgggctctgtgtgaggctttaaccttagctaccgggcccatctccacattgtgggaaggaaatccagggaggttttggaacactaccattgcggtgtcaatggctaacatttttagagggagttacttggccggagctggacttctcttttctattatgaagaacacaaccaacacaagaaggggaactggcaacataggagagacgcttggagagaaatggaaaagccgattgaacgcattgggaaaaagtgaattccagatctacaagaaaagtggaatccaggaagtggatagaaccttagcaaaagaaggcattaaaagaggagaaacggaccatcacgctgtgtcgcgaggctcagcaaaactgagatggttcgttgagagaaacatggtcacaccagaagggaaagtagtggacctcggttgtggcagaggaggctggtcatactattgtggaggactaaagaatgtaagagaagtcaaaggcctaacaaaaggaggaccaggacacgaagaacccatccccatgtcaacatatgggtggaatctagtgcgtcttcaaagtggagttgacgttttcttcatcccgccagaaaagtgtgacacattattgtgtgacataggggagtcatcaccaaatcccacagtggaagcaggacgaacactcagagtccttaacttagtagaaaattggttgaacaacaacactcaattttgcataaaggttctcaacccatatatgccctcagtcatagaaaaaatggaagcactacaaaggaaatatggaggagccttagtgaggaatccactctcacgaaactccacacatgagatgtactgggtatccaatgcttccgggaacatagtgtcatcagtgaacatgatttcaaggatgttgatcaacagatttacaatgagatacaagaaagccacttacgagccggatgttgacctcggaagcggaacccgtaacatcgggattgaaagtgagataccaaacctagatataattgggaaaagaatagaaaaaataaagcaagagcatgaaacatcatggcactatgaccaagaccacccatacaaaacgtgggcataccatggtagctatgaaacaaaacagactggatcagcatcatccatggtcaacggagtggtcaggctgctgacaaaaccttgggacgtcgtccccatggtgacacagatggcaatgacagacacgactccatttggacaacagcgcgtttttaaagagaaagtggacacgagaacccaagaaccgaaagaaggcacgaagaaactaatgaaaataacagcagagtggctttggaaagaattagggaagaaaaagacacccaggatgtgcaccagagaagaattcacaagaaaggtgagaagcaatgcagccttgggggccatattcactgatgagaacaagtggaagtcggcacgtgaggctgttgaagatagtaggttttgggagctggttgacaaggaaaggaatctccatcttgaaggaaagtgtgaaacatgtgtgtacaacatgatgggaaaaagagagaagaagctaggggaattcggcaaggcaaaaggcagcagagccatatggtacatgtggcttggagcacgcttcttagagtttgaagccctaggattcttaaatgaagatcactggttctccagagagaactccctgagtggagtggaaggagaagggctgcacaagctaggttacattctaagagacgtgagcaagaaagagggaggagcaatgtatgccgatgacaccgcaggatgggatacaagaatcacactagaagacctaaaaaatgaagaaatggtaacaaaccacatggaaggagaacacaagaaactagccgaggccattttcaaactaacgtaccaaaacaaggtggtgcgtgtgcaaagaccaacaccaagaggcacagtaatggacatcatatcgagaagagaccaaagaggtagtggacaagttggcacctatggactcaatactttcaccaatatggaagcccaactaatcagacagatggagggagaaggagtctttaaaagcattcagcacctaacaatcacagaagaaatcgctgtgcaaaactggttagcaagagtggggcgcgaaaggttatcaagaatggccatcagtggagatgattgtgttgtgaaacctttagatgacaggttcgcaagcgctttaacagctctaaatgacatgggaaagattaggaaagacatacaacaatgggaaccttcaagaggatggaatgattggacacaagtgcccttctgttcacaccatttccatgagttaatcatgaaagacggtcgcgtactcgttgttccatgtagaaaccaagatgaactgattggcagagcccgaatctcccaaggagcagggtggtctttgcgggagacggcctgtttggggaagtcttacgcccaaatgtggagcttgatgtacttccacagacgcgacctcaggctggcggcaaatgctatttgctcggcagtaccatcacattgggttccaacaagtcgaacaacctggtccatacatgctaaacatgaatggatgacaacggaagacatgctgacagtctggaacagggtgtggattcaagaaaacccatggatggaagacaaaactccagtggaatcatgggaggaaatcccatacttggggaaaagagaagaccaatggtgcggctcattgattgggttaacaagcagggccacctgggcaaagaacatccaagcagcaataaatcaagttagatcccttataggcaatgaagaatacacagattacatgccatccatgaaaagattcagaagagaagaggaagaagcaggagttctgtggtagaaagcaaaactaacatgaaacaaggctagaagtcaggtcggattaagccatagtacggaaaaaactatgctacctgtgagccccgtccaaggacgttaaaagaagtcaggccatcataaatgccatagcttgagtaaactatgcagcctgtagctccacctgagaaggtgtaaaaaatccgggaggccacaaaccatggaagctgtacgcatggcgtagtggactagcggttagaggagacccctcccttacaaatcgcagcaacaatgggggcccaaggcgagatgaagctgtagtctcgctggaaggactagaggttagaggagacccccccgaaacaaaaaacagcatattgacgctgggaaagaccagagatcctgctgtctcctcagcatcattccaggcacagaacgccagaaaatggaatggtgctgttgaatcaacaggttct

SEQ ID NO: 24 - protein, 3406 aa, Artificial Sequence
  Synthetic polypeptide
MNNQRKKAKNTPFNMLKRERNRVSTVQQLTKRFSLGMLQGRGPLKLFMALVAFLRFLTIPPTAGILKRWGTIKKSKAINVLRGFRKEIGRMLNILNRRRRSAGTSVGIVGLLLTTAMAAEVTRRGSAYYMYLDRNDAGEAISFPTTLGMNKCYIQIMDLGHMCDATMSYECPMLDEGVEPDDVDCWCNTTSTWVVYGTCHHKKGEARRSRRAVTLPSHSTRKLQTRSQTWLESREYTKHLIRVENWIFRNPGFALAAAAIAWLLGSSTSQKVIYLVMILLIAPAYSIRCIGVSNRDFVEGMSGGTWVDIVLEHGGCVTVMAQDKPTVDIELVTTTVSNMAEVRSYCYEASISDMASDSRCPTQGEAYLDKQSDTQYVCKRTLVDRGWGNGCGLFGKGSLVTCAKFACSKKMTGKSIQPENLEYRIMLSVHGSQHSGMIVNDTGHETDENRAKVEITPNSPRAEATLGGFGSLGLDCEPRTGLDFSDLYYLTMNNKHWLVHKEWFHDIPLPWHAGADTGTPHWNNKEALVEFKDAHAKRQTVVVLGSQEGAVHTALAGALEAEMDGAKGRLSSGHLKCRLKMDKLRLKGVSYSLCTAAFTFTKIPAETLHGTVTVEVQYAGTDGPCKVPAQMAVDMQTLTPVGRLITANPVITESTENSKMMLELDPPFGDSYIVIGVGEKKITHHWHRSGSTIGKAFEATVRGAKRMAVLGDTAWDFGSVGGALNSLGKGIHQIFGAAFKSLFGGMSWFSRILIGTLLMWLGLNTKNGSTSLMCLAAGFVTLYLGVMVQADSGCVVSWKNKELKCGSGIFITDNVHTWTEQYKFQPESPSKLASAIQKAHEEGICGIRSVTRLENLMWKQITPELNHILSENEVKLTIMTGDIKGIMQAGKRSLRPQPTELKYSWKTWGKAKMLSTESHNQTFLIDGPETAECPNTNRAWNSLEVEDYGFGVFTTNIWLKLKEKQDVFCDSKLMSAAIKDNRAVHADMGYWIESALNDTWKIEKASFIEVKNCHWPKSHTLWSNGVLESEMIIPKNLAGPVSQHNYRPGYHTQITGPWHLGKLEMDFDFCDGTTVVVTEDCGNRGPSLRTTTASGKLITEWCCRSCTLPPLRYRGEDGCWYGMEIRPLKEKEENLVNSLVTAGHGQVDNFSLGVLGMALFLEEMLRTRVGTKHAILLVAVSFVTLITGNMSFRDLGRVMVMVGATMTDDIGMGVTYLALLAAFKVRPTFAAGLLLRKLTSNELMMTTIGIVLLSQSTIPETILELTDALALGMMVLKMVRNMEKYQLAVTIMAILCVPNAVILQNAWKVSCTILAVVSVSPLLLTSSQQKTDWIPLALTIKGLNPTAIFLTTLSRTSKKRSWPLNEAIMAVGMVSILASSLLKNDIPMTGPLVAGGLLTVCYVLTGRSADLELERAADVKWEDQAEISGSSPILSITISEDGSMSIKNEEEEQTLTILIRTGLLVISGLFPVSIPITAAAWYLWEVKKQRAGVLWDVPSPPPMGKAELEDGAYRIKQKGILGYSQIGAGVYKEGTFHTMWHVTRGAVLMHKGKRIEPSWADVKKDLISYGGGWKLEGEWKEGEEVQVLALEPGKNPRAVQTKPGLFKTNAGTIGAVSLDFSPGTSGSPIIDKKGKVVGLYGNGVVTRSGAYVSAIAQTEKSIEDNPEIEDDIFRKRRLTIMDLHPGAGKTKRYLPAIVREAIKRGLRTLILAPTRVVAAEMEEALRGLPIRYQTPAIRAEHTGREIVDLMCHATFTMRLLSPVRVPNYNLIIMDEAHFTDPASIAARGYISTRVEMGEAAGIFMTATPPGSRDPFPQSNAPIIDEEREIPERSWNSGHEWVTDFKGKTVWFVPSIKAGNDIAACLRKNGKKVIQLSRKTFDSEYVKTRTNDWDFVVTTDISEMGANFKAERVIDPRRCMKPVILTDGEERVILAGPMPVTHSSAAQRRGRIGRNPKNENDQYIYMGEPLENDEDCAHWKEAKMLLDNINTPEGIIPSMFEPEREKVDAIDGEYRLRGEARKTFVDLMRRGDLPVWLAYRVAAEGINYADRRWCFDGVKNNQILEENVEVEIWTKEGERKKLKPRWLDARIYSDPLALKEFKEFAAGRKSLTLNLITEMGRLPTFMTQKARNALDNLAVLHTAEAGGRAYNHALSELPETLETLLLLTLLATVTGGIFLFLMSGRGIGKMTLGMCCIITASILLWYAQIQPHWIAASIILEFFLIVLLIPEPEKQRTPQDNQLTYVVIAILTVVAATMANEMGFLEKTKKDLGLGSIATQQPESNILDIDLRPASAWTLYAVATTFVTPMLRHSIENSSVNVSLTAIANQATVLMGLGKGWPLSKMDIGVPLLAIGCYSQVNPITLTAALFLLVAHYAIIGPGLQAKATREAQKRAAAGIMKNPTVDGITVIDLDPIPYDPKFEKQLGQVMLLVLCVTQVLMMRTTWALCEALTLATGPISTLWEGNPGRFWNTTIAVSMANIFRGSYLAGAGLLFSIMKNTTNTRRGTGNIGETLGEKWKSRLNALGKSEFQIYKKSGIQEVDRTLAKEGIKRGETDHHAVSRGSAKLRWFVERNMVTPEGKVVDLGCGRGGWSYYCGGLKNVREVKGLTKGGPGHEEPIPMSTYGWNLVRLQSGVDVFFIPPEKCDTLLCDIGESSPNPTVEAGRTLRVLNLVENWLNNNTQFCIKVLNPYMPSVIEKMEALQRKYGGALVRNPLSRNSTHEMYWVSNASGNIVSSVNMISRMLINRFTMRYKKATYEPDVDLGSGTRNIGIESEIPNLDIIGKRIEKIKQEHETSWHYDQDHPYKTWAYHGSYETKQTGSASSMVNGVVRLLTKPWDVVPMVTQMAMTDTTPFGQQRVFKEKVDTRTQEPKEGTKKLMKITAEWLWKELGKKKTPRMCTREEFTRKVRSNAALGAIFTDENKWKSAREAVEDSRFWELVDKERNLHLEGKCETCVYNMMGKREKKLGEFGKAKGSRAIWYMWLGARFLEFEALGFLNEDHWFSRENSLSGVEGEGLHKLGYILRDVSKKEGGAMYADDTAGWDTRITLEDLKNEEMVTNHMEGEHKKLAEAIFKLTYQNKVVRVQRPTPRGTVMDIISRRDQRGSGQVGTYGLNTFTNMEAQLIRQMEGEGVFKSIQHLTITEEIAVQNWLARVGRERLSRMAISGDDCVVKPLDDRFASALTALNDMGKIRKDIQQWEPSRGWNDWTQVPFCSHHFHELIMKDGRVLVVPCRNQDELIGRARISQGAGWSLRETACLGKSYAQMWSLMYFHRRDLRLAANAICSAVPSHWVPTSRTTWSIHAKHEWMTTEDMLTVWNRVWIQENPWMEDKTPVESWEEIPYLGKREDQWCGSLIGLTSRATWAKNIQAAINQVRSLIGNEEYTDYMPSMKRFRREEEEAGVLW

SEQ ID NO: 25 - DNA, 10768 bp, Artificial Sequence
  Synthetic construct
agttgttagtctacgtggaccgacaaagacagattctttgagggagctaagctcaatgtagttctaacagttttttaattagagagcagatctctgatgaataaccaacggaaaaaggcgaaaaacacgcctttcaatatgctgaaacgcgagagaaaccgcgtgtcgactgtgcaacagctgacaaagagattctcacttggaatgctgcagggacgaggaccattaaaactgttcatggccctggtggcgttccttcgtttcctaacaatcccaccaacagcagggatattgaagagatggggaacaattaaaaaatcaaaagctattaatgttttgagagggttcaggaaagagattggaaggatgctgaacatcttgaataggagacgcagatccgcgggtactagtgtcggaattgttggcctcctgctgaccacagctatggcagcggaggtcactagacgtgggagtgcatactatatgtacttggacagaaacgatgctggggaggccatatcttttccaaccacattggggatgaataagtgttatatacagatcatggatcttggacacatgtgtgatgccaccatgagctatgaatgccctatgctggatgagggggtggaaccagatgacgtcgattgttggtgcaacacgacgtcaacttgggttgtgtacggaacctgccatcacaaaaaaggtgaagcacggagaagtagaagagctgtgacgctcccctcccattccactaggaagctgcaaacgcggtcgcaaacctggttggaatcaagagaatacacaaagcacttgattagagtcgaaaattggatattcaggaaccctggcttcgcgttagcagcagctgccatcgcttggcttttgggaagctcaacgagccaaaaagtcatatacttggtcatgatactgctgattgccccggcatacagcatcaggtgcataggagtcagcaatagggactttgtggaaggtatgtcaggtgggacttgggttgatattgtcttggaacatggaggttgtgtcaccgtaatggcacaggacaaaccgactgtcgacatagagctggttacaacaacagtcagcaacatggcggaggtaagatcctactgctatgaggcatcaatatcagacatggcttcggacagccgctgcccaacacaaggtgaagcctaccttgacaagcaatcagacactcaatatgtctgcaaaagaacgttagtggacagaggctggggaaatggatgtggactttttggcaaagggagtctggtgacatgcgctaagtttgcatgctccaagaaaatgaccgggaagagcatccagccagagaatctggagtaccggataatgctgtcagttcatggctcccagcacagtgggatgatcgttaatgacacaggacatgaaactgatgagaatagagcgaaggttgagataacgcccaattcaccaagagccgaagccaccctggggggttttggaagcctaggacttgattgtgaaccgaggacaggccttgacttttcagatttgtattacttgactatgaataacaagcactggttggttcacaaggagtggttccacgacattccattaccttggcacgctggggcagacaccggaactccacactggaacaacaaagaagcactggtagagttcaaggacgcacatgccaaaaggcaaactgtcgtggttctagggagtcaagaaggagcagttcacacggcccttgctggagctctggaggctgagatggatggtgcaaagggaaggctgtcctctggccacttgaaatgtcgcctgaaaatggataaacttagattgaagggcgtgtcatactccttgtgtaccgcagcgttcacattcaccaagatcccggctgaaacactgcacgggacagtcacagtggaggtacagtacgcagggacagatggaccttgcaaggttccagctcagatggcggtggacatgcaaactctgaccccagttgggaggttgataaccgctaaccccgtaatcactgaaagcactgagaactctaagatgatgctggaacttgatccaccatttggggactcttacattgtcataggagtcggggagaagaagatcacccaccactggcacaggagtggcagcaccattggaaaagcatttgaagccactgtgagaggtgccaagagaatggcagtcttgggagacacagcctgggactttggatcagttggaggcgctctcaactcattgggcaagggcatccatcaaatttttggagcagctttcaaatcattgtttggaggaatgtcctggttctcaagaattctcattggaacgttgctgatgtggttgggtctgaacacaaagaatggatctacttcccttatgtgcttggccgccggctttgtgacactgtatttgggagtcatggtgcaggccgatagtggttgcgttgtgagctggaaaaacaaagaactgaaatgtggcagtgggattttcatcacagacaacgtgcacacatggacagaacaatacaagttccaaccagaatccccttcaaaactagcttcagctatccagaaagcccatgaagaggacatttgtggaatccgctcagtaacaagactggagaatctgatgtggaaacaaataacaccagaattgaatcacattctatcagaaaatgaggtgaagttaactattatgacaggagacatcaaaggaatcatgcaggcaggaaaacgatctctgcggcctcagcccactgagctgaagtattcatggaaaacatggggcaaagcaaaaatgctctctacagagtctcataaccagacctttctcattgatggccccgaaacagcagaatgccccaacacaaatagagcttggaattcgttggaagttgaagactatggctttggagtattcaccaccaatatatggctaaaattgaaagaaaaacaggatgtattctgcgactcaaaactcatgtcagcggccataaaagacaacagagccgtccatgccgatatgggttattggatagaaagtgcactcaatgacacatggaagatagagaaagcctctttcattgaagttaaaaactgccactggccaaaatcacacaccctctggagcaatggagtgctagaaagtgagatgataattccaaagaatctcgctggaccagtgtctcaacacaactatagaccaggctaccatacacaaataacaggaccatggcatctaggtaagcttgagatggactttgatttctgtgatggaacaacagtggtagtgactgaggactgcggaaatagaggaccctctttgagaacaaccactgcctctggaaaactcataacagaatggtgctgccgatcttgcacattaccaccgctaagatacagaggtgaggatgggtgctggtacgggatggaaatcagaccattgaaggagaaagaagagaatttggtcaactccttggtcacagctggacatgggcaggtcgacaacttttcactaggagtcttgggaatggcattgttcctggaggaaatgcttaggacccgagtaggaacgaaacatgcaatactactagttgcagtttcttttgtgacattgatcacagggaacatgtcctttagagacctgggaagagtgatggttatggtaggcgccactatgacggatgacataggtatgggcgtgacttatcttgccctactagcagccttcaaagtcagaccaacttttgcagctggactactcttgagaaagctgacctccaatgaattgatgatgactactataggaattgtactcctctcccagagcaccataccagagaccattcttgagttgactgatgcgttagccttaggcatgatggtcctcaaaatggtgagaaatatggaaaagtatcaattggcagtgactatcatggctatcttgtgcgtcccaaacgcagtgatattacaaaacgcatggaaagtgagttgcacaatattggcagtggtgtccgtttccccactgttcttaacatcctcacagcaaaaaacagattggataccattagcattgacgatcaaaggtctcaatccaacagctatttttctaacaaccctctcaagaaccagcaagaaaaggagctggccattaaatgaggctatcatggcagtcgggatggtgagcattttagccagttctctcctaaaaaatgatattcccatgacaggaccattagtggctggagggctcctcactgtgtgctacgtgctcactggacgatcggccgatttggaactggagagagcagccgatgtcaaatgggaagaccaggcagagatatcaggaagcagtccaatcctgtcaataacaatatcagaagatggtagcatgtcgataaaaaatgaagaggaagaacaaacactgaccatactcattagaacaggattgctggtgatctcaggactttttcctgtatcaataccaatcacggcagcagcatggtacctgtgggaagtgaagaaacaacgggccggagtattgtgggatgttccttcacccccacccatgggaaaggctgaactggaagatggagcctatagaattaagcaaaaagggattcttggatattcccagatcggagccggagtttacaaagaaggaacattccatacaatgtggcatgtcacacgtggcgctgttctaatgcataaaggaaagaggattgaaccatcatgggcggacgtcaagaaagacctaatatcatatggaggaggctggaagttagaaggagaatggaaggaaggagaagaagtccaggtattggcactggagcctggaaaaaatccaagagccgtccaaacgaaacctggtcttttcaaaaccaacgccggaacaataggtgctgtatctctggacttttctcctggaacgtcaggatctccaattatcgacaaaaaaggaaaagttgtgggtctttatggtaatggtgttgttacaaggagtggagcatatgtgagtgctatagcccagactgaaaaaagcattgaagacaacccagagatcgaagatgacattttccgaaagagaagactgaccatcatggacctccacccaggagcgggaaagacgaagagataccttccggccatagtcagagaagctataaaacggggtttgagaacattaatcttggcccccactagagttgtggcagctgaaatggaggaagcccttagaggacttccaataagataccagaccccagccatcagagctgtgcacaccgggcgggagattgtggacctaatgtgtcatgccacatttaccatgaggctgctatcaccagttagagtgccaaactacaacctgattatcatggacgaagcccatttcacagacccagcaagtatagcagctagaggatacatctcaactcgagtggagatgggtgaggcagctgggatttttatgacagccactcccccgggaagcagagacccatttcctcagagcaatgcaccaatcatagatgaagaaagagaaatccctgaacgctcgtggaattccggacatgaatgggtcacggattttaaagggaagactgtttggttcgttccaagtataaaagcaggaaatgatatagcagcttgcctgaggaaaaatggaaagaaagtgatacaactcagtaggaagacctttgattctgagtatgtcaagactagaaccaatgattgggacttcgtggttacaactgacatttcagaaatgggtgccaatttcaaggctgagagggttatagaccccagacgctgcatgaaaccagtcatactaacagatggtgaagagcgggtgattctggcaggacctatgccagtgacccactctagtgcagcacaaagaagagggagaataggaagaaatccaaaaaatgagaatgaccagtacatatacatgggggaacctctggaaaatgatgaagactgtgcacactggaaagaagctaaaatgctcctagataacatcaacacgccagaaggaatcattcctagcatgttcgaaccagagcgtgaaaaggtggatgccattgatggcgaataccgcttgagaggagaagcaaggaaaacctttgtagacttaatgagaagaggagacctaccagtctggttggcctacagagtggcagctgaaggcatcaactacgcagacagaaggtggtgttttgatggagtcaagaacaaccaaatcctagaagaaaacgtggaagttgaaatctggacaaaagaaggggaaaggaagaaattgaaacccagatggttggatgctaggatctattctgacccactggcgctaaaagaatttaaggaatttgcagccggaagaaagtctctgaccctgaacctaatcacagaaatgggtaggctcccaaccttcatgactcagaaggcaagaaacgcactggacaacttagcagtgctgcacacggctgaggcaggtggaagggcgtacaaccatgctctcagtgaactgccggagaccctggagacattgcttttactgacacttctggctacagtcacgggagggatctttttattcttgatgagcgcaaggggcatagggaagatgaccctgggaatgtgctgcataatcacggctagcatcctcctatggtacgcacaaatacagccacactggatagcagcttcaataatactggagttttttctcatagttttgcttattccagaacctgaaaaacagagaacaccccaagacaaccaactgacctacgttgtcatagccatcctcacagtggtggccgcaaccatggcaaacgagatgggtttcctagaaaaaacgaagaaagatctcggattgggaagcattgcaacccagcaacccgagagcaacatcctggacatagatctacgtcctgcatcagcatggacgctgtatgccgtggccacaacatttgttacaccaatgttgagacatagcattgaaaattcctcagtgaatgtgtccctaacagctatagccaaccaagccacagtgttaatgggtctcgggaaaggatggccattgtcaaagatggacatcggagttccccttctcgccattggatgctactcacaagtcaaccccataactctcacagcagctcttttcttattggtagcacattatgccatcatagggccaggactccaagcaaaagcaaccagagaagctcagaaaagagcagcggcgggcatcatgaaaaacccaactgtcgatggaataacagtgattgacctagatccaataccttatgatccaaagtttgaaaagcagttgggacaagtaatgctcctagtcctctgcgtgactcaagtattgatgatgaggactacatgggctctgtgtgaggctttaaccttagctaccgggcccatctccacattgtgggaaggaaatccagggaggttttggaacactaccattgcggtgtcaatggctaacatttttagagggagttacttggccggagctggacttctcttttctattatgaagaacacaaccaacacaagaaggggaactggcaacataggagagacgcttggagagaaatggaaaagccgattgaacgcattgggaaaaagtgaattccagatctacaagaaaagtggaatccaggaagtggatagaaccttagcaaaagaaggcattaaaagaggagaaacggaccatcacgctgtgtcgcgaggctcagcaaaactgagatggttcgttgagagaaacatggtcacaccagaagggaaagtagtggacctcggttgtggcagaggaggctggtcatactattgtggaggactaaagaatgtaagagaagtcaaaggcctaacaaaaggaggaccaggacacgaagaacccatccccatgtcaacatatgggtggaatctagtgcgtcttcaaagtggagttgacgttttcttcatcccgccagaaaagtgtgacacattattgtgtgacataggggagtcatcaccaaatcccacagtggaagcaggacgaacactcagagtccttaacttagtagaaaattggttgaacaacaacactcaattttgcataaaggttctcaacccatatatgccctcagtcatagaaaaaatggaagcactacaaaggaaatatggaggagccttagtgaggaatccactctcacgaaactccacacatgagatgtactgggtatccaatgcttccgggaacatagtgtcatcagtgaacatgatttcaaggatgttgatcaacagatttacaatgagatacaagaaagccacttacgagccggatgttgacctcggaagcggaacccgtaacatcgggattgaaagtgagataccaaacctagatataattgggaaaagaatagaaaaaataaagcaagagcatgaaacatcatggcactatgaccaagaccacccatacaaaacgtgggcataccatggtagctatgaaacaaaacagactggatcagcatcatccatggtcaacggagtggtcaggctgctgacaaaaccttgggacgtcgtccccatggtgacacagatggcaatgacagacacgactccatttggacaacagcgcgtttttaaagagaaagtggacacgagaacccaagaaccgaaagaaggcacgaagaaactaatgaaaataacagcagagtggctttggaaagaattagggaagaaaaagacacccaggatgtgcaccagagaagaattcacaagaaaggtgagaagcaatgcagccttgggggccatattcactgatgagaacaagtggaagtcggcacgtgaggctgttgaagatagtaggttttgggagctggttgacaaggaaaggaatctccatcttgaaggaaagtgtgaaacatgtgtgtacaacatgatgggaaaaagagagaagaagctaggggaattcggcaaggcaaaaggcagcagagccatatggtacatgtggcttggagcacgcttcttagagtttgaagccctaggattcttaaatgaagatcactggttctccagagagaactccctgagtggagtggaaggagaagggctgcacaagctaggttacattctaagagacgtgagcaagaaagagggaggagcaatgtatgccgatgacaccgcaggatgggatacaagaatcacactagaagacctaaaaaatgaagaaatggtaacaaaccacatggaaggagaacacaagaaactagccgaggccattttcaaactaacgtaccaaaacaaggtggtgcgtgtgcaaagaccaacaccaagaggcacagtaatggacatcatatcgagaagagaccaaagaggtagtggacaagttggcacctatggactcaatactttcaccaatatggaagcccaactaatcagacagatggagggagaaggagtctttaaaagcattcagcacctaacaatcacagaagaaatcgctgtgcaaaactggttagcaagagtggggcgcgaaaggttatcaagaatggccatcagtggagatgattgtgttgtgaaacctttagatgacaggttcgcaagcgctttaacagctctaaatgacatgggaaagattaggaaagacatacaacaatgggaaccttcaagaggatggaatgattggacacaagtgcccttctgttcacaccatttccatgagttaatcatgaaagacggtcgcgtactcgttgttccatgtagaaaccaagatgaactgattggcagagcccgaatctcccaaggagcagggtggtctttgcgggagacggcctgtttggggaagtcttacgcccaaatgtggagcttgatgtacttccacagacgcgacctcaggctggcggcaaatgctatttgctcggcagtaccatcacattgggttccaacaagtcgaacaacctggtccatacatgctaaacatgaatggatgacaacggaagacatgctgacagtctggaacagggtgtggattcaagaaaacccatggatggaagacaaaactccagtggaatcatgggaggaaatcccatacttggggaaaagagaagaccaatggtgcggctcattgattgggttaacaagcagggccacctgggcaaagaacatccaagcagcaataaatcaagttagatcccttataggcaatgaagaatacacagattacatgccatccatgaaaagattcagaagagaagaggaagaagcaggagttctgtggtagaaagcaaaactaacatgaaacaaggctagaagtcaggtcggattaagccatagtacggaaaaaactatgctacctgtgagccccgtccaaggacgttaaaagaagtcaggccatcataaatgccatagcttgagtaaactatgcagcctgtagctccacctgagaaggtgtaaaaaatccgggaggccacaaaccatggaagctgtacgcatggcgtagtggactagcggttagaggagacccctcccttacaaatcgcagcaacaatgggggcccaaggcgagatgaagctgtagtctcgctggaaggactagaggttagaggagacccccccgaaacaaaaaacagcatattgacgctgggaaagaccagagatcctgctgtctcctcagcatcattccaggcacagaacgccagaaaatggaatggtgctgttgaatcaacaggttct

SEQ ID NO: 26 - protein, 3406 aa, Artificial Sequence
  Synthetic polypeptide
MNNQRKKAKNTPFNMLKRERNRVSTVQQLTKRFSLGMLQGRGPLKLFMALVAFLRFLTIPPTAGILKRWGTIKKSKAINVLRGFRKEIGRMLNILNRRRRSAGTSVGIVGLLLTTAMAAEVTRRGSAYYMYLDRNDAGEAISFPTTLGMNKCYIQIMDLGHMCDATMSYECPMLDEGVEPDDVDCWCNTTSTWVVYGTCHHKKGEARRSRRAVTLPSHSTRKLQTRSQTWLESREYTKHLIRVENWIFRNPGFALAAAAIAWLLGSSTSQKVIYLVMILLIAPAYSIRCIGVSNRDFVEGMSGGTWVDIVLEHGGCVTVMAQDKPTVDIELVTTTVSNMAEVRSYCYEASISDMASDSRCPTQGEAYLDKQSDTQYVCKRTLVDRGWGNGCGLFGKGSLVTCAKFACSKKMTGKSIQPENLEYRIMLSVHGSQHSGMIVNDTGHETDENRAKVEITPNSPRAEATLGGFGSLGLDCEPRTGLDFSDLYYLTMNNKHWLVHKEWFHDIPLPWHAGADTGTPHWNNKEALVEFKDAHAKRQTVVVLGSQEGAVHTALAGALEAEMDGAKGRLSSGHLKCRLKMDKLRLKGVSYSLCTAAFTFTKIPAETLHGTVTVEVQYAGTDGPCKVPAQMAVDMQTLTPVGRLITANPVITESTENSKMMLELDPPFGDSYIVIGVGEKKITHHWHRSGSTIGKAFEATVRGAKRMAVLGDTAWDFGSVGGALNSLGKGIHQIFGAAFKSLFGGMSWFSRILIGTLLMWLGLNTKNGSTSLMCLAAGFVTLYLGVMVQADSGCVVSWKNKELKCGSGIFITDNVHTWTEQYKFQPESPSKLASAIQKAHEEDICGIRSVTRLENLMWKQITPELNHILSENEVKLTIMTGDIKGIMQAGKRSLRPQPTELKYSWKTWGKAKMLSTESHNQTFLIDGPETAECPNTNRAWNSLEVEDYGFGVFTTNIWLKLKEKQDVFCDSKLMSAAIKDNRAVHADMGYWIESALNDTWKIEKASFIEVKNCHWPKSHTLWSNGVLESEMIIPKNLAGPVSQHNYRPGYHTQITGPWHLGKLEMDFDFCDGTTVVVTEDCGNRGPSLRTTTASGKLITEWCCRSCTLPPLRYRGEDGCWYGMEIRPLKEKEENLVNSLVTAGHGQVDNFSLGVLGMALFLEEMLRTRVGTKHAILLVAVSFVTLITGNMSFRDLGRVMVMVGATMTDDIGMGVTYLALLAAFKVRPTFAAGLLLRKLTSNELMMTTIGIVLLSQSTIPETILELTDALALGMMVLKMVRNMEKYQLAVTIMAILCVPNAVILQNAWKVSCTILAVVSVSPLFLTSSQQKTDWIPLALTIKGLNPTAIFLTTLSRTSKKRSWPLNEAIMAVGMVSILASSLLKNDIPMTGPLVAGGLLTVCYVLTGRSADLELERAADVKWEDQAEISGSSPILSITISEDGSMSIKNEEEEQTLTILIRTGLLVISGLFPVSIPITAAAWYLWEVKKQRAGVLWDVPSPPPMGKAELEDGAYRIKQKGILGYSQIGAGVYKEGTFHTMWHVTRGAVLMHKGKRIEPSWADVKKDLISYGGGWKLEGEWKEGEEVQVLALEPGKNPRAVQTKPGLFKTNAGTIGAVSLDFSPGTSGSPIIDKKGKVVGLYGNGVVTRSGAYVSAIAQTEKSIEDNPEIEDDIFRKRRLTIMDLHPGAGKTKRYLPAIVREAIKRGLRTLILAPTRVVAAEMEEALRGLPIRYQTPAIRAVHTGREIVDLMCHATFTMRLLSPVRVPNYNLIIMDEAHFTDPASIAARGYISTRVEMGEAAGIFMTATPPGSRDPFPQSNAPIIDEEREIPERSWNSGHEWVTDFKGKTVWFVPSIKAGNDIAACLRKNGKKVIQLSRKTFDSEYVKTRTNDWDFVVTTDISEMGANFKAERVIDPRRCMKPVILTDGEERVILAGPMPVTHSSAAQRRGRIGRNPKNENDQYIYMGEPLENDEDCAHWKEAKMLLDNINTPEGIIPSMFEPEREKVDAIDGEYRLRGEARKTFVDLMRRGDLPVWLAYRVAAEGINYADRRWCFDGVKNNQILEENVEVEIWTKEGERKKLKPRWLDARIYSDPLALKEFKEFAAGRKSLTLNLITEMGRLPTFMTQKARNALDNLAVLHTAEAGGRAYNHALSELPETLETLLLLTLLATVTGGIFLFLMSARGIGKMTLGMCCIITASILLWYAQIQPHWIAASIILEFFLIVLLIPEPEKQRTPQDNQLTYVVIAILTVVAATMANEMGFLEKTKKDLGLGSIATQQPESNILDIDLRPASAWTLYAVATTFVTPMLRHSIENSSVNVSLTAIANQATVLMGLGKGWPLSKMDIGVPLLAIGCYSQVNPITLTAALFLLVAHYAIIGPGLQAKATREAQKRAAAGIMKNPTVDGITVIDLDPIPYDPKFEKQLGQVMLLVLCVTQVLMMRTTWALCEALTLATGPISTLWEGNPGRFWNTTIAVSMANIFRGSYLAGAGLLFSIMKNTTNTRRGTGNIGETLGEKWKSRLNALGKSEFQIYKKSGIQEVDRTLAKEGIKRGETDHHAVSRGSAKLRWFVERNMVTPEGKVVDLGCGRGGWSYYCGGLKNVREVKGLTKGGPGHEEPIPMSTYGWNLVRLQSGVDVFFIPPEKCDTLLCDIGESSPNPTVEAGRTLRVLNLVENWLNNNTQFCIKVLNPYMPSVIEKMEALQRKYGGALVRNPLSRNSTHEMYWVSNASGNIVSSVNMISRMLINRFTMRYKKATYEPDVDLGSGTRNIGIESEIPNLDIIGKRIEKIKQEHETSWHYDQDHPYKTWAYHGSYETKQTGSASSMVNGVVRLLTKPWDVVPMVTQMAMTDTTPFGQQRVFKEKVDTRTQEPKEGTKKLMKITAEWLWKELGKKKTPRMCTREEFTRKVRSNAALGAIFTDENKWKSAREAVEDSRFWELVDKERNLHLEGKCETCVYNMMGKREKKLGEFGKAKGSRAIWYMWLGARFLEFEALGFLNEDHWFSRENSLSGVEGEGLHKLGYILRDVSKKEGGAMYADDTAGWDTRITLEDLKNEEMVTNHMEGEHKKLAEAIFKLTYQNKVVRVQRPTPRGTVMDIISRRDQRGSGQVGTYGLNTFTNMEAQLIRQMEGEGVFKSIQHLTITEEIAVQNWLARVGRERLSRMAISGDDCVVKPLDDRFASALTALNDMGKIRKDIQQWEPSRGWNDWTQVPFCSHHFHELIMKDGRVLVVPCRNQDELIGRARISQGAGWSLRETACLGKSYAQMWSLMYFHRRDLRLAANAICSAVPSHWVPTSRTTWSIHAKHEWMTTEDMLTVWNRVWIQENPWMEDKTPVESWEEIPYLGKREDQWCGSLIGLTSRATWAKNIQAAINQVRSLIGNEEYTDYMPSMKRFRREEEEAGVLW